European Patent Application EP 4 137 573 A2, published February 22, 2023. Title: COMPOSITIONS FOR MODULATING SOD-1 EXPRESSION. Applicant: Isis Pharmaceuticals, Inc. The sequence listing filed with the application follows.

SEQUENCE LISTING (1461 sequences)

SEQ ID NO: 1 - DNA, 981 bp, Homo sapiens
gtttggggccagagtgggcgaggcgcggaggtctggcctataaagtagtcgcggagacggggtgctggtttgcgtcgtagtctcctgcagcgtctggggtttccgttgcagtcctcggaaccaggacctcggcgtggcctagcgagttatggcgacgaaggccgtgtgcgtgctgaagggcgacggcccagtgcagggcatcatcaatttcgagcagaaggaaagtaatggaccagtgaaggtgtggggaagcattaaaggactgactgaaggcctgcatggattccatgttcatgagtttggagataatacagcaggctgtaccagtgcaggtcctcactttaatcctctatccagaaaacacggtgggccaaaggatgaagagaggcatgttggagacttgggcaatgtgactgctgacaaagatggtgtggccgatgtgtctattgaagattctgtgatctcactctcaggagaccattgcatcattggccgcacactggtggtccatgaaaaagcagatgacttgggcaaaggtggaaatgaagaaagtacaaagacaggaaacgctggaagtcgtttggcttgtggtgtaattgggatcgcccaataaacattcccttggatgtagtctgaggccccttaactcatctgttatcctgctagctgtagaaatgtatcctgataaacattaaacactgtaatcttaaaagtgtaattgtgtgactttttcagagttgctttaaagtacctgtagtgagaaactgatttatgatcacttggaagatttgtatagttttataaaactcagttaaaatgtctgtttcaatgacctgtattttgccagacttaaatcacagatgggtattaaacttgtcagaatttctttgtcattcaagcctgtgaataaaaaccctgtatggcacttattatgaggctattaaaagaatccaaattcaaactaaaaaaaaaaaaaaaaaa

SEQ ID NO: 2 - DNA, 11001 bp, Homo sapiens
cactgcactccagcctgggtgacagagcgagaccctgtctcaaaaatcaaacaaacaaccccctcgccccggacaaaagtagtttgcactattttctcatttcacaatatgtttttgaaatatttcccttgaaaggtaagtcatatttatcattcctgttgtatggaggcatcataaattatttcaccattctaccctccttgagtgttgtggcctttaggccagacaaaaacgcaggtgatgcctagaagccaactagttgccgtttggttatctgtagggttgtggccttgccaaacaggaaaaatataaaaagaataccgaattctgccaaccaaataagaaactctatactaaggactaagaaaattgcaggggaagaaaaggtaagtcccgggattgaggtgtagcgactttctataccctcagaaaactaaaaaacaagacaaaaaaatgaaaactacaaaagcatccatcttggggcgtcccaattgctgagtaacaaatgagacgctgtggccaaactcagtcataactaatgacatttctagacaaagtgacttcagattttcaaagcgtaccctgtttacatcattttgccaatttcgcgtactgcaaccggcgggccacgcccccgtgaaaagaaggttgttttctccacatttcggggttctggacgtttcccggctgcggggcggggggagtctccggcgcacgcggccccttggccccgcccccagtcattcccggccactcgcgacccgaggctgccgcagggggcgggctgagcgcgtgcgaggcgattggtttggggccagagtgggcgaggcgcggaggtctggcctataaagtagtcgcggagacggggtgctggtttgcgtcgtagtctcctgcagcgtctggggtttccgttgcagtcctcggaaccaggacctcggcgtggcctagcgagttatggcgacgaaggccgtgtgcgtgctgaagggcgacggcccagtgcagggcatcatcaatttcgagcagaaggcaagggctgggacggaggcttgtttgcgaggccgctcccacccgctcgtccccccgcgcacctttgctaggagcgggtcgcccgccaggcctcggggccgccctggtccagcgcccggtcccggcccgtgccgcccggtcggtgccttcgcccccagcggtgcggtgcccaagtgctgagtcaccgggcgggcccgggcgcggggcgtgggaccgaggccgccgcggggctgggcctgcgcgtggcgggagcgcggggagggattgccgcgggccggggaggggcgggggcgggcgtgctgccctctgtggtccttgggccgccgccgcgggtctgtcgtggtgcctggagcggctgtgctcgtcccttgcttggccgtgttctcgttcctgagggtcccgcggacaccgagtggcgcagtgccaggcccagcccggggatggcgactgcgcctgggcccgcctggtgtcttcgcatccctctccgctttccggcttcagcgctctaggtcagggagtcttcgcttttgtacagctctaaggctaggaatggtttttatatttttaaaaggctttggaaaacaaaaatacgcaacagagaccgtttgtgtgacactttgcagggaagtttgctggcctctgttctaggtcatgattgggctgcaagggcagagaaggtagccttgaacagaggtccttttcctcctcctaagctccgggagccagaggtttaactgacccttttggggatttttgagggcagtgatcttaactttgggtgcacagttagcttatttgaagatcttactaaaaatacaccagagcccaacctccgaccaattacatcaaaacctgtcctagtgcagggtgagtattgctgttttttgaaagtttccaaaagtgattttgatgtgcacctacgattgagaactgtcgtttgaggacagtgggtggagtttcgtatttggaaattagaagacctggagtttccattacaccgaattggcacttaataactgttgtcggagcatttcttaagccacattttcgtaaagtggctttaaaattgctctgccagtaggcaggttgctaagatggtcagagacaaacttctgaacgactcttgtaaaatatacagaaatattttcagaacttttatcagtaaaattacaaaacgtgttgcaaggaaggtgcttgtgataacactgtccccagaaccttagtgaagttaccaactggtggaaaattttctcttgcactcggcttaaaaatcatgagggaatatttactatacgaatgagattcagtctttaaaggggtttacagaaacgtgagaggacaggaacagttagtctgtgtaaatgtctgaaatatatgtgagggagataatgagtttagcctttttctttaataggtctccagattttctggaaaaggttctttggcatttgactccattttgctgtttcatttgtcagacttctttttgtccctctttacttctccccacataattcaccagtactagtgttttgtttttcagaccaagtctcgctctgtcgcccaggctggagtgcagtggcgcgatctcagctcactgcaacctccgcctcccaggttcaagcaattctcctgcctcagcctcccgggtagctgggactacaggcgcgcgccgccacgcctggctaattttttatattttagtagagacggcgtttcaccatgttggccaggatggtctcgatctgttgacgtcgtgatccacccgcctcggcctcccaaagtgctgggattacaggcgtgagccaccccgcccggccaccagtgctattcttaagacgcctctgaggaatcccttctccctggccattgagaatccatgcatgaacccaggttttccaccttccctgagcagcttgcatagttccttcttttaagcgcctgacttcgttttgtttggtgcccgttgtacctgagaatgagccttggatagtggagcattccagctttccagatatgcagagataatacattggctatcagctacttggcttggcctattccgtgtttaaaatcttggactctttgctagtttttacagatcagaatttttcacgtattaatccagttttcctagcttctcttgaagaatttttggagatctcttcatactgagccttcattagcccaggacagtactgctgtagcagttcatatattttttcgcttcccaggcctgtgttattcacttaagttcatagcctggtccctgcagggttgtacccgagcacagctacttagatgtcctgaatgtattaccggttaaatggaggtttcaaagaacctgctgtttttggccctgtgctcttgataacagagtgtttgagggacaactttcacatttgagtttttccaaaattaaaggttgtagaagagtcacagtatctattgtcaaaaagaaaagaatttaaaaaggcagcaattgccaggatacttcatttgagcaatgatattttccagtggaaagtcacatcttaagggttaatgccccttaactgttggccgtatttgaaaacaaaccaagctaaaaacaagagacactgacatgttgtatgacggtgtggtgtggatgttgtgtttattttagtcctgagatctagttgtaacttccttgatttctgtatgtagccacggagcaccattacctgtcaccattacctgaatggctatactgcttgctttcattttggtagagtggaaaggttacctaggtttcagtgcttgaaaagatttcagaaagcagtagtacgtctggttagactagaatcagtcctctcctgggggcagtggaatataatattttctgactgctaattaaaaatacctgtgatagccgggcgtggtggcttacgcctgtaatcccagcactttgggaggccgagacgggtggatcacgaggtcagcagatggagaccatcctggctaacacggtgaaaccccgtctctactaaaaatgcaaaaaaattagccgggtgtggtggtgggcgcctgtagtcccagctactcaggaggctgaggcaggagaatggcatgaacctgggaggcggagcttgcagtgagccgagatcatgtcactgcactccagcctgggcgacagagcgagactcgtctcaaaaaaaaaaagaaaaaaacttatgatggacacttaaaaacactcactgagtggggagtggagagcaggggtcccagggtagcctgttggacatttccagggcgactttttctttttttttttttaaagtcaagtgagtatgccatatggaaaagggtgtgcgtggagaaaaagcaaggggctccagagtgtaggatgagacatacaccttttgggttaaaaaggctgaggcaggagaatggcgtgaacccgggaggcggagcttgcagtgagctgagatcatgccactgcactccagcctgggcgacagagcgagactcttgtctcaaaataaaaaacgtttacatgtacatgtatattcaacatgtacaaatataacctattcaaaagtatttactacataaataggtacttacattacctatttactgtaatagtcaaagcctatgaagtatctaacactgatgtgtaggtactcactttgcttgccactctattaggtgctttttatgttatttaatcatgaagcctggccacagggtgcttgtgcattgagtgtgggaacaagattaccatctcccttttgaggacacaggcctagagcagttaagcagcttgctggaggttcactggctagaaagtggtcagcctgggatttggacacagatttttccactcccaagtctggctgctttttacttcactgtgaggggtaaaggtaaatcagctgttttctttgttcagaaactctctccaactttgcacttttcttaaaggaaagtaatggaccagtgaaggtgtggggaagcattaaaggactgactgaaggcctgcatggattccatgttcatgagtttggagataatacagcaggtgggtgttgtgctgtgctggtgacccatacttgttcaccctagttagataaacagtagagtagcccctaaacgttaaaacccctcaacttgtttttgtttttgagaaagggtcttgctctgtcgctcaggctggagtgcagtggcgctgtgcgatcatggctgaccttagccttgacctcccaggctccattgatcctcatgccttggcccgtagctgggactacaggtacacaccaccacgcctggctaatttttgtatttttttctagaggtggggtttcatcatgttgcccaggctggtcttgaactgctgggctcaagtggtctatcctcctcgacctcccaaagtgctgggattacatgtgtgagccactgtgcctgggaaaaccctcaacttttcttttaaaaaagaggtcaactttattgtatataagcactgtgctaaaattgcaggaactgggaccatatcctgatttttgtaataatgccagcagagtacacacaagaaaagtaactgcactagattgtgaagactggggtggacctgcttctgaaggtccagtgccctttgtcttaagatttggtgtagtgtgtctttagaaaccaaaaaaagagaagaagatcaaccttaagattagccacaaaactgggctttgatacctaggtgtggaaaagaaagggaaagagttgatgttttgtcttacagcatcattgtagaagagggtgtttttttgtttgtttgttttttgagacggagtcttactctgtggcccaggctggagtgcagtggcgcgatctcggctcactgcaagctccgcctcccgggttcatgccattctcctgcctcagccccctgagtagctgggactacaggtgcccgccaccccgcctggctaattttttgtatttttagtagagacggggtttcactgtgttagccaagatggtctctctcctgacctcgtgatccgcctgtctcagcctcccaaagtgctgggattacaggcatgagccaccgcacccagccagaagagggtgttttttaaagaaggcaaataggaaataaaaacttgggctcttaacttttgtaatgatcccaggtgtttgagctgggggttgagggtgggtgcctcgagcaaaggggctgcatttatttgcataatgccatgtaagagtagctctacaccccaaacacaggcttcttagtgggaccaaagtatgatacaaactgaagatggaatgcagaggattattggtactttggaatatgcttaaaaaaaatttttttaaagtatttttaaaaaatcaggcaacccctgaaccagagtaggttcagagaaactgccaaattttattttcttaatttgggattggaagcaagttaacagaagtttatgagttaagttgcatttagtgatcttttgccatatttgagtaataatctgatttttttgtttatagatttcttcttaaattaactttattcatcttgctaatttagtttcaaatagtgatttgtaatgatcagatttgatccatttctgtaattgctgaaattcccccgagttgctttttggctttaccgcctctggtctgggaggtgattgctctgctgcttcctgtaacttgcctgcctttctccctgtgtgggactcctgcgggtgagagcgtggctgaagacagccgtgttatgaaagggcctcctgtgctgtcgaggttgtgctctgtgaatgtcatcccctggtgcacagcagcaccttctacacaggatacagttggaatgccgccccctcgagttgtgtaaggcagcagccttggcccttgcacataagatgctgttgaatattctgcctgcaccaagtaaagggcacagatagaactgcttggcatatgttgctggggagatgagttttttgtaaagtatactacgttcttaagaatttggatcataaccatgggattttaataatagaaaaactgttgaagatcagtctggtcccttatttttacagtgaagaagccaaagcccagagaagggtgttaactttacaagtgtcagacagtagttagaacttggtggggtttttttttttttttttttgagatggagtcttgctctgttgcccaggctggagtgcagtggtgcgatctcagctcactgcaacctctgcctcccaggttcaagcgattctcctgcctcagcctactaagtagctgggactataggtgcgcaccaccacgcctagctaatttttgtattttttcagtagagacagggttttgctatgctggccaggctggtctcaaactcctgacctcagatgatccagccacctcagcttcccaaagtgctggggttccaggtgttagccaccatgcctggccatagacttgtttctgttcccttctcactgtggctgtaccaaggtgttgcttatcccagaagtcgtgatgcaggtcagcactttctccatgggaagttttagcagtgtttctttttagaatgtatttgggaactttaattcataatttagcttttttttcttcttcttataaataggctgtaccagtgcaggtcctcactttaatcctctatccagaaaacacggtgggccaaaggatgaagagaggtaacaagatgcttaactcttgtaataatggcgatagctttctggagttcatatggtatactacttgtaaatatgtgctaagataattccgtgtttcccccacctttgcttttgaacttgctgactcatctaaacccctgctcccaaatgctggaatgcttttacttcctgggcttaaaggaattgacaaatggggacacttaaaacgatttggttttgtagcatttattgaatatagaactaatacaagtgccaaaggggaactaatacaggaaatgtcatgaacagtactgtcaaccactagcaaaatcaatcatcattgtgaaacataggaagcttctgtagataaaaaaaaaaattgatactgaaaactagtcgagactccatttatatgtgtatgttttctgaaagcctttcagaaaaatattaaatttaaggacaagatttttatatcagaggccttgggacatagctttgttagctatgccagtaattaacaggcataactcagtaactgagagtttaccctttggtacttctgaaatcaggtgcagccccatctttcttcccagagcattagtgtgtagacgtgaagccttgtttgaagagctgtatttagaatgcctagctacttgtttgcaaatttgtgtctactcagtcaagttttaatttagctcatgaactaccttgatgtttagtggcatcagccctaatccatctgatgctttttcattattaggcatgttggagacttgggcaatgtgactgctgacaaagatggtgtggccgatgtgtctattgaagattctgtgatctcactctcaggagaccattgcatcattggccgcacactggtggtaagttttcataaaaggatatgcataaaacttcttctaacatacagtcatgtatcttttcactttgattgttagtcgcggtttctaaagatccagataaactgtacttgcagttcaaattaggaaaagcaattttattggacaattacggtgaaaatgaattattttatctaggtcagttaagaacactgttctgctaagatgcagtaaaaagcaggttacatttgaccatattagatctgagtttggaaaacagaagtagtctttagttttaaaatggccagattttcttgccaggattgggtttctcacttgttaaacagaacattttgttaagtttaaaacctgggatggacttaagtattcatgttcattcatgttcattcaggactgcaggttatcatgacttgtttaacttgtgggaagctgttgtcccaagttatcctggggaactgcatctggttcttgcaaaacaccaagtagacaggctctcttttacctccccttgagggcattaacattcagtagtcacttccattcagttaaccctttatttttatggtttttcttgagccatagttgtaaagcagaaaaatcatttataaaggtttgttgaacaaaattcaaaatactgttgcttaaagtattaagattttttaggattataccttacttataggcccgtcattcatttggcatgaaattttgagttttattcactttcactttcctttttttccaaagcaattaaaaaaactgccaaagtaagagtgactgcggaactaaggttactgtaacttaccatggaggattaagggtagcgtgtggtggtctacaacatagttatttgggttttagtatttcatttagacagcaacacttacctaatgtttaaaggtaatgtctttgcaacaccaagaaaaagctttgagtagtagtttctacttttaaactactaaatattagtatatctctctactaggattaatgttatttttctaatattatgaggttcttaaacatcttttgggtattgttgggaggaggtagtgattacttgacagcccaaagttatcttcttaaaattttttacaggtccatgaaaaagcagatgacttgggcaaaggtggaaatgaagaaagtacaaagacaggaaacgctggaagtcgtttggcttgtggtgtaattgggatcgcccaataaacattcccttggatgtagtctgaggccccttaactcatctgttatcctgctagctgtagaaatgtatcctgataaacattaaacactgtaatcttaaaagtgtaattgtgtgactttttcagagttgctttaaagtacctgtagtgagaaactgatttatgatcacttggaagatttgtatagttttataaaactcagttaaaatgtctgtttcaatgacctgtattttgccagacttaaatcacagatgggtattaaacttgtcagaatttctttgtcattcaagcctgtgaataaaaaccctgtatggcacttattatgaggctattaaaagaatccaaattcaaactaaattagctctgatacttatttatataaacagcttcagtggaacagatttagtaatactaacagtgatagcattttattttgaaagtgttttgagaccatcaaaatgcatactttaaaacagcaggtcttttagctaaaactaacacaactctgcttagacaaataggctgtcctttgaaagctttagggaaatgttcctgcttagtcattttagcattttgattcataaagtacctcctcattttaaaaagacattatgatgtaagagagccatttgataactttttagtgagctttgaaaggcaagttacagcctcagctagctagtaagattatctacctgccagaatggcacaaattctacattcaagggtagacgctggcacaacctacttacagattagccctttaaagcaatctgtagcattagaagatggaaccaaggaaatgtttgactgtgggttctggctgttgagaaataatttacacaccgaattagtgaaatgagtcactttctcttaatgtatttatgtacctgagagaatgcttttcaatgttaacctaactcaggtttgactaaattattcaattggaaattgtagaatattatttctgataaaccagaaataagtgaaatgctgtttgttcataaatatgtactttatcaaatgtaggagagatcatttaggagaggaaaagctaaattggaagacaaatctgtagtgtttccaaagttttaaaattatggtaaacaacagtatgttcacagtaagtggttaaaacaaccattctttaaatctcagtagagaatttttaaaaagcagtatttaacacatttccctaatgtagtttgttgcctatgtggaataactcaattagagactcac

SEQ ID NO: 3 - DNA, 13001 bp, Macaca mulata
cctggaacccagagaaacttcagccttgggcaaaggccgtttggccagcatttgcactgtttatgcaaccgtttagaatatacgaattatctggaaactactactaaatacaacacgcaaaactgcaaatatgtatacttcctagaggatgataaaaaaaatgtgaattgtgttttctctgatagaggatgcattagagtctgagggtctaaataacataaataataaataagtaaataaatagatagtagtgtactccaaacgaggctggaatagcttctatcgttgtttcacgctggacttgaattaagtctgagtattttgccatgctcagtacgaaatactaggctggacgtggtggcttatgtctgtaatcccagcactttgggaggccgaggtgggcagactggcttgagctcaagagtttgaaaccagcctgggcaacatggtaaaaccccatctctacccaaaatacaaaaatcagccaggtgtggtgccacatgcctgtggtctcaggtacttgggaggctgaggcagcaggatgacttttgaacccaggaggtcgaggctgcagtgagctatgatcgtgccactgcactccagcctgggtgacagagcaataccctgtctcaaaaatcaaataaacaaccccttcgccccggactaaagtagtttgtactattttctcatttcatcaaagtttttgaaatatttcccttgaaaggtaagtcatatttatcattcctgttgtatggagacatcacaaattatttcaccattctaccctccttgagtgttgtggccttggggccaggcaaaaacgcaggagatgcctagaagccaactagttgccgttttggttatctgtggggctgtagcgttgccaaacaggaaaaatataaaaagaataccgaattctgccaaccaaataagaaactatgtgctaaggactaaaacaactgcaggggaagaaaaggtgaggccagggattgaggtgtagcgactttctatgccctcagaaaattaaaaaacaagacaaaaaaaaaaaaagaaaactacaaaagcatccatcttgggccgtcctaatttctgagtaacaaatgagatgctgtggcgaaagtcagtcataaccaatgacatttctagacaaagtgacttcagattttcaaggcgtaccttgtttacatcattttgccaatttcgcgtcctgcaaccgtcgggccacgcccccgtgaaaaaaaggctgtgtttttttccacatttcggggttctggacctttcccggctgcggggcggggggaagtctgaggcgcacgcggccccttggccccgcccccagtcatttcctgccactcgcgtcccgaggctgccgcagggggcgggctgagcgcgtgcgctgtgactggtttggggccagagtgggcggggcgcggaggtccggcctataaagtagtcgcggcgccgtggtaccgctttgcggcgtagtctcctgcagcgtttgcggtcagtctcgcaatattcggaagcaggaccgcggcgtggcctagcaagtcatggcgatgaaggccgtgtgcgtgttgaagggcgacagcccagtgcagggcaccatcaatttcgagcagaaggcaagggccggggcggaggcttgtttgcgaggccgctcccgcccgcttgtcgccccgagcacctgtgctaggagcgggtggccagccaggcctcgggaccgccctggtcccgcgcccggcctcggcccgtgccgcccggtcggtgcctttgcccccagcggtgcggtgccggctaagtgctgagtcatcgggcgggcccgggtgcggggtgtgggaccgaggccgccgcggggctgggcctgcgcgtggcgggagcgcggggagggattgccgcgggggcgggcgtgggcgtgctgccctccggggtccgtgggcggccgccgcgggctctgtcgtggtgcttggagcagctgtgctcctcccttgcttggctgtgttctcgttcctgagggtcccgcggacaccgagtggcgcagtgacaggcccggcccggggtggcgactgcgcctgggcccggctggtgtcttagcatccctctccgcgttccggcttcagcgctctgggtcagggagtctccgcttttgtacagctctaaggctaagtatggtttttatatttttaaaaggctttggtaaacaaaaatacgcaacagagaccgtttgtgtgacactttgcaggagtttgttggcctctgttctaggtcatggttgggctgcaagggcagagaaggtagccttggatagaggtccttttcctcctcctaagctccgagagccagagttttaactgaccgttttggggactttcgagggcaatgattcttaactttgggtgcacaattagcttatttgaagatcttactaaaaatacaccagagcccaacctcagaccaattacatcaaaacctgtcccagcgcaggtgattattgctgttttttaagtttccaaatgtgattttgatgtgcacctacgattgaggactgttgtttgaggacagtgggtggggtttggaatttggaaattgggaagacctgaagtttccattacacggaattggtacttagtaactcttgtcggagcatttcttaagccacattttctgtgaagtggctttaaaattgctctgccagtaggcaggttgctaagatggtcagagacaaacttctgaacgactcttgtaaaatgtagtacagaaatattttcataactattatcagtaaaattgcaaaacgtcttgcaaggaaggtgcttgtgataacactgtccccagagccttagtgaagttaccaactggtggaaaattgtctggtactcggcttaaaagtcatgagagaatatttatcatatgaatgagattcagtctttaaaggggtttacagaaaggtgagaggacaggaacagttagtctgtgcaagtgtctgaaatgtgtatgagggagatacgagtttagcttttttctttaatacgtctccagattttctggaaaaggttctttggcatttgactccattttgctatttcatttgtcagacttcgttttgtccctctttacttattcccacataattcactagtactagtgctgtgttttgtttctgagaccgagtcttgctctcttgcccaggctggagtgcagtggcgcgatctcggctcactgcaacctccgcttcctgggttcaagcaattctcctgcctcaggctcccgggtagctgggattacaggcgcgtgccaccacgcccagctaattttttgtattttagtagggaccgggtttcaccatgttggccaggatggtcacgatctcttgacctggtgatccacccgcctcggcttcccagagtggtgggattacaggcgtgagccaccgcgcccggccaccagtactagtcttaagacgcctctgtggaattccttctccctggcctttgagaatccatgcatgaacccaggtttctgtcattttccaccttccctgagcagcgagcatagttccttcttttaagcgcctgacttcgttttggttggtgccccttgtacctgagaaagagccttggatagtggagcattccagctttccagatatgcagagataataaattggctataaactacctggcgtggcctattccgtgtttaaaatcttagactcgtggctagtttttacaaatcagaatctttcacctaatagtccagttttcctagcttctcttgaagaattgttggagatctcttcatactgagccttcattagcccaggacagtactgctggagctttccaggcctgtgttactcacttgagttcacagcctggtccctgtagggttgtacctaagcacaactacttacatgttcccaatgtattacccgttaaatggaggtttgaaagaacctcctctttttggccctgtgctcttgataacacagcatatttgagggacaactttcacatttgagtttttccaaaattagaggttgtagaagagtcacagtgtctattctgaaaaagaaaagaatttttaaaaggccgcaattgccagaatccttcgtttgagcagtggtattttccagtggaaagtcatgtcttaagggttaatgccccttaactgttgtccctatttgaaaaccaagctaaaaacaagagacacaaacatgtatgacggtgtggtgtggatgatgtgtttattttagtcctgagatctactcgtaacgtccttgatttctgtatgtagccacggagcaccattacctgtcaccattgcctgaatggcgatactgcttgctttctttttggtagagtggaaaggttatctaggtttcagtgcttgaaaagatttcagaaaacagtagtacctctggttagactagaatcagtcctctcctgagggcagtgaaataggatattttctgactgctaattaaaaatacctatgatagccggacgtggtggctcacgcctgtaatcccagcagtttgggaggcggaaggggcggatcacgaggtcatgagatcgagaccatcctggctaacacggtgaaaccccgtctctgctaaaaatacaaaaaattaactgggcttggtggtggttggcgcttgtagtcccagctactcaggaggctgagggaggagaatggcatgaacctgggaggcggagcttgcagtgagccgagatcatgccactgctcttcagcctgggcgacagagctagactccatctcaaaaaaaaaaaaaaaacaaaaaaactttgatggaaacttaaaaacacacactgagtggggagtggagagcaggggtcctagggtagcctgttggacgtctccagggtgcctttttctttgttttaaagtgtgtatgctgtatggaagagtgtctatatggagaagcagcaaggggctaaagagcatatgatgagacatacaccttttgggttaaaaaggctgaggcaggagaatggcgtgaacccgggaggtggagcttgcagtgagccgagatcgcgccactgccctccagcctgggtgacagagcgagactctgtctcaaaacaaaccaaaaaggtttacgtgtacatgtatattcaacatgtacaaatatgacctattcaagtgtctactaaataggtacttatattacatatttactgtaatagtcaaaccctatgaagtatctaactctgatgtgtaggtactcactttgcttaccactctatttggtgctttttatgtttaatcacgaagcctggccacagggcgcttgtgcattgagtgtgggaacaagattaccatctcccttttgaggacacaggcctagagcagttaagcagcttgctggaggtaccctggctagaaagtggtcggcctgggatttggacacagatttttccactcccgagtctggcttctttttactttactctgaggggtaaaggtaaatcagctgttttctttgttcagaaactctctccaactttgcacttttctttgattaaaggaaagtaatggaccagtgaaggtgtggggaagcattacaggattgactgaaggcctgcatggattccatgttcatcagtttggagataatacacaaggtgggtgttgtgctgtgctggtgacccatacttgttcaacctagttagataaacagtagagtagcccctaaatgttaaaactcctcaacttggttttgtttttgagacagggtcttgctctgtcacccaggctggagtgcagtggtgctgtgcgatcatggctcaccttagcctcgacctcccaggctccagttatcctcatgccttggcctgtagctgggactacaggcatacgccaccacacctggctactttctgtatttttttctagccgtggggtttcatgttgtccaggctagtcttgaactgctgggctcaagtggtttatcctcctgcacctcccaaagtgctgggattacaggtgtgagccactgtgcctggcaaaaccctcaacttttcttttaaaaaaagaggtcaactttattgtataaacactgtgctaaaatggcagaaactaggaccatatcttggtttttgtaataatgccagcagagtatacacaagaagaaaagtaactgcactagattgtgaagactggggtggacctgcttcttaatgcccagtgccctttgtcttaagatttggtgtagtatatctttagaaaccaaaaaaaaaaaaaaagtgaagttaaaataactttgaagatcaaccttaagattagccacaaaactggtttttgtcacctaggtgtggaaaagaaagggaaagagttgatgttttttgtcttatggcatcattgtagaagaggattttttttttttttttggagacaagtcttactctgtcgcccaggctggagcgcagtggcgccatcttggctcgctgcaagctgtgcctcctgggttcacgccattctcttgcctcagcctcctgagtagctgggactacaggcgccgccaccacgcctggttaatttttttgtttttttagtagagatggggtttcactgtgttagccaagatggtcttgatctcctgacctcgtgatccacccatctcggcctcccaaagtgctgggattacaggcatgagccactgtgcccagccagaagaaagtgttttttaaagaaggcaataggaaataacttgggttcttaacttttgtaatgatcccaggtgtttgagctgggggttgagggtgggtgcctcaagcgaaggggctgcattcgtttgcataatgtcatgtaagagtagctccacaccgcaaacacaggctccttagtgggacaaaagtaggatacaacctggagatggaatgcagaggatcactggtactttggaatatgcttaaaaaatttttttagtatttttaaaaaatcaggcagcccctgaacctgagtaggttcagagaaactgccaagttttatattcttaatttgggattggaagcaagttaacaaaagtttatgagttaaattgcatttagtggtcttttgccatatttgagttatctgaattttttgtttataggtttcttcttaaattaacttcattcatcttgctaatttagtttcaaatagtgatttgtagtgatcagatttgatccatttctgtaattgctgaaattccccaagttgctttttggcttcccgcctctggtttgggaggtgattgcgctgctgcttcctgtaacttgcctgcctttctccccgtgtgggactcctgggggtgagaggacttgttacgaaggcagccgtgttacgaaagggcctcctgtgccgtcgaggttgtgctctgtgaatgtcatcccctggcccacaggagcaccttctacacagggtacagtcggaatgccgccccctggagttgtgtaaggcagcagccttggcccttgcacataagatgctgttgaatattctgcctgcaccaagtaaagggcacaggtagaactgcttggcagtatgttgctggggagatgagttttttgtagttaaagtgtactacattcttacaaatttggatcttaaccatgggattttaatgatagaaaaactgttgaagatgagtctggtcccttattgtacagtgaagcagcagaagccccgaggaagggtgttgactttacgagtgtcagatagtagttagaacttgcttttttttttgagacgcagccttgctctgttgcctaggctggagtacagtggtgcaatctcagcttactgcaatctctgcctcccaggttcaagcgattctcctgcctctgcctatcaggtagctgggactacacgtgcacaccaccatgcctagctaatttttgtatttttcagtagagacagggtttcgccatgttggccaggctggtctcaaactcctgacctcagatgattcacccacctcagcttcccaaagtgctgggattccaggtgttagccaccatgcccggccatagacttgtttctgttcccttctcaccatgcctggaccaaggtgttgcttatcccagaagttgtgatgcaggtccctgctctctccatgggaagttttagcaatgtttctttttagaatgtatttgggaactttaattcataatttagctttttttttttttctttttcttgtaaataggctgtaccagtgcaggtcctcactttaatcctctatccagacaacacggtgggccaaaggatgaagagaggtaacaagatgcttaactcttgtaataatggcgatagctttctggagttcatatggtatactacttgtaaatatgtgctaagataattccgtgttctcccccacctttgtttttgaacttgctgactcatctaaacccctgctcccaaatgctggaatgcttttacttcctgggcttaaaggaattgacaaatggggacacttaaaacgatttggttttgtagcatttattgaatatagaactaatacaggtgccaaaggggaacttatacaggaaatgtcatgagtaacagtactgtcaaccactagcagaatcaatcatcgtgaaacataggaagcgtctgtagataaaaaaaaaattgatattgaaaactagtcgagactccatttgtatgtgtatgttttctgaaagcctttcaggaaaatactaaatctaaggacaagatttttatatcagaggcctcgggacatagctttgttagctatgccaataattaacaggcataactcagtaactgagagtctaccctttggtacttctgaaatgaggtgcacccccatctttcttcccagagcatgagtttgtagacttgaagccttgtttgaagagctgtgtttagaatgcccagctacttgtttgcaaatttgtgtttgctcagtcaagttttaatttagctcatgaactaccttgatgttcagtggagtcagccctaatccatctgatgcttttccattattaggcatgttggagacctgggcaatgtgactgctggcaaagatggtgtggccaaggtgtctttcgaagattctgtgatctcgctctcaggagaccattccatcattggccgcacattggtggtgagttttcataaaaggatctacataaaacttcgtctaacatacagtcatgtatctcttcactttatgattgttagtcgtggtttctaaagatccagataaattatacttgcagttcaaattaggaaaagcaattttattggacaattatggtgaaaatcaattattttatctgggtcagtcaagaacactgttctgctaagatgcagtagaaagcaggttacatttgaccatattagatctgagtttggaaaacagagtagtctttagttttaaaatggccagattttcttgccaggattgggtttctcacttgtgaaacagaacattttgttaagtttaaaacctgggatggacttcagtattcatgttcatccaggactgcaggttatcatgacttgtttaacttgtgggaagctgttgccccaagttattctggggaatgcatctggttcatgcaaaacaccaggtagactggctctcttttacctccctttgagggcattaacattcattagtcacttccactcagttaacccttttatttttaaggttttcttgagccatagttgtaaagcagaaaaattgtttacaaaggtttgttgaacaaaattcaaaatactgttgctaaagtattaaggttttttaggattatgtcttatttataggcctgtcattcatttggtatgaaattttgagcgttactcactttcactttcctttttttccaaagcaattaaattgccaaagagtgactgctgaactacagttactgtaacttatcatggaggactaagggtagtgtgtggtggtctacaacatagttatttgggtttttagtatttcatttagagatagcaacacttacctaatgtttaaaggtaatgtctttgcaacaccaagaaaaagctttgaatagtagtttttacttttaaactactaagtattagtatatctactaggattaatgttatttttctaatattatgaggttcttaaactatcttttgggtattgttgggaggaggtagtgattacttgacagcccaaagttatcttcttacaattttttacaggtccatgaaaaagcagatgacttgggcaaaggtggaaatgaagaaagtaaaaagacaggaaacgctggaggtcgtctggcttgtggtgtaattgggatcgcccaataaacattcccttggatgtagtctgaggcccattaactcatctgttatcctgctagctgtagaaatgtatcttgataaacattaaacactgtaatcttaagagtgtaattgtgtgacgtttgcttagtacctgtaatgagaaactggttgatgatcacttggaagatttgtatagttttataaaactcaattaaaatgtctgtttcaatgacctgtattttgccagacttaatcacagatgggtattaaacttgtcagaatttcttcaattctcattcaagcctgtgaataaaaaccctgtatggcactcattttgagtctattaaaagaatccaagttcaaactaaattagctctgatacttatttatataaacagcttcagtggaacagatttagtaatgctaacagtgatagcattttactttgaaagtgttttgagatcatcaaaatgcatacttttaaaacagcaggtcttttagctaatacgaacacaactctgcttagacaacaggctgtcctttgaaagctttagggaaatgttcttgcttagtcattttagcattttgattcataaagtacctcattttaaaaagacgttatcgtgtaagagagccatttgataacttagtgagtttaaaaggcaagttacagcctcagctagctaataagattatctacctgccagaatggcacaaattgtacattcaagggtggacgttggcacaacctacttaacagattagccctttaaagaaatctatagcattggaagatagaaccaaggaaatgtttgactgtgggttctggctgtttattaatttacacaccgaattagtgaaatgagtcactttcaatgtatttacgtacctgagagagagtgcttttaaatgttattgactattcaattggaaattgtaaattgtagaatatttctgataaaccatgaataagtgacaatctgttcataaatacgtactttatcaaatgtaggagaggaaaagctaaattgggaagacaaatctgtagtgtttccaaagttttaaaattatgttaaagaacaatatgcttacagtaagtggttaaaaccaccattctttaaatctcggtaatgtttaaaaaacactatttaacccatttccctgatgtagtttgttgcctatgtggaattagagactcacgcctttcaaacttcaaatataatcatgctaccagttaggagtagtcatttcatgtgcatataggatgctcttaagttggaaatacaggctgtaagtccttcaagtctggatgttgagtaatcacgttttcttccagaagccatttgttaggacttttttttgggccagtgtaaaattaaggacaagttttataatttaaatttacagatacaacaattttctctcattttctaaaggcaggaatataaggacattgccctagatatattctccccatcaaaccaaaggccttgctgctgagtattatttaaaaaccagagtaataaagcagctttgcctgaggatgacggcaaagacaaagttaactgctaagcatactgaaaccaagagtttaaaaaagtaattcaaaacaacttgaaggccataaatatttggatagtgtgacatcaggtcttggcactggatttcctgcaatttcagataaaggcttgacttggctttggatgtcttcatgtaattcttggataacctacaacaatttttcctagttaacccaccaactttaagcaaaagaaaaaaagtgtatgtgggggaaaagttcagtttacctctgcccagcaggggaattaaaaaactggtaaagaaaggcaataggcaaggcttatataaggaaacaataataggttgcactgaagtcctcaaacacaacaaaaagcttttagattgcaaatgttaaccttgattcttttacccttttgaagaattcagtgggatggttggaaaaaaaaaaacaacacacacacacatgcaaccttctaacgtaatacccacgcagtcagataatttatagtacaacatgtaacactggaattaacttttcccccagcaaaatcttacaaattaattagggcaacatataccacaaagccaatggggaaaaaaaaaaacctcgattgaattgcaaacacagcttttcaattgacattaaaacaactaacctttaccttatgactgaaacactaaaattcaaaagtattacatatgaaagtgagaataactacataaaatgtctattttcatcaaataagtctaatttagactccaatacagtattaacagctcaaactttgatggtgaacaatccttttccaccttaatgcagtgtaggaagaatagcacacattaaagtttgttacgaaaatagagtttattaaaaacatccctattgttttgaggagctttcaccgttaccttgtcttaaattaaaaaaaaaaaaaaatagagagcacttctaattacgatttgtaaactttttaaagtcaaaacttttaaaaagttacagcaaaaagggtaatatttattcatattttcagtattttttgttattttgtggctatttttaaatagaagggaagcaatcaaattgcttacagttccccaccagctggcgcggggctgcagtacagcgggagcggatataatacagcatctgtacacctcaa

SEQ ID NO: 4 - skipped

SEQ ID NO: 5 - DNA, 25 bp, Artificial sequence
  Primer
aggagaaaaacaaagaacaccagaa

SEQ ID NO: 6 - DNA, 25 bp, Artificial sequence
  Primer
caattagggcaactcagaaatagct

SEQ ID NO: 7 - DNA, 22 bp, Artificial sequence
  Probe
ccaactggtcccccagccaaga

SEQ ID NO: 8 - DNA, 20 bp, Artificial sequence
  Primer
gaaaccagcctggacaccaa

SEQ ID NO: 9 - DNA, 24 bp, Artificial sequence
  Primer
tccacagtctttaccacgatgttc

SEQ ID NO: 10 - DNA, 25 bp, Artificial sequence
  Probe
tccgtgtcagaaggccacctcaaga

SEQ ID NO: 11 - DNA, 22 bp, Artificial sequence
  Primer
ctctcaggagaccattgcatca

SEQ ID NO: 12 - DNA, 27 bp, Artificial sequence
  Primer
tcctgtctttgtactttcttcatttcc

SEQ ID NO: 13 - DNA, 24 bp, Artificial sequence
  Probe
ccgcacactggtggtccatgaaaa

SEQ ID NO: 14 - DNA, 20 bp, Artificial sequence
  Primer
cgtggcctagcgagttatgg

SEQ ID NO: 15 - DNA, 20 bp, Artificial sequence
  Primer
gaaattgatgatgccctgca

SEQ ID NO: 16 - DNA, 21 bp, Artificial sequence
  Probe
acgaaggccgtgtgcgtgctg

SEQ ID NO: 17 - DNA, 26 bp, Artificial sequence
  Primer
tggagataatacacaaggctgtacca

SEQ ID NO: 18 - DNA, 23 bp, Artificial sequence
  Primer
caacatgcctctcttcatccttt

SEQ ID NO: 19 - DNA, 27 bp, Artificial sequence
  Probe
atcctctatccagacaacacggtgggc

SEQ ID NO: 20 - skipped

SEQ ID NO: 21 - DNA, 20 bp, Artificial sequence
  Synthetic oligonucleotide
ccgtcgcccttcagcacgca

SEQ ID NO: 22 - DNA, 20 bp, Artificial sequence
  Synthetic oligonucleotide
cactggtccattactttcct

SEQ ID NO: 23 - DNA, 20 bp, Artificial sequence
  Synthetic oligonucleotide
acaccttcactggtccatta

SEQ ID NO: 24 - DNA, 20 bp, Artificial sequence
  Synthetic oligonucleotide
ccacaccttcactggtccat

SEQ ID NO: 25 - DNA, 20 bp, Artificial sequence
  Synthetic oligonucleotide
caacatgcctctcttcatcc

SEQ ID NO: 26 - DNA, 20 bp, Artificial sequence
  Synthetic oligonucleotide
ccaacatgcctctcttcatc

SEQ ID NO: 27 - DNA, 20 bp, Artificial sequence
  Synthetic oligonucleotide
tccaacatgcctctcttcat

SEQ ID NO: 28 - DNA, 20 bp, Artificial sequence
  Synthetic oligonucleotide
ctccaacatgcctctcttca

SEQ ID NO: 29 - DNA, 20 bp, Artificial sequence
  Synthetic oligonucleotide
tctccaacatgcctctcttc

SEQ ID NO: 30 - DNA, 20 bp, Artificial sequence
  Synthetic oligonucleotide
gtctccaacatgcctctctt

SEQ ID NO: 31 - DNA, 20 bp, Artificial sequence
  Synthetic oligonucleotide
cacctttgcccaagtcatct

SEQ ID NO: 32 - DNA, 20 bp, Artificial sequence
  Synthetic oligonucleotide
ccacctttgcccaagtcatc

SEQ ID NO: 33 - DNA, 20 bp, Artificial sequence
  Synthetic oligonucleotide
tccacctttgcccaagtcat

SEQ ID NO: 34 - DNA, 20 bp, Artificial sequence
  Synthetic oligonucleotide
ttccacctttgcccaagtca

SEQ ID NO: 35 - DNA, 20 bp, Artificial sequence
  Synthetic oligonucleotide
tttccacctttgcccaagtc

SEQ ID NO: 36 - DNA, 20 bp, Artificial sequence
  Synthetic oligonucleotide
atttccacctttgcccaagt

SEQ ID NO: 37 - DNA, 20 bp, Artificial sequence
  Synthetic oligonucleotide
catttccacctttgcccaag

SEQ ID NO: 38 - DNA, 20 bp, Artificial sequence
  Synthetic oligonucleotide
tcatttccacctttgcccaa

SEQ ID NO: 39 - DNA, 20 bp, Artificial sequence
  Synthetic oligonucleotide
ttcatttccacctttgccca

SEQ ID NO: 40 - DNA, 20 bp, Artificial sequence
  Synthetic oligonucleotide
cttcatttccacctttgccc

SEQ ID NO: 41 - DNA, 20 bp, Artificial sequence
  Synthetic oligonucleotide
tcttcatttccacctttgcc

SEQ ID NO: 42 - DNA, 20 bp, Artificial sequence
  Synthetic oligonucleotide
ttcttcatttccacctttgc

SEQ ID NO: 43 - DNA, 20 bp, Artificial sequence
  Synthetic oligonucleotide
tttcttcatttccacctttg

SEQ ID NO: 44 - DNA, 20 bp, Artificial sequence
  Synthetic oligonucleotide
ctttcttcatttccaccttt

SEQ ID NO: 45 - DNA, 20 bp, Artificial sequence
  Synthetic oligonucleotide
actttcttcatttccacctt

SEQ ID NO: 46 - DNA, 20 bp, Artificial sequence
  Synthetic oligonucleotide
tactttcttcatttccacct

SEQ ID NO: 47 - DNA, 20 bp, Artificial sequence
  Synthetic oligonucleotide
ggcgatcccaattacaccac

SEQ ID NO: 48 - DNA, 20 bp, Artificial sequence
  Synthetic oligonucleotide
ggaatgtttattgggcgatc

SEQ ID NO: 49 - DNA, 20 bp, Artificial sequence
  Synthetic oligonucleotide
cctcagactacatccaaggg

SEQ ID NO: 50 - DNA, 20 bp, Artificial sequence
  Synthetic oligonucleotide
atacaaatcttccaagtgat

SEQ ID NO: 51 - DNA, 20 bp, Artificial sequence
  Synthetic oligonucleotide
tgagttttataaaactatac

SEQ ID NO: 52 - DNA, 20 bp, Artificial sequence
  Synthetic oligonucleotide
tcattgaaacagacatttta

SEQ ID NO: 53 - DNA, 20 bp, Artificial sequence
  Synthetic oligonucleotide
atacaggtcattgaaacaga

SEQ ID NO: 54 - DNA, 20 bp, Artificial sequence
  Synthetic oligonucleotide
gtcgcccttcagcacgcaca

SEQ ID NO: 55 - DNA, 20 bp, Artificial sequence
  Synthetic oligonucleotide
tttaatacccatctgtgatt

SEQ ID NO: 56 - DNA, 20 bp, Artificial sequence
  Synthetic oligonucleotide
agtttaatacccatctgtga

SEQ ID NO: 57 - DNA, 20 bp, Artificial sequence
  Synthetic oligonucleotide
ggtttttattcacaggcttg

SEQ ID NO: 58 - DNA, 20 bp, Artificial sequence
  Synthetic oligonucleotide
agggtttttattcacaggct

SEQ ID NO: 59 - DNA, 20 bp, Artificial sequence
  Synthetic oligonucleotide
atacagggtttttattcaca

SEQ ID NO: 60 - DNA, 20 bp, Artificial sequence
  Synthetic oligonucleotide
ccatacagggtttttattca

SEQ ID NO: 61 - DNA, 20 bp, Artificial sequence
  Synthetic oligonucleotide
acgctgcaggagactacgac

SEQ ID NO: 62 - DNA, 20 bp, Artificial sequence
  Synthetic oligonucleotide
cgaggactgcaacggaaacc

SEQ ID NO: 63 - DNA, 20 bp, Artificial sequence
  Synthetic oligonucleotide
taggccacgccgaggtcctg

SEQ ID NO: 64 - DNA, 20 bp, Artificial sequence
  Synthetic oligonucleotide
ttcagcacgcacacggcctt

SEQ ID NO: 65 - DNA, 20 bp, Artificial sequence
  Synthetic oligonucleotide
ccttcagcacgcacacggcc

SEQ ID NO: 66 - DNA, 20 bp, Artificial sequence
  Synthetic oligonucleotide
gcccttcagcacgcacacgg

SEQ ID NO: 67 - DNA, 20 bp, Artificial sequence
  Synthetic oligonucleotide
tcgcccttcagcacgcacac

SEQ ID NO: 68 - DNA, 20 bp, Artificial sequence
  Synthetic oligonucleotide
cgtcgcccttcagcacgcac

SEQ ID NO: 69 - DNA, 20 bp, Artificial sequence
  Synthetic oligonucleotide
gccctgcactgggccgtcgc

SEQ ID NO: 70 - DNA, 20 bp, Artificial sequence
  Synthetic oligonucleotide
aattgatgatgccctgcact

SEQ ID NO: 71 - DNA, 20 bp, Artificial sequence
  Synthetic oligonucleotide
agtcctttaatgcttcccca

SEQ ID NO: 72 - DNA, 20 bp, Artificial sequence
  Synthetic oligonucleotide
aggccttcagtcagtccttt

SEQ ID NO: 73 - DNA, 20 bp, Artificial sequence
  Synthetic oligonucleotide
gctgtattatctccaaactc

SEQ ID NO: 74 - DNA, 20 bp, Artificial sequence
  Synthetic oligonucleotide
tgcccaagtctccaacatgc

SEQ ID NO: 75 - DNA, 20 bp, Artificial sequence
  Synthetic oligonucleotide
acacatcggccacaccatct

SEQ ID NO: 76 - DNA, 20 bp, Artificial sequence
  Synthetic oligonucleotide
tctcctgagagtgagatcac

SEQ ID NO: 77 - DNA, 20 bp, Artificial sequence
  Synthetic oligonucleotide
accaccagtgtgcggccaat

SEQ ID NO: 78 - DNA, 20 bp, Artificial sequence
  Synthetic oligonucleotide
tcatggaccaccagtgtgcg

SEQ ID NO: 79 - DNA, 20 bp, Artificial sequence
  Synthetic oligonucleotide
gtactttcttcatttccacc

SEQ ID NO: 80 - DNA, 20 bp, Artificial sequence
  Synthetic oligonucleotide
ttgtactttcttcatttcca

SEQ ID NO: 81 - DNA, 20 bp, Artificial sequence
  Synthetic oligonucleotide
ctttgtactttcttcatttc

SEQ ID NO: 82 - DNA, 20 bp, Artificial sequence
  Synthetic oligonucleotide
gataacagatgagttaaggg

SEQ ID NO: 83 - DNA, 20 bp, Artificial sequence
  Synthetic oligonucleotide
cacaattacacttttaagat

SEQ ID NO: 84 - DNA, 20 bp, Artificial sequence
  Synthetic oligonucleotide
aatcagtttctcactacagg

SEQ ID NO: 85 - DNA, 20 bp, Artificial sequence
  Synthetic oligonucleotide
cataaatcagtttctcacta

SEQ ID NO: 86 - DNA, 20 bp, Artificial sequence
  Synthetic oligonucleotide
aactgagttttataaaacta

SEQ ID NO: 87 - DNA, 20 bp, Artificial sequence
  Synthetic oligonucleotide
ccatctgtgatttaagtctg

SEQ ID NO: 88 - DNA, 20 bp, Artificial sequence
  Synthetic oligonucleotide
aagtgccatacagggttttt

SEQ ID NO: 89 - DNA, 20 bp, Artificial sequence
  Synthetic oligonucleotide
taataagtgccatacagggt

SEQ ID NO: 90 - DNA, 20 bp, Artificial sequence
  Synthetic oligonucleotide
ctcataataagtgccataca

SEQ ID NO: 91 - DNA, 20 bp, Artificial sequence
  Synthetic oligonucleotide
gcctcataataagtgccata

SEQ ID NO: 92 - DNA, 20 bp, Artificial sequence
  Synthetic oligonucleotide
ttttaatagcctcataataa

SEQ ID NO: 93 - DNA, 20 bp, Artificial sequence
  Synthetic oligonucleotide
ggattcttttaatagcctca

SEQ ID NO: 94 - DNA, 20 bp, Artificial sequence
  Synthetic oligonucleotide
ctcactacaggtactttaaa

SEQ ID NO: 95 - DNA, 20 bp, Artificial sequence
  Synthetic oligonucleotide
aatcttccaagtgatcataa

SEQ ID NO: 96 - DNA, 20 bp, Artificial sequence
  Synthetic oligonucleotide
attgaaacagacattttaac

SEQ ID NO: 97 - DNA, 20 bp, Artificial sequence
  Synthetic oligonucleotide
caaagaaattctgacaagtt

SEQ ID NO: 98 - DNA, 20 bp, Artificial sequence
  Synthetic oligonucleotide
acaggcttgaatgacaaaga

SEQ ID NO: 99 - DNA, 20 bp, Artificial sequence
  Synthetic oligonucleotide
tcataataagtgccatacag

SEQ ID NO: 100 - DNA, 20 bp, Artificial sequence
  Synthetic oligonucleotide
caggccttcagtcagtcctt

SEQ ID NO: 101 - DNA, 20 bp, Artificial sequence
  Synthetic oligonucleotide
cacattgcccaagtctccaa

SEQ ID NO: 102 - DNA, 20 bp, Artificial sequence
  Synthetic oligonucleotide
tcggccacaccatctttgtc

SEQ ID NO: 103 - DNA, 20 bp, Artificial sequence
  Synthetic oligonucleotide
catcggccacaccatctttg

SEQ ID NO: 104 - DNA, 20 bp, Artificial sequence
  Synthetic oligonucleotide
tagacacatcggccacacca

SEQ ID NO: 105 - DNA, 20 bp, Artificial sequence
  Synthetic oligonucleotide
ctcctgagagtgagatcaca

SEQ ID NO: 106 - DNA, 20 bp, Artificial sequence
  Synthetic oligonucleotide
catggaccaccagtgtgcgg

SEQ ID NO: 107 - DNA, 20 bp, Artificial sequence
  Synthetic oligonucleotide
taggccagacctccgcgcct

SEQ ID NO: 108 - DNA, 20 bp, Artificial sequence
  Synthetic oligonucleotide
actttataggccagacctcc

SEQ ID NO: 109 - DNA, 20 bp, Artificial sequence
  Synthetic oligonucleotide
gacgcaaaccagcaccccgt

SEQ ID NO: 110 - DNA, 20 bp, Artificial sequence
  Synthetic oligonucleotide
ggttccgaggactgcaacgg

SEQ ID NO: 111 - DNA, 20 bp, Artificial sequence
  Synthetic oligonucleotide
tcctggttccgaggactgca

SEQ ID NO: 112 - DNA, 20 bp, Artificial sequence
  Synthetic oligonucleotide
gaggtcctggttccgaggac

SEQ ID NO: 113 - DNA, 20 bp, Artificial sequence
  Synthetic oligonucleotide
gtcgccataactcgctaggc

SEQ ID NO: 114 - DNA, 20 bp, Artificial sequence
  Synthetic oligonucleotide
tcagcacgcacacggccttc

SEQ ID NO: 115 - DNA, 20 bp, Artificial sequence
  Synthetic oligonucleotide
cttcagcacgcacacggcct

SEQ ID NO: 116 - DNA, 20 bp, Artificial sequence
  Synthetic oligonucleotide
cccttcagcacgcacacggc

SEQ ID NO: 117 - DNA, 20 bp, Artificial sequence
  Synthetic oligonucleotide
cgcccttcagcacgcacacg

SEQ ID NO: 118 - DNA, 20 bp, Artificial sequence
  Synthetic oligonucleotide
cgcccactctggccccaaac

SEQ ID NO: 119 - DNA, 20 bp, Artificial sequence
  Synthetic oligonucleotide
ccgcgactactttataggcc

SEQ ID NO: 120 - DNA, 20 bp, Artificial sequence
  Synthetic oligonucleotide
ccttctgctcgaaattgatg

SEQ ID NO: 121 - DNA, 20 bp, Artificial sequence
  Synthetic oligonucleotide
tccttctgctcgaaattgat

SEQ ID NO: 122 - DNA, 20 bp, Artificial sequence
  Synthetic oligonucleotide
ttccttctgctcgaaattga

SEQ ID NO: 123 - DNA, 20 bp, Artificial sequence
  Synthetic oligonucleotide
tttccttctgctcgaaattg

SEQ ID NO: 124 - DNA, 20 bp, Artificial sequence
  Synthetic oligonucleotide
ctttccttctgctcgaaatt

SEQ ID NO: 125 - DNA, 20 bp, Artificial sequence
  Synthetic oligonucleotide
actttccttctgctcgaaat

SEQ ID NO: 126 - DNA, 20 bp, Artificial sequence
  Synthetic oligonucleotide
tactttccttctgctcgaaa

SEQ ID NO: 127 - DNA, 20 bp, Artificial sequence
  Synthetic oligonucleotide
ttactttccttctgctcgaa

SEQ ID NO: 128 - DNA, 20 bp, Artificial sequence
  Synthetic oligonucleotide
attactttccttctgctcga

SEQ ID NO: 129 - DNA, 20 bp, Artificial sequence
  Synthetic oligonucleotide
cattactttccttctgctcg

SEQ ID NO: 130 - DNA, 20 bp, Artificial sequence
  Synthetic oligonucleotide
ccattactttccttctgctc

SEQ ID NO: 131 - DNA, 20 bp, Artificial sequence
  Synthetic oligonucleotide
tccattactttccttctgct

SEQ ID NO: 132 - DNA, 20 bp, Artificial sequence
  Synthetic oligonucleotide
gtccattactttccttctgc

SEQ ID NO: 133 - DNA, 20 bp, Artificial sequence
  Synthetic oligonucleotide
ggtccattactttccttctg

SEQ ID NO: 134 - DNA, 20 bp, Artificial sequence
  Synthetic oligonucleotide
tggtccattactttccttct

SEQ ID NO: 135 - DNA, 20 bp, Artificial sequence
  Synthetic oligonucleotide
ctggtccattactttccttc

SEQ ID NO: 136 - DNA, 20 bp, Artificial sequence
  Synthetic oligonucleotide
actggtccattactttcctt

SEQ ID NO: 137 - DNA, 20 bp, Artificial sequence
  Synthetic oligonucleotide
tcactggtccattactttcc

SEQ ID NO: 138 - DNA, 20 bp, Artificial sequence
  Synthetic oligonucleotide
ttcactggtccattactttc

SEQ ID NO: 139 - DNA, 20 bp, Artificial sequence
  Synthetic oligonucleotide
cttcactggtccattacttt

SEQ ID NO: 140 - DNA, 20 bp, Artificial sequence
  Synthetic oligonucleotide
ccttcactggtccattactt

SEQ ID NO: 141 - DNA, 20 bp, Artificial sequence
  Synthetic oligonucleotide
accttcactggtccattact

SEQ ID NO: 142 - DNA, 20 bp, Artificial sequence
  Synthetic oligonucleotide
caccttcactggtccattac

SEQ ID NO: 143 - DNA, 20 bp, Artificial sequence
  Synthetic oligonucleotide
cacaccttcactggtccatt

SEQ ID NO: 144 - DNA, 20 bp, Artificial sequence
  Synthetic oligonucleotide
cccacaccttcactggtcca

SEQ ID NO: 145 - DNA, 20 bp, Artificial sequence
  Synthetic oligonucleotide
ccccacaccttcactggtcc

SEQ ID NO: 146 - DNA, 20 bp, Artificial sequence
  Synthetic oligonucleotide
tccccacaccttcactggtc

SEQ ID NO: 147 - DNA, 20 bp, Artificial sequence
  Synthetic oligonucleotide
ttccccacaccttcactggt

SEQ ID NO: 148 - DNA, 20 bp, Artificial sequence
  Synthetic oligonucleotide
cttccccacaccttcactgg

SEQ ID NO: 149 - DNA, 20 bp, Artificial sequence
  Synthetic oligonucleotide
gcttccccacaccttcactg

SEQ ID NO: 150 - DNA, 20 bp, Artificial sequence
  Synthetic oligonucleotide
tgcttccccacaccttcact

SEQ ID NO: 151 - DNA, 20 bp, Artificial sequence
  Synthetic oligonucleotide
atgcttccccacaccttcac

SEQ ID NO: 152 - DNA, 20 bp, Artificial sequence
  Synthetic oligonucleotide
aatgcttccccacaccttca

SEQ ID NO: 153 - DNA, 20 bp, Artificial sequence
  Synthetic oligonucleotide
taatgcttccccacaccttc

SEQ ID NO: 154 - DNA, 20 bp, Artificial sequence
  Synthetic oligonucleotide
tccatgcaggccttcagtca

SEQ ID NO: 155 - DNA, 20 bp, Artificial sequence
  Synthetic oligonucleotide
atccatgcaggccttcagtc

SEQ ID NO: 156 - DNA, 20 bp, Artificial sequence
  Synthetic oligonucleotide
aatccatgcaggccttcagt

SEQ ID NO: 157 - DNA, 20 bp, Artificial sequence
  Synthetic oligonucleotide
gaatccatgcaggccttcag

SEQ ID NO: 158 - DNA, 20 bp, Artificial sequence
  Synthetic oligonucleotide
ggaatccatgcaggccttca

SEQ ID NO: 159 - DNA, 20 bp, Artificial sequence
  Synthetic oligonucleotide
tggaatccatgcaggccttc

SEQ ID NO: 160 - DNA, 20 bp, Artificial sequence
  Synthetic oligonucleotide
atggaatccatgcaggcctt

SEQ ID NO: 161 - DNA, 20 bp, Artificial sequence
  Synthetic oligonucleotide
catggaatccatgcaggcct

SEQ ID NO: 162 - DNA, 20 bp, Artificial sequence
  Synthetic oligonucleotide
acatggaatccatgcaggcc

SEQ ID NO: 163 - DNA, 20 bp, Artificial sequence
  Synthetic oligonucleotide
aacatggaatccatgcaggc

SEQ ID NO: 164 - DNA, 20 bp, Artificial sequence
  Synthetic oligonucleotide
gaacatggaatccatgcagg

SEQ ID NO: 165 - DNA, 20 bp, Artificial sequence
  Synthetic oligonucleotide
tgaacatggaatccatgcag

SEQ ID NO: 166 - DNA, 20 bp, Artificial sequence
  Synthetic oligonucleotide
atgaacatggaatccatgca

SEQ ID NO: 167 - DNA, 20 bp, Artificial sequence
  Synthetic oligonucleotide
gacctgcactggtacagcct

SEQ ID NO: 168 - DNA, 20 bp, Artificial sequence
  Synthetic oligonucleotide
ggacctgcactggtacagcc

SEQ ID NO: 169 - DNA, 20 bp, Artificial sequence
  Synthetic oligonucleotide
aggacctgcactggtacagc

SEQ ID NO: 170 - DNA, 20 bp, Artificial sequence
  Synthetic oligonucleotide
gaggacctgcactggtacag

SEQ ID NO: 171 - DNA, 20 bp, Artificial sequence
  Synthetic oligonucleotide
tgaggacctgcactggtaca

SEQ ID NO: 172 - DNA, 20 bp, Artificial sequence
  Synthetic oligonucleotide
gtgaggacctgcactggtac

SEQ ID NO: 173 - DNA, 20 bp, Artificial sequence
  Synthetic oligonucleotide
agtgaggacctgcactggta

SEQ ID NO: 174 - DNA, 20 bp, Artificial sequence
  Synthetic oligonucleotide
aagtgaggacctgcactggt

SEQ ID NO: 175 - DNA, 20 bp, Artificial sequence
  Synthetic oligonucleotide
aaagtgaggacctgcactgg

SEQ ID NO: 176 - DNA, 20 bp, Artificial sequence
  Synthetic oligonucleotide
taaagtgaggacctgcactg

SEQ ID NO: 177 - DNA, 20 bp, Artificial sequence
  Synthetic oligonucleotide
ttaaagtgaggacctgcact

SEQ ID NO: 178 - DNA, 20 bp, Artificial sequence
  Synthetic oligonucleotide
attaaagtgaggacctgcac

SEQ ID NO: 179 - DNA, 20 bp, Artificial sequence
  Synthetic oligonucleotide
gattaaagtgaggacctgca

SEQ ID NO: 180 - DNA, 20 bp, Artificial sequence
  Synthetic oligonucleotide
ggattaaagtgaggacctgc

SEQ ID NO: 181 - DNA, 20 bp, Artificial sequence
  Synthetic oligonucleotide
aggattaaagtgaggacctg

SEQ ID NO: 182 - DNA, 20 bp, Artificial sequence
  Synthetic oligonucleotide
gaggattaaagtgaggacct

SEQ ID NO: 183 - DNA, 20 bp, Artificial sequence
  Synthetic oligonucleotide
agaggattaaagtgaggacc

SEQ ID NO: 184 - DNA, 20 bp, Artificial sequence
  Synthetic oligonucleotide
tagaggattaaagtgaggac

SEQ ID NO: 185 - DNA, 20 bp, Artificial sequence
  Synthetic oligonucleotide
atagaggattaaagtgagga

SEQ ID NO: 186 - DNA, 20 bp, Artificial sequence
  Synthetic oligonucleotide
gatagaggattaaagtgagg

SEQ ID NO: 187 - DNA, 20 bp, Artificial sequence
  Synthetic oligonucleotide
ggatagaggattaaagtgag

SEQ ID NO: 188 - DNA, 20 bp, Artificial sequence
  Synthetic oligonucleotide
tggatagaggattaaagtga

SEQ ID NO: 189 - DNA, 20 bp, Artificial sequence
  Synthetic oligonucleotide
ctggatagaggattaaagtg

SEQ ID NO: 190 - DNA, 20 bp, Artificial sequence
  Synthetic oligonucleotide
tctggatagaggattaaagt

SEQ ID NO: 191 - DNA, 20 bp, Artificial sequence
  Synthetic oligonucleotide
atcctttggcccaccgtgtt

SEQ ID NO: 192 - DNA, 20 bp, Artificial sequence
  Synthetic oligonucleotide
catcctttggcccaccgtgt

SEQ ID NO: 193 - DNA, 20 bp, Artificial sequence
  Synthetic oligonucleotide
tcatcctttggcccaccgtg

SEQ ID NO: 194 - DNA, 20 bp, Artificial sequence
  Synthetic oligonucleotide
ttcatcctttggcccaccgt

SEQ ID NO: 195 - DNA, 20 bp, Artificial sequence
  Synthetic oligonucleotide
cttcatcctttggcccaccg

SEQ ID NO: 196 - DNA, 20 bp, Artificial sequence
  Synthetic oligonucleotide
tcttcatcctttggcccacc

SEQ ID NO: 197 - DNA, 20 bp, Artificial sequence
  Synthetic oligonucleotide
ctcttcatcctttggcccac

SEQ ID NO: 198 - DNA, 20 bp, Artificial sequence
  Synthetic oligonucleotide
tctcttcatcctttggccca

SEQ ID NO: 199 - DNA, 20 bp, Artificial sequence
  Synthetic oligonucleotide
ctctcttcatcctttggccc

SEQ ID NO: 200 - DNA, 20 bp, Artificial sequence
  Synthetic oligonucleotide
cctctcttcatcctttggcc

SEQ ID NO: 201 - DNA, 20 bp, Artificial sequence
  Synthetic oligonucleotide
gcctctcttcatcctttggc

SEQ ID NO: 202 - DNA, 20 bp, Artificial sequence
  Synthetic oligonucleotide
tgcctctcttcatcctttgg

SEQ ID NO: 203 - DNA, 20 bp, Artificial sequence
  Synthetic oligonucleotide
atgcctctcttcatcctttg

SEQ ID NO: 204 - DNA, 20 bp, Artificial sequence
  Synthetic oligonucleotide
catgcctctcttcatccttt

SEQ ID NO: 205 - DNA, 20 bp, Artificial sequence
  Synthetic oligonucleotide
acatgcctctcttcatcctt

SEQ ID NO: 206 - DNA, 20 bp, Artificial sequence
  Synthetic oligonucleotide
aacatgcctctcttcatcct

SEQ ID NO: 207 - DNA, 20 bp, Artificial sequence
  Synthetic oligonucleotide
tgctttttcatggaccacca

SEQ ID NO: 208 - DNA, 20 bp, Artificial sequence
  Synthetic oligonucleotide
ctgctttttcatggaccacc

SEQ ID NO: 209 - DNA, 20 bp, Artificial sequence
  Synthetic oligonucleotide
tctgctttttcatggaccac

SEQ ID NO: 210 - DNA, 20 bp, Artificial sequence
  Synthetic oligonucleotide
atctgctttttcatggacca

SEQ ID NO: 211 - DNA, 20 bp, Artificial sequence
  Synthetic oligonucleotide
catctgctttttcatggacc

SEQ ID NO: 212 - DNA, 20 bp, Artificial sequence
  Synthetic oligonucleotide
tcatctgctttttcatggac

SEQ ID NO: 213 - DNA, 20 bp, Artificial sequence
  Synthetic oligonucleotide
gtcatctgctttttcatgga

SEQ ID NO: 214 - DNA, 20 bp, Artificial sequence
  Synthetic oligonucleotide
agtcatctgctttttcatgg

SEQ ID NO: 215 - DNA, 20 bp, Artificial sequence
  Synthetic oligonucleotide
aagtcatctgctttttcatg

SEQ ID NO: 216 - DNA, 20 bp, Artificial sequence
  Synthetic oligonucleotide
caagtcatctgctttttcat

SEQ ID NO: 217 - DNA, 20 bp, Artificial sequence
  Synthetic oligonucleotide
ccaagtcatctgctttttca

SEQ ID NO: 218 - DNA, 20 bp, Artificial sequence
  Synthetic oligonucleotide
cccaagtcatctgctttttc

SEQ ID NO: 219 - DNA, 20 bp, Artificial sequence
  Synthetic oligonucleotide
gcccaagtcatctgcttttt

SEQ ID NO: 220 - DNA, 20 bp, Artificial sequence
  Synthetic oligonucleotide
tgcccaagtcatctgctttt

SEQ ID NO: 221 - DNA, 20 bp, Artificial sequence
  Synthetic oligonucleotide
ttgcccaagtcatctgcttt

SEQ ID NO: 222 - DNA, 20 bp, Artificial sequence
  Synthetic oligonucleotide
tttgcccaagtcatctgctt

SEQ ID NO: 223 - DNA, 20 bp, Artificial sequence
  Synthetic oligonucleotide
ctttgcccaagtcatctgct

SEQ ID NO: 224 - DNA, 20 bp, Artificial sequence
  Synthetic oligonucleotide
cctttgcccaagtcatctgc

SEQ ID NO: 225 - DNA, 20 bp, Artificial sequence
  Synthetic oligonucleotide
acctttgcccaagtcatctg

SEQ ID NO: 226 - DNA, 20 bp, Artificial sequence
  Synthetic oligonucleotide
cccaattacaccacaagcca

SEQ ID NO: 227 - DNA, 20 bp, Artificial sequence
  Synthetic oligonucleotide
tcccaattacaccacaagcc

SEQ ID NO: 228 - DNA, 20 bp, Artificial sequence
  Synthetic oligonucleotide
atcccaattacaccacaagc

SEQ ID NO: 229 - DNA, 20 bp, Artificial sequence
  Synthetic oligonucleotide
gatcccaattacaccacaag

SEQ ID NO: 230 - DNA, 20 bp, Artificial sequence
  Synthetic oligonucleotide
cgatcccaattacaccacaa

SEQ ID NO: 231 - DNA, 20 bp, Artificial sequence
  Synthetic oligonucleotide
gcgatcccaattacaccaca

SEQ ID NO: 232 - DNA, 20 bp, Artificial sequence
  Synthetic oligonucleotide
gggcgatcccaattacacca

SEQ ID NO: 233 - DNA, 20 bp, Artificial sequence
  Synthetic oligonucleotide
tgggcgatcccaattacacc

SEQ ID NO: 234 - DNA, 20 bp, Artificial sequence
  Synthetic oligonucleotide
ttgggcgatcccaattacac

SEQ ID NO: 235 - DNA, 20 bp, Artificial sequence
  Synthetic oligonucleotide
attgggcgatcccaattaca

SEQ ID NO: 236 - DNA, 20 bp, Artificial sequence
  Synthetic oligonucleotide
tattgggcgatcccaattac

SEQ ID NO: 237 - DNA, 20 bp, Artificial sequence
  Synthetic oligonucleotide
ttattgggcgatcccaatta

SEQ ID NO: 238 - DNA, 20 bp, Artificial sequence
  Synthetic oligonucleotide
tttattgggcgatcccaatt

SEQ ID NO: 239 - DNA, 20 bp, Artificial sequence
  Synthetic oligonucleotide
gtttattgggcgatcccaat

SEQ ID NO: 240 - DNA, 20 bp, Artificial sequence
  Synthetic oligonucleotide
tgtttattgggcgatcccaa

SEQ ID NO: 241 - DNA, 20 bp, Artificial sequence
  Synthetic oligonucleotide
atgtttattgggcgatccca

SEQ ID NO: 242 - DNA, 20 bp, Artificial sequence
  Synthetic oligonucleotide
aatgtttattgggcgatccc

SEQ ID NO: 243 - DNA, 20 bp, Artificial sequence
  Synthetic oligonucleotide
gaatgtttattgggcgatcc

SEQ ID NO: 244 - DNA, 20 bp, Artificial sequence
  Synthetic oligonucleotide
tccaagggaatgtttattgg

SEQ ID NO: 245 - DNA, 20 bp, Artificial sequence
  Synthetic oligonucleotide
atccaagggaatgtttattg

SEQ ID NO: 246 - DNA, 20 bp, Artificial sequence
  Synthetic oligonucleotide
catccaagggaatgtttatt

SEQ ID NO: 247 - DNA, 20 bp, Artificial sequence
  Synthetic oligonucleotide
acatccaagggaatgtttat

SEQ ID NO: 248 - DNA, 20 bp, Artificial sequence
  Synthetic oligonucleotide
tacatccaagggaatgttta

SEQ ID NO: 249 - DNA, 20 bp, Artificial sequence
  Synthetic oligonucleotide
ctacatccaagggaatgttt

SEQ ID NO: 250 - DNA, 20 bp, Artificial sequence
  Synthetic oligonucleotide
actacatccaagggaatgtt

SEQ ID NO: 251 - DNA, 20 bp, Artificial sequence
  Synthetic oligonucleotide
gactacatccaagggaatgt

SEQ ID NO: 252 - DNA, 20 bp, Artificial sequence
  Synthetic oligonucleotide
agactacatccaagggaatg

SEQ ID NO: 253 - DNA, 20 bp, Artificial sequence
  Synthetic oligonucleotide
cagactacatccaagggaat

SEQ ID NO: 254 - DNA, 20 bp, Artificial sequence
  Synthetic oligonucleotide
tcagactacatccaagggaa

SEQ ID NO: 255 - DNA, 20 bp, Artificial sequence
  Synthetic oligonucleotide
ctcagactacatccaaggga

SEQ ID NO: 256 - DNA, 20 bp, Artificial sequence
  Synthetic oligonucleotide
gcctcagactacatccaagg

SEQ ID NO: 257 - DNA, 20 bp, Artificial sequence
  Synthetic oligonucleotide
ggcctcagactacatccaag

SEQ ID NO: 258 - DNA, 20 bp, Artificial sequence
  Synthetic oligonucleotide
gggcctcagactacatccaa

SEQ ID NO: 259 - DNA, 20 bp, Artificial sequence
  Synthetic oligonucleotide
caggataacagatgagttaa

SEQ ID NO: 260 - DNA, 20 bp, Artificial sequence
  Synthetic oligonucleotide
gcaggataacagatgagtta

SEQ ID NO: 261 - DNA, 20 bp, Artificial sequence
  Synthetic oligonucleotide
agcaggataacagatgagtt

SEQ ID NO: 262 - DNA, 20 bp, Artificial sequence
  Synthetic oligonucleotide
tagcaggataacagatgagt

SEQ ID NO: 263 - DNA, 20 bp, Artificial sequence
  Synthetic oligonucleotide
ctagcaggataacagatgag

SEQ ID NO: 264 - DNA, 20 bp, Artificial sequence
  Synthetic oligonucleotide
gctagcaggataacagatga

SEQ ID NO: 265 - DNA, 20 bp, Artificial sequence
  Synthetic oligonucleotide
agctagcaggataacagatg

SEQ ID NO: 266 - DNA, 20 bp, Artificial sequence
  Synthetic oligonucleotide
cagctagcaggataacagat

SEQ ID NO: 267 - DNA, 20 bp, Artificial sequence
  Synthetic oligonucleotide
acagctagcaggataacaga

SEQ ID NO: 268 - DNA, 20 bp, Artificial sequence
  Synthetic oligonucleotide
tacagctagcaggataacag

SEQ ID NO: 269 - DNA, 20 bp, Artificial sequence
  Synthetic oligonucleotide
ctacagctagcaggataaca

SEQ ID NO: 270 - DNA, 20 bp, Artificial sequence
  Synthetic oligonucleotide
tctacagctagcaggataac

SEQ ID NO: 271 - DNA, 20 bp, Artificial sequence
  Synthetic oligonucleotide
ttctacagctagcaggataa

SEQ ID NO: 272 - DNA, 20 bp, Artificial sequence
  Synthetic oligonucleotide
tttctacagctagcaggata

SEQ ID NO: 273 - DNA, 20 bp, Artificial sequence
  Synthetic oligonucleotide
atttctacagctagcaggat

SEQ ID NO: 274 - DNA, 20 bp, Artificial sequence
  Synthetic oligonucleotide
catttctacagctagcagga

SEQ ID NO: 275 - DNA, 20 bp, Artificial sequence
  Synthetic oligonucleotide
acatttctacagctagcagg

SEQ ID NO: 276 - DNA, 20 bp, Artificial sequence
  Synthetic oligonucleotide
tacatttctacagctagcag

SEQ ID NO: 277 - DNA, 20 bp, Artificial sequence
  Synthetic oligonucleotide
atacatttctacagctagca

SEQ ID NO: 278 - DNA, 20 bp, Artificial sequence
  Synthetic oligonucleotide
gatacatttctacagctagc

SEQ ID NO: 279 - DNA, 20 bp, Artificial sequence
  Synthetic oligonucleotide
acagtgtttaatgtttatca

SEQ ID NO: 280 - DNA, 20 bp, Artificial sequence
  Synthetic oligonucleotide
tacagtgtttaatgtttatc

SEQ ID NO: 281 - DNA, 20 bp, Artificial sequence
  Synthetic oligonucleotide
ttacagtgtttaatgtttat

SEQ ID NO: 282 - DNA, 20 bp, Artificial sequence
  Synthetic oligonucleotide
attacagtgtttaatgttta

SEQ ID NO: 283 - DNA, 20 bp, Artificial sequence
  Synthetic oligonucleotide
gattacagtgtttaatgttt

SEQ ID NO: 284 - DNA, 20 bp, Artificial sequence
  Synthetic oligonucleotide
agattacagtgtttaatgtt

SEQ ID NO: 285 - DNA, 20 bp, Artificial sequence
  Synthetic oligonucleotide
aagattacagtgtttaatgt

SEQ ID NO: 286 - DNA, 20 bp, Artificial sequence
  Synthetic oligonucleotide
taagattacagtgtttaatg

SEQ ID NO: 287 - DNA, 20 bp, Artificial sequence
  Synthetic oligonucleotide
ttaagattacagtgtttaat

SEQ ID NO: 288 - DNA, 20 bp, Artificial sequence
  Synthetic oligonucleotide
caaatcttccaagtgatcat

SEQ ID NO: 289 - DNA, 20 bp, Artificial sequence
  Synthetic oligonucleotide
acaaatcttccaagtgatca

SEQ ID NO: 290 - DNA, 20 bp, Artificial sequence
  Synthetic oligonucleotide
tacaaatcttccaagtgatc

SEQ ID NO: 291 - DNA, 20 bp, Artificial sequence
  Synthetic oligonucleotide
tatacaaatcttccaagtga

SEQ ID NO: 292 - DNA, 20 bp, Artificial sequence
  Synthetic oligonucleotide
ctatacaaatcttccaagtg

SEQ ID NO: 293 - DNA, 20 bp, Artificial sequence
  Synthetic oligonucleotide
actatacaaatcttccaagt

SEQ ID NO: 294 - DNA, 20 bp, Artificial sequence
  Synthetic oligonucleotide
aactatacaaatcttccaag

SEQ ID NO: 295 - DNA, 20 bp, Artificial sequence
  Synthetic oligonucleotide
aaactatacaaatcttccaa

SEQ ID NO: 296 - DNA, 20 bp, Artificial sequence
  Synthetic oligonucleotide
aaaactatacaaatcttcca

SEQ ID NO: 297 - DNA, 20 bp, Artificial sequence
  Synthetic oligonucleotide
taaaactatacaaatcttcc

SEQ ID NO: 298 - DNA, 20 bp, Artificial sequence
  Synthetic oligonucleotide
ataaaactatacaaatcttc

SEQ ID NO: 299 - DNA, 20 bp, Artificial sequence
  Synthetic oligonucleotide
tataaaactatacaaatctt

SEQ ID NO: 300 - DNA, 20 bp, Artificial sequence
  Synthetic oligonucleotide
ttataaaactatacaaatct

SEQ ID NO: 301 - DNA, 20 bp, Artificial sequence
  Synthetic oligonucleotide
tttataaaactatacaaatc

SEQ ID NO: 302 - DNA, 20 bp, Artificial sequence
  Synthetic oligonucleotide
ttttataaaactatacaaat

SEQ ID NO: 303 - DNA, 20 bp, Artificial sequence
  Synthetic oligonucleotide
gttttataaaactatacaaa

SEQ ID NO: 304 - DNA, 20 bp, Artificial sequence
  Synthetic oligonucleotide
agttttataaaactatacaa

SEQ ID NO: 305 - DNA, 20 bp, Artificial sequence
  Synthetic oligonucleotide
gagttttataaaactataca

SEQ ID NO: 306 - DNA, 20 bp, Artificial sequence
  Synthetic oligonucleotide
cattgaaacagacattttaa

SEQ ID NO: 307 - DNA, 20 bp, Artificial sequence
  Synthetic oligonucleotide
gtcattgaaacagacatttt

SEQ ID NO: 308 - DNA, 20 bp, Artificial sequence
  Synthetic oligonucleotide
ggtcattgaaacagacattt

SEQ ID NO: 309 - DNA, 20 bp, Artificial sequence
  Synthetic oligonucleotide
aggtcattgaaacagacatt

SEQ ID NO: 310 - DNA, 20 bp, Artificial sequence
  Synthetic oligonucleotide
caggtcattgaaacagacat

SEQ ID NO: 311 - DNA, 20 bp, Artificial sequence
  Synthetic oligonucleotide
acaggtcattgaaacagaca

SEQ ID NO: 312 - DNA, 20 bp, Artificial sequence
  Synthetic oligonucleotide
tacaggtcattgaaacagac

SEQ ID NO: 313 - DNA, 20 bp, Artificial sequence
  Synthetic oligonucleotide
aatacaggtcattgaaacag

SEQ ID NO: 314 - DNA, 20 bp, Artificial sequence
  Synthetic oligonucleotide
aaatacaggtcattgaaaca

SEQ ID NO: 315 - DNA, 20 bp, Artificial sequence
  Synthetic oligonucleotide
aaaatacaggtcattgaaac

SEQ ID NO: 316 - DNA, 20 bp, Artificial sequence
  Synthetic oligonucleotide
caaaatacaggtcattgaaa

SEQ ID NO: 317 - DNA, 20 bp, Artificial sequence
  Synthetic oligonucleotide
ccttgccttctgctcgaaat

SEQ ID NO: 318 - DNA, 20 bp, Artificial sequence
  Synthetic oligonucleotide
aataaagttgacctcttttt

SEQ ID NO: 319 - DNA, 20 bp, Artificial sequence
  Synthetic oligonucleotide
ctctgatataaaaatcttgt

SEQ ID NO: 320 - DNA, 20 bp, Artificial sequence
  Synthetic oligonucleotide
gccccgcggcggcctcggtc

SEQ ID NO: 321 - DNA, 20 bp, Artificial sequence
  Synthetic oligonucleotide
gctatcgccattattacaag

SEQ ID NO: 322 - DNA, 20 bp, Artificial sequence
  Synthetic oligonucleotide
ctcaaatgtgaaagttgtcc

SEQ ID NO: 323 - DNA, 20 bp, Artificial sequence
  Synthetic oligonucleotide
gttctatattcaataaatgc

SEQ ID NO: 324 - DNA, 20 bp, Artificial sequence
  Synthetic oligonucleotide
aattaaagttcccaaataca

SEQ ID NO: 325 - DNA, 20 bp, Artificial sequence
  Synthetic oligonucleotide
gatcattacaaaagttaaga

SEQ ID NO: 326 - DNA, 20 bp, Artificial sequence
  Synthetic oligonucleotide
ccttctctgcccttgcagcc

SEQ ID NO: 327 - DNA, 20 bp, Artificial sequence
  Synthetic oligonucleotide
acccaaataactatgttgta

SEQ ID NO: 328 - DNA, 20 bp, Artificial sequence
  Synthetic oligonucleotide
ccaggttttaaacttaacaa

SEQ ID NO: 329 - DNA, 20 bp, Artificial sequence
  Synthetic oligonucleotide
atctcaggactaaaataaac

SEQ ID NO: 330 - DNA, 20 bp, Artificial sequence
  Synthetic oligonucleotide
aaataactatgttgtagacc

SEQ ID NO: 331 - DNA, 20 bp, Artificial sequence
  Synthetic oligonucleotide
aagaaccttttccagaaaat

SEQ ID NO: 332 - DNA, 20 bp, Artificial sequence
  Synthetic oligonucleotide
ggaacagaaacaagtctatg

SEQ ID NO: 333 - DNA, 20 bp, Artificial sequence
  Synthetic oligonucleotide
agaaagctatcgccattatt

SEQ ID NO: 334 - DNA, 20 bp, Artificial sequence
  Synthetic oligonucleotide
ttcccaaatacattctaaaa

SEQ ID NO: 335 - DNA, 20 bp, Artificial sequence
  Synthetic oligonucleotide
aactgctctaggcctgtgtc

SEQ ID NO: 336 - DNA, 20 bp, Artificial sequence
  Synthetic oligonucleotide
aaatggatcaaatctgatca

SEQ ID NO: 337 - DNA, 20 bp, Artificial sequence
  Synthetic oligonucleotide
gtaggtgcacatcaaaatca

SEQ ID NO: 338 - DNA, 20 bp, Artificial sequence
  Synthetic oligonucleotide
tctgatataaaaatcttgtc

SEQ ID NO: 339 - DNA, 20 bp, Artificial sequence
  Synthetic oligonucleotide
accatatgaactccagaaag

SEQ ID NO: 340 - DNA, 20 bp, Artificial sequence
  Synthetic oligonucleotide
aacatcaaggtagttcatga

SEQ ID NO: 341 - DNA, 20 bp, Artificial sequence
  Synthetic oligonucleotide
gcaattacagaaatggatca

SEQ ID NO: 342 - DNA, 20 bp, Artificial sequence
  Synthetic oligonucleotide
ttttaagcatattccaaagt

SEQ ID NO: 343 - DNA, 20 bp, Artificial sequence
  Synthetic oligonucleotide
tcaacccccagctcaaacac

SEQ ID NO: 344 - DNA, 20 bp, Artificial sequence
  Synthetic oligonucleotide
agaaaaataacattaatcct

SEQ ID NO: 345 - DNA, 20 bp, Artificial sequence
  Synthetic oligonucleotide
aagattttaaacacggaata

SEQ ID NO: 346 - DNA, 20 bp, Artificial sequence
  Synthetic oligonucleotide
agcagtcacattgcccaagt

SEQ ID NO: 347 - DNA, 20 bp, Artificial sequence
  Synthetic oligonucleotide
cagtgtttaatgtttatcag

SEQ ID NO: 348 - DNA, 20 bp, Artificial sequence
  Synthetic oligonucleotide
gcaaaatacaggtcattgaa

SEQ ID NO: 349 - DNA, 20 bp, Artificial sequence
  Synthetic oligonucleotide
ggcaaaatacaggtcattga

SEQ ID NO: 350 - DNA, 20 bp, Artificial sequence
  Synthetic oligonucleotide
tggcaaaatacaggtcattg

SEQ ID NO: 351 - DNA, 20 bp, Artificial sequence
  Synthetic oligonucleotide
ctggcaaaatacaggtcatt

SEQ ID NO: 352 - DNA, 20 bp, Artificial sequence
  Synthetic oligonucleotide
tctggcaaaatacaggtcat

SEQ ID NO: 353 - DNA, 20 bp, Artificial sequence
  Synthetic oligonucleotide
gtctggcaaaatacaggtca

SEQ ID NO: 354 - DNA, 20 bp, Artificial sequence
  Synthetic oligonucleotide
agtctggcaaaatacaggtc

SEQ ID NO: 355 - DNA, 20 bp, Artificial sequence
  Synthetic oligonucleotide
aagtctggcaaaatacaggt

SEQ ID NO: 356 - DNA, 20 bp, Artificial sequence
  Synthetic oligonucleotide
taagtctggcaaaatacagg

SEQ ID NO: 357 - DNA, 20 bp, Artificial sequence
  Synthetic oligonucleotide
ttaagtctggcaaaatacag

SEQ ID NO: 358 - DNA, 20 bp, Artificial sequence
  Synthetic oligonucleotide
gtttaatacccatctgtgat

SEQ ID NO: 359 - DNA, 20 bp, Artificial sequence
  Synthetic oligonucleotide
aagtttaatacccatctgtg

SEQ ID NO: 360 - DNA, 20 bp, Artificial sequence
  Synthetic oligonucleotide
caagtttaatacccatctgt

SEQ ID NO: 361 - DNA, 20 bp, Artificial sequence
  Synthetic oligonucleotide
acaagtttaatacccatctg

SEQ ID NO: 362 - DNA, 20 bp, Artificial sequence
  Synthetic oligonucleotide
gacaagtttaatacccatct

SEQ ID NO: 363 - DNA, 20 bp, Artificial sequence
  Synthetic oligonucleotide
tgacaagtttaatacccatc

SEQ ID NO: 364 - DNA, 20 bp, Artificial sequence
  Synthetic oligonucleotide
ctgacaagtttaatacccat

SEQ ID NO: 365 - DNA, 20 bp, Artificial sequence
  Synthetic oligonucleotide
tctgacaagtttaataccca

SEQ ID NO: 366 - DNA, 20 bp, Artificial sequence
  Synthetic oligonucleotide
ttctgacaagtttaataccc

SEQ ID NO: 367 - DNA, 20 bp, Artificial sequence
  Synthetic oligonucleotide
attctgacaagtttaatacc

SEQ ID NO: 368 - DNA, 20 bp, Artificial sequence
  Synthetic oligonucleotide
aattctgacaagtttaatac

SEQ ID NO: 369 - DNA, 20 bp, Artificial sequence
  Synthetic oligonucleotide
aaattctgacaagtttaata

SEQ ID NO: 370 - DNA, 20 bp, Artificial sequence
  Synthetic oligonucleotide
gaaattctgacaagtttaat

SEQ ID NO: 371 - DNA, 20 bp, Artificial sequence
  Synthetic oligonucleotide
agaaattctgacaagtttaa

SEQ ID NO: 372 - DNA, 20 bp, Artificial sequence
  Synthetic oligonucleotide
aagaaattctgacaagttta

SEQ ID NO: 373 - DNA, 20 bp, Artificial sequence
  Synthetic oligonucleotide
ttattcacaggcttgaatga

SEQ ID NO: 374 - DNA, 20 bp, Artificial sequence
  Synthetic oligonucleotide
tttattcacaggcttgaatg

SEQ ID NO: 375 - DNA, 20 bp, Artificial sequence
  Synthetic oligonucleotide
ttttattcacaggcttgaat

SEQ ID NO: 376 - DNA, 20 bp, Artificial sequence
  Synthetic oligonucleotide
tttttattcacaggcttgaa

SEQ ID NO: 377 - DNA, 20 bp, Artificial sequence
  Synthetic oligonucleotide
gtttttattcacaggcttga

SEQ ID NO: 378 - DNA, 20 bp, Artificial sequence
  Synthetic oligonucleotide
gggtttttattcacaggctt

SEQ ID NO: 379 - DNA, 20 bp, Artificial sequence
  Synthetic oligonucleotide
cagggtttttattcacaggc

SEQ ID NO: 380 - DNA, 20 bp, Artificial sequence
  Synthetic oligonucleotide
acagggtttttattcacagg

SEQ ID NO: 381 - DNA, 20 bp, Artificial sequence
  Synthetic oligonucleotide
tacagggtttttattcacag

SEQ ID NO: 382 - DNA, 20 bp, Artificial sequence
  Synthetic oligonucleotide
catacagggtttttattcac

SEQ ID NO: 383 - DNA, 20 bp, Artificial sequence
  Synthetic oligonucleotide
gccatacagggtttttattc

SEQ ID NO: 384 - DNA, 20 bp, Artificial sequence
  Synthetic oligonucleotide
tgccatacagggtttttatt

SEQ ID NO: 385 - DNA, 20 bp, Artificial sequence
  Synthetic oligonucleotide
gtgccatacagggtttttat

SEQ ID NO: 386 - DNA, 20 bp, Artificial sequence
  Synthetic oligonucleotide
agtgccatacagggttttta

SEQ ID NO: 387 - DNA, 20 bp, Artificial sequence
  Synthetic oligonucleotide
tggaaaaactcaaatgtgaa

SEQ ID NO: 388 - DNA, 20 bp, Artificial sequence
  Synthetic oligonucleotide
tttccctttcttttccacac

SEQ ID NO: 389 - DNA, 20 bp, Artificial sequence
  Synthetic oligonucleotide
tctttccctttcttttccac

SEQ ID NO: 390 - DNA, 20 bp, Artificial sequence
  Synthetic oligonucleotide
taccttctctgcccttgcag

SEQ ID NO: 391 - DNA, 20 bp, Artificial sequence
  Synthetic oligonucleotide
gcaagggccaaggctgctgc

SEQ ID NO: 392 - DNA, 20 bp, Artificial sequence
  Synthetic oligonucleotide
aaagctaaattatgaattaa

SEQ ID NO: 393 - DNA, 20 bp, Artificial sequence
  Synthetic oligonucleotide
ctaatgaaggctcagtatga

SEQ ID NO: 394 - DNA, 20 bp, Artificial sequence
  Synthetic oligonucleotide
ggagtcaaatgccaaagaac

SEQ ID NO: 395 - DNA, 20 bp, Artificial sequence
  Synthetic oligonucleotide
tgaattaaagttcccaaata

SEQ ID NO: 396 - DNA, 20 bp, Artificial sequence
  Synthetic oligonucleotide
acttggtgcaggcagaatat

SEQ ID NO: 397 - DNA, 20 bp, Artificial sequence
  Synthetic oligonucleotide
cctctgatataaaaatcttg

SEQ ID NO: 398 - DNA, 20 bp, Artificial sequence
  Synthetic oligonucleotide
aaagttggagagagtttctg

SEQ ID NO: 399 - DNA, 20 bp, Artificial sequence
  Synthetic oligonucleotide
tctctgcccttgcagcccaa

SEQ ID NO: 400 - DNA, 20 bp, Artificial sequence
  Synthetic oligonucleotide
ttacttggtgcaggcagaat

SEQ ID NO: 401 - DNA, 20 bp, Artificial sequence
  Synthetic oligonucleotide
aatggagtcaaatgccaaag

SEQ ID NO: 402 - DNA, 20 bp, Artificial sequence
  Synthetic oligonucleotide
tatgaattaaagttcccaaa

SEQ ID NO: 403 - DNA, 20 bp, Artificial sequence
  Synthetic oligonucleotide
agttctatattcaataaatg

SEQ ID NO: 404 - DNA, 20 bp, Artificial sequence
  Synthetic oligonucleotide
tacaagtagtataccatatg

SEQ ID NO: 405 - DNA, 20 bp, Artificial sequence
  Synthetic oligonucleotide
tagccttagagctgtacaaa

SEQ ID NO: 406 - DNA, 20 bp, Artificial sequence
  Synthetic oligonucleotide
gtccccatttgtcaattcct

SEQ ID NO: 407 - DNA, 20 bp, Artificial sequence
  Synthetic oligonucleotide
aacctgcctactggcagagc

SEQ ID NO: 408 - DNA, 20 bp, Artificial sequence
  Synthetic oligonucleotide
cttgttcccacactcaatgc

SEQ ID NO: 409 - DNA, 20 bp, Artificial sequence
  Synthetic oligonucleotide
acaagtcatgataacctgca

SEQ ID NO: 410 - DNA, 20 bp, Artificial sequence
  Synthetic oligonucleotide
tgttttccaaactcagatct

SEQ ID NO: 411 - DNA, 20 bp, Artificial sequence
  Synthetic oligonucleotide
agaacctcataatattagaa

SEQ ID NO: 412 - DNA, 20 bp, Artificial sequence
  Synthetic oligonucleotide
ggttttaaacttaacaaaat

SEQ ID NO: 413 - DNA, 20 bp, Artificial sequence
  Synthetic oligonucleotide
ctctggtgtatttttagtaa

SEQ ID NO: 414 - DNA, 20 bp, Artificial sequence
  Synthetic oligonucleotide
tatctctgcatatctggaaa

SEQ ID NO: 415 - DNA, 20 bp, Artificial sequence
  Synthetic oligonucleotide
cagcctttttaacccaaaag

SEQ ID NO: 416 - DNA, 20 bp, Artificial sequence
  Synthetic oligonucleotide
tggaatgctccactatccaa

SEQ ID NO: 417 - DNA, 20 bp, Artificial sequence
  Synthetic oligonucleotide
cgttcagaagtttgtctctg

SEQ ID NO: 418 - DNA, 20 bp, Artificial sequence
  Synthetic oligonucleotide
ctgctcagggaaggtggaaa

SEQ ID NO: 419 - DNA, 20 bp, Artificial sequence
  Synthetic oligonucleotide
tcaagagaagctaggaaaac

SEQ ID NO: 420 - DNA, 20 bp, Artificial sequence
  Synthetic oligonucleotide
tccctttcttttccacacct

SEQ ID NO: 421 - DNA, 20 bp, Artificial sequence
  Synthetic oligonucleotide
ttgttcccacactcaatgca

SEQ ID NO: 422 - DNA, 20 bp, Artificial sequence
  Synthetic oligonucleotide
tcaccagcacagcacaacac

SEQ ID NO: 423 - DNA, 20 bp, Artificial sequence
  Synthetic oligonucleotide
cctgggatcattacaaaagt

SEQ ID NO: 424 - DNA, 20 bp, Artificial sequence
  Synthetic oligonucleotide
agtagtataccatatgaact

SEQ ID NO: 425 - DNA, 20 bp, Artificial sequence
  Synthetic oligonucleotide
tctaatatggtcaaatgtaa

SEQ ID NO: 426 - DNA, 20 bp, Artificial sequence
  Synthetic oligonucleotide
ggttgggctctggtgtattt

SEQ ID NO: 427 - DNA, 20 bp, Artificial sequence
  Synthetic oligonucleotide
tgccctttacttggtgcagg

SEQ ID NO: 428 - DNA, 20 bp, Artificial sequence
  Synthetic oligonucleotide
agagagtttctgaacaaaga

SEQ ID NO: 429 - DNA, 20 bp, Artificial sequence
  Synthetic oligonucleotide
gaatttcagcaattacagaa

SEQ ID NO: 430 - DNA, 20 bp, Artificial sequence
  Synthetic oligonucleotide
acaagttaaacaagtcatga

SEQ ID NO: 431 - DNA, 20 bp, Artificial sequence
  Synthetic oligonucleotide
tgtgccctttacttggtgca

SEQ ID NO: 432 - DNA, 20 bp, Artificial sequence
  Synthetic oligonucleotide
ttaggaggaggaaaaggacc

SEQ ID NO: 433 - DNA, 20 bp, Artificial sequence
  Synthetic oligonucleotide
actggcagagcaattttaaa

SEQ ID NO: 434 - DNA, 20 bp, Artificial sequence
  Synthetic oligonucleotide
agtcaaatgccaaagaacct

SEQ ID NO: 435 - DNA, 20 bp, Artificial sequence
  Synthetic oligonucleotide
aagcatcagatggattaggg

SEQ ID NO: 436 - DNA, 20 bp, Artificial sequence
  Synthetic oligonucleotide
gtccgcgggaccctcaggaa

SEQ ID NO: 437 - DNA, 20 bp, Artificial sequence
  Synthetic oligonucleotide
caattacagaaatggatcaa

SEQ ID NO: 438 - DNA, 20 bp, Artificial sequence
  Synthetic oligonucleotide
gctgtcaagtaatcactacc

SEQ ID NO: 439 - DNA, 20 bp, Artificial sequence
  Synthetic oligonucleotide
agtgcaaagttggagagagt

SEQ ID NO: 440 - DNA, 20 bp, Artificial sequence
  Synthetic oligonucleotide
acttgcttccaatcccaaat

SEQ ID NO: 441 - DNA, 20 bp, Artificial sequence
  Synthetic oligonucleotide
aactcaaatgtgaaagttgt

SEQ ID NO: 442 - DNA, 20 bp, Artificial sequence
  Synthetic oligonucleotide
ttttagtaagatcttcaaat

SEQ ID NO: 443 - DNA, 20 bp, Artificial sequence
  Synthetic oligonucleotide
atttcagcaattacagaaat

SEQ ID NO: 444 - DNA, 20 bp, Artificial sequence
  Synthetic oligonucleotide
ttaagtgtccccatttgtca

SEQ ID NO: 445 - DNA, 20 bp, Artificial sequence
  Synthetic oligonucleotide
ttagcaacctgcctactggc

SEQ ID NO: 446 - DNA, 20 bp, Artificial sequence
  Synthetic oligonucleotide
tattacaagagttaagcatc

SEQ ID NO: 447 - DNA, 20 bp, Artificial sequence
  Synthetic oligonucleotide
atgttgaatatacatgtaca

SEQ ID NO: 448 - DNA, 20 bp, Artificial sequence
  Synthetic oligonucleotide
tttgtctctgaccatcttag

SEQ ID NO: 449 - DNA, 20 bp, Artificial sequence
  Synthetic oligonucleotide
ttttccaccagttggtaact

SEQ ID NO: 450 - DNA, 20 bp, Artificial sequence
  Synthetic oligonucleotide
caacagcttcccacaagtta

SEQ ID NO: 451 - DNA, 20 bp, Artificial sequence
  Synthetic oligonucleotide
caaatgtgaaagttgtccct

SEQ ID NO: 452 - DNA, 20 bp, Artificial sequence
  Synthetic oligonucleotide
gctaccttctctgcccttgc

SEQ ID NO: 453 - DNA, 20 bp, Artificial sequence
  Synthetic oligonucleotide
tcttagcagaacagtgttct

SEQ ID NO: 454 - DNA, 20 bp, Artificial sequence
  Synthetic oligonucleotide
atacattctaaaaagaaaca

SEQ ID NO: 455 - DNA, 20 bp, Artificial sequence
  Synthetic oligonucleotide
gcacatatttacaagtagta

SEQ ID NO: 456 - DNA, 20 bp, Artificial sequence
  Synthetic oligonucleotide
gggtcaccagcacagcacaa

SEQ ID NO: 457 - DNA, 20 bp, Artificial sequence
  Synthetic oligonucleotide
gtgcaagggccaaggctgct

SEQ ID NO: 458 - DNA, 20 bp, Artificial sequence
  Synthetic oligonucleotide
acctgggttcatgcatggat

SEQ ID NO: 459 - DNA, 20 bp, Artificial sequence
  Synthetic oligonucleotide
atcactatttgaaactaaat

SEQ ID NO: 460 - DNA, 20 bp, Artificial sequence
  Synthetic oligonucleotide
atacaataaagttgacctct

SEQ ID NO: 461 - DNA, 20 bp, Artificial sequence
  Synthetic oligonucleotide
ttttaaacttaacaaaatgt

SEQ ID NO: 462 - DNA, 20 bp, Artificial sequence
  Synthetic oligonucleotide
ctccccgcgctcccgccacg

SEQ ID NO: 463 - DNA, 20 bp, Artificial sequence
  Synthetic oligonucleotide
gaaggctcagtatgaagaga

SEQ ID NO: 464 - DNA, 20 bp, Artificial sequence
  Synthetic oligonucleotide
agaaaacagctgatttacct

SEQ ID NO: 465 - DNA, 20 bp, Artificial sequence
  Synthetic oligonucleotide
ccacaagttaaacaagtcat

SEQ ID NO: 466 - DNA, 20 bp, Artificial sequence
  Synthetic oligonucleotide
caaatttgcaaacaagtagc

SEQ ID NO: 467 - DNA, 20 bp, Artificial sequence
  Synthetic oligonucleotide
cctaatttgaactgcaagta

SEQ ID NO: 468 - DNA, 20 bp, Artificial sequence
  Synthetic oligonucleotide
aaaaaactcatctccccagc

SEQ ID NO: 469 - DNA, 20 bp, Artificial sequence
  Synthetic oligonucleotide
aggctcagtatgaagagatc

SEQ ID NO: 470 - DNA, 20 bp, Artificial sequence
  Synthetic oligonucleotide
tgttatcaagagcacagggc

SEQ ID NO: 471 - DNA, 20 bp, Artificial sequence
  Synthetic oligonucleotide
cctcaaaagggagatggtaa

SEQ ID NO: 472 - DNA, 20 bp, Artificial sequence
  Synthetic oligonucleotide
agtatgggtcaccagcacag

SEQ ID NO: 473 - DNA, 20 bp, Artificial sequence
  Synthetic oligonucleotide
tcacaatctagtgcagttac

SEQ ID NO: 474 - DNA, 20 bp, Artificial sequence
  Synthetic oligonucleotide
caagtgagaaacccaatcct

SEQ ID NO: 475 - DNA, 20 bp, Artificial sequence
  Synthetic oligonucleotide
agaaaatctggccattttaa

SEQ ID NO: 476 - DNA, 20 bp, Artificial sequence
  Synthetic oligonucleotide
acaggtaatggtgctccgtg

SEQ ID NO: 477 - DNA, 20 bp, Artificial sequence
  Synthetic oligonucleotide
tgaaaggctttcagaaaaca

SEQ ID NO: 478 - DNA, 20 bp, Artificial sequence
  Synthetic oligonucleotide
caggcaagttacaggaagca

SEQ ID NO: 479 - DNA, 20 bp, Artificial sequence
  Synthetic oligonucleotide
cagcaagctgcttaactgct

SEQ ID NO: 480 - DNA, 20 bp, Artificial sequence
  Synthetic oligonucleotide
tgttgcaaagacattacctt

SEQ ID NO: 481 - DNA, 20 bp, Artificial sequence
  Synthetic oligonucleotide
gaaactaaattagcaagatg

SEQ ID NO: 482 - DNA, 20 bp, Artificial sequence
  Synthetic oligonucleotide
tcaagagcacagggccaaaa

SEQ ID NO: 483 - DNA, 20 bp, Artificial sequence
  Synthetic oligonucleotide
aggaggaggaaaaggacctc

SEQ ID NO: 484 - DNA, 20 bp, Artificial sequence
  Synthetic oligonucleotide
cctcagcctttttaacccaa

SEQ ID NO: 485 - DNA, 20 bp, Artificial sequence
  Synthetic oligonucleotide
ctatgttgtagaccaccaca

SEQ ID NO: 486 - DNA, 20 bp, Artificial sequence
  Synthetic oligonucleotide
ctccgtggctacatacagaa

SEQ ID NO: 487 - DNA, 20 bp, Artificial sequence
  Synthetic oligonucleotide
tttatctggatctttagaaa

SEQ ID NO: 488 - DNA, 20 bp, Artificial sequence
  Synthetic oligonucleotide
aaaaaaaggaaagtgaaagt

SEQ ID NO: 489 - DNA, 20 bp, Artificial sequence
  Synthetic oligonucleotide
ggttcatgcatggattctca

SEQ ID NO: 490 - DNA, 20 bp, Artificial sequence
  Synthetic oligonucleotide
ctgcaaagtgtcacacaaac

SEQ ID NO: 491 - DNA, 20 bp, Artificial sequence
  Synthetic oligonucleotide
ttcagaagtaccaaagggta

SEQ ID NO: 492 - DNA, 20 bp, Artificial sequence
  Synthetic oligonucleotide
taaaagcattccagcatttg

SEQ ID NO: 493 - DNA, 20 bp, Artificial sequence
  Synthetic oligonucleotide
tagtataccatatgaactcc

SEQ ID NO: 494 - DNA, 20 bp, Artificial sequence
  Synthetic oligonucleotide
tgcatatctggaaagctgga

SEQ ID NO: 495 - DNA, 20 bp, Artificial sequence
  Synthetic oligonucleotide
cttaactgctctaggcctgt

SEQ ID NO: 496 - DNA, 20 bp, Artificial sequence
  Synthetic oligonucleotide
aggcaccgaccgggcggcac

SEQ ID NO: 497 - DNA, 20 bp, Artificial sequence
  Synthetic oligonucleotide
tgcaaagttggagagagttt

SEQ ID NO: 498 - DNA, 20 bp, Artificial sequence
  Synthetic oligonucleotide
tcctcaaaagggagatggta

SEQ ID NO: 499 - DNA, 20 bp, Artificial sequence
  Synthetic oligonucleotide
agtataccatatgaactcca

SEQ ID NO: 500 - DNA, 20 bp, Artificial sequence
  Synthetic oligonucleotide
tatttgtacatgttgaatat

SEQ ID NO: 501 - DNA, 20 bp, Artificial sequence
  Synthetic oligonucleotide
acccaaaaggtgtatgtctc

SEQ ID NO: 502 - DNA, 20 bp, Artificial sequence
  Synthetic oligonucleotide
ctttggaaaaaaaggaaagt

SEQ ID NO: 503 - DNA, 20 bp, Artificial sequence
  Synthetic oligonucleotide
gggagaaaggcaggcaagtt

SEQ ID NO: 504 - DNA, 20 bp, Artificial sequence
  Synthetic oligonucleotide
ttaagcccaggaagtaaaag

SEQ ID NO: 505 - DNA, 20 bp, Artificial sequence
  Synthetic oligonucleotide
agacattacctttaaacatt

SEQ ID NO: 506 - DNA, 20 bp, Artificial sequence
  Synthetic oligonucleotide
gtggcttaagaaatgctccg

SEQ ID NO: 507 - DNA, 20 bp, Artificial sequence
  Synthetic oligonucleotide
gtgagaagggaacagaaaca

SEQ ID NO: 508 - DNA, 20 bp, Artificial sequence
  Synthetic oligonucleotide
aaaagcatcagatggattag

SEQ ID NO: 509 - DNA, 20 bp, Artificial sequence
  Synthetic oligonucleotide
ttccaccagttggtaacttc

SEQ ID NO: 510 - DNA, 20 bp, Artificial sequence
  Synthetic oligonucleotide
tttttagtaagatcttcaaa

SEQ ID NO: 511 - DNA, 20 bp, Artificial sequence
  Synthetic oligonucleotide
atctgtgtccaaatcccagg

SEQ ID NO: 512 - DNA, 20 bp, Artificial sequence
  Synthetic oligonucleotide
taagatcttcaaataagcta

SEQ ID NO: 513 - DNA, 20 bp, Artificial sequence
  Synthetic oligonucleotide
atcaactctttccctttctt

SEQ ID NO: 514 - DNA, 20 bp, Artificial sequence
  Synthetic oligonucleotide
tgtgtcctcaaaagggagat

SEQ ID NO: 515 - DNA, 20 bp, Artificial sequence
  Synthetic oligonucleotide
tacctcctcccaacaatacc

SEQ ID NO: 516 - DNA, 20 bp, Artificial sequence
  Synthetic oligonucleotide
ttctgctttacaactatggc

SEQ ID NO: 517 - DNA, 20 bp, Artificial sequence
  Synthetic oligonucleotide
gtacatgttgaatatacatg

SEQ ID NO: 518 - DNA, 20 bp, Artificial sequence
  Synthetic oligonucleotide
tttgtggctaatcttaaggt

SEQ ID NO: 519 - DNA, 20 bp, Artificial sequence
  Synthetic oligonucleotide
tcctgcctcagcctttttaa

SEQ ID NO: 520 - DNA, 20 bp, Artificial sequence
  Synthetic oligonucleotide
cggtgtccgcgggaccctca

SEQ ID NO: 521 - DNA, 20 bp, Artificial sequence
  Synthetic oligonucleotide
gaaatggatcaaatctgatc

SEQ ID NO: 522 - DNA, 20 bp, Artificial sequence
  Synthetic oligonucleotide
ggtagttcatgagctaaatt

SEQ ID NO: 523 - DNA, 20 bp, Artificial sequence
  Synthetic oligonucleotide
aatggagtctcgactagttt

SEQ ID NO: 524 - DNA, 20 bp, Artificial sequence
  Synthetic oligonucleotide
caagtatgggtcaccagcac

SEQ ID NO: 525 - DNA, 20 bp, Artificial sequence
  Synthetic oligonucleotide
ggtgtccgcgggaccctcag

SEQ ID NO: 526 - DNA, 20 bp, Artificial sequence
  Synthetic oligonucleotide
cgccacgcgcaggcccagcc

SEQ ID NO: 527 - DNA, 20 bp, Artificial sequence
  Synthetic oligonucleotide
tctaggcctgtgtcctcaaa

SEQ ID NO: 528 - DNA, 20 bp, Artificial sequence
  Synthetic oligonucleotide
actgtcctgggctaatgaag

SEQ ID NO: 529 - DNA, 20 bp, Artificial sequence
  Synthetic oligonucleotide
aagcatcttgttacctctct

SEQ ID NO: 530 - DNA, 20 bp, Artificial sequence
  Synthetic oligonucleotide
gcccaggaagtaaaagcatt

SEQ ID NO: 531 - DNA, 20 bp, Artificial sequence
  Synthetic oligonucleotide
gtaagatcttcaaataagct

SEQ ID NO: 532 - DNA, 20 bp, Artificial sequence
  Synthetic oligonucleotide
aaagggagatggtaatcttg

SEQ ID NO: 533 - DNA, 20 bp, Artificial sequence
  Synthetic oligonucleotide
gccaaggctgctgccttaca

SEQ ID NO: 534 - DNA, 20 bp, Artificial sequence
  Synthetic oligonucleotide
cagactaactgttcctgtcc

SEQ ID NO: 535 - DNA, 20 bp, Artificial sequence
  Synthetic oligonucleotide
tttgtcaattcctttaagcc

SEQ ID NO: 536 - DNA, 20 bp, Artificial sequence
  Synthetic oligonucleotide
actacctcctcccaacaata

SEQ ID NO: 537 - DNA, 20 bp, Artificial sequence
  Synthetic oligonucleotide
tacctctcttcatcctttgg

SEQ ID NO: 538 - DNA, 20 bp, Artificial sequence
  Synthetic oligonucleotide
actgctctaggcctgtgtcc

SEQ ID NO: 539 - DNA, 20 bp, Artificial sequence
  Synthetic oligonucleotide
cctcctcccaacaataccca

SEQ ID NO: 540 - DNA, 20 bp, Artificial sequence
  Synthetic oligonucleotide
ggcaggcaagttacaggaag

SEQ ID NO: 541 - DNA, 20 bp, Artificial sequence
  Synthetic oligonucleotide
tcgcccactctggccccaaa

SEQ ID NO: 542 - DNA, 20 bp, Artificial sequence
  Synthetic oligonucleotide
cctcgcccactctggcccca

SEQ ID NO: 543 - DNA, 20 bp, Artificial sequence
  Synthetic oligonucleotide
cgcctcgcccactctggccc

SEQ ID NO: 544 - DNA, 20 bp, Artificial sequence
  Synthetic oligonucleotide
cgcgcctcgcccactctggc

SEQ ID NO: 545 - DNA, 20 bp, Artificial sequence
  Synthetic oligonucleotide
tccgcgcctcgcccactctg

SEQ ID NO: 546 - DNA, 20 bp, Artificial sequence
  Synthetic oligonucleotide
cctccgcgcctcgcccactc

SEQ ID NO: 547 - DNA, 20 bp, Artificial sequence
  Synthetic oligonucleotide
gacctccgcgcctcgcccac

SEQ ID NO: 548 - DNA, 20 bp, Artificial sequence
  Synthetic oligonucleotide
cagacctccgcgcctcgccc

SEQ ID NO: 549 - DNA, 20 bp, Artificial sequence
  Synthetic oligonucleotide
gccagacctccgcgcctcgc

SEQ ID NO: 550 - DNA, 20 bp, Artificial sequence
  Synthetic oligonucleotide
aggccagacctccgcgcctc

SEQ ID NO: 551 - DNA, 20 bp, Artificial sequence
  Synthetic oligonucleotide
ataggccagacctccgcgcc

SEQ ID NO: 552 - DNA, 20 bp, Artificial sequence
  Synthetic oligonucleotide
ttataggccagacctccgcg

SEQ ID NO: 553 - DNA, 20 bp, Artificial sequence
  Synthetic oligonucleotide
ctttataggccagacctccg

SEQ ID NO: 554 - DNA, 20 bp, Artificial sequence
  Synthetic oligonucleotide
tactttataggccagacctc

SEQ ID NO: 555 - DNA, 20 bp, Artificial sequence
  Synthetic oligonucleotide
actactttataggccagacc

SEQ ID NO: 556 - DNA, 20 bp, Artificial sequence
  Synthetic oligonucleotide
cgactactttataggccaga

SEQ ID NO: 557 - DNA, 20 bp, Artificial sequence
  Synthetic oligonucleotide
cgcgactactttataggcca

SEQ ID NO: 558 - DNA, 20 bp, Artificial sequence
  Synthetic oligonucleotide
tccgcgactactttataggc

SEQ ID NO: 559 - DNA, 20 bp, Artificial sequence
  Synthetic oligonucleotide
tctccgcgactactttatag

SEQ ID NO: 560 - DNA, 20 bp, Artificial sequence
  Synthetic oligonucleotide
cgtctccgcgactactttat

SEQ ID NO: 561 - DNA, 20 bp, Artificial sequence
  Synthetic oligonucleotide
cccgtctccgcgactacttt

SEQ ID NO: 562 - DNA, 20 bp, Artificial sequence
  Synthetic oligonucleotide
accccgtctccgcgactact

SEQ ID NO: 563 - DNA, 20 bp, Artificial sequence
  Synthetic oligonucleotide
gcaccccgtctccgcgacta

SEQ ID NO: 564 - DNA, 20 bp, Artificial sequence
  Synthetic oligonucleotide
cagcaccccgtctccgcgac

SEQ ID NO: 565 - DNA, 20 bp, Artificial sequence
  Synthetic oligonucleotide
accagcaccccgtctccgcg

SEQ ID NO: 566 - DNA, 20 bp, Artificial sequence
  Synthetic oligonucleotide
aaaccagcaccccgtctccg

SEQ ID NO: 567 - DNA, 20 bp, Artificial sequence
  Synthetic oligonucleotide
gcaaaccagcaccccgtctc

SEQ ID NO: 568 - DNA, 20 bp, Artificial sequence
  Synthetic oligonucleotide
acgcaaaccagcaccccgtc

SEQ ID NO: 569 - DNA, 20 bp, Artificial sequence
  Synthetic oligonucleotide
cgacgcaaaccagcaccccg

SEQ ID NO: 570 - DNA, 20 bp, Artificial sequence
  Synthetic oligonucleotide
tacgacgcaaaccagcaccc

SEQ ID NO: 571 - DNA, 20 bp, Artificial sequence
  Synthetic oligonucleotide
actacgacgcaaaccagcac

SEQ ID NO: 572 - DNA, 20 bp, Artificial sequence
  Synthetic oligonucleotide
agactacgacgcaaaccagc

SEQ ID NO: 573 - DNA, 20 bp, Artificial sequence
  Synthetic oligonucleotide
ggagactacgacgcaaacca

SEQ ID NO: 574 - DNA, 20 bp, Artificial sequence
  Synthetic oligonucleotide
caggagactacgacgcaaac

SEQ ID NO: 575 - DNA, 20 bp, Artificial sequence
  Synthetic oligonucleotide
tgcaggagactacgacgcaa

SEQ ID NO: 576 - DNA, 20 bp, Artificial sequence
  Synthetic oligonucleotide
gctgcaggagactacgacgc

SEQ ID NO: 577 - DNA, 20 bp, Artificial sequence
  Synthetic oligonucleotide
gcaacggaaaccccagacgc

SEQ ID NO: 578 - DNA, 20 bp, Artificial sequence
  Synthetic oligonucleotide
ctgcaacggaaaccccagac

SEQ ID NO: 579 - DNA, 20 bp, Artificial sequence
  Synthetic oligonucleotide
gactgcaacggaaaccccag

SEQ ID NO: 580 - DNA, 20 bp, Artificial sequence
  Synthetic oligonucleotide
ggactgcaacggaaacccca

SEQ ID NO: 581 - DNA, 20 bp, Artificial sequence
  Synthetic oligonucleotide
aggactgcaacggaaacccc

SEQ ID NO: 582 - DNA, 20 bp, Artificial sequence
  Synthetic oligonucleotide
tccgaggactgcaacggaaa

SEQ ID NO: 583 - DNA, 20 bp, Artificial sequence
  Synthetic oligonucleotide
gttccgaggactgcaacgga

SEQ ID NO: 584 - DNA, 20 bp, Artificial sequence
  Synthetic oligonucleotide
tggttccgaggactgcaacg

SEQ ID NO: 585 - DNA, 20 bp, Artificial sequence
  Synthetic oligonucleotide
cctggttccgaggactgcaa

SEQ ID NO: 586 - DNA, 20 bp, Artificial sequence
  Synthetic oligonucleotide
gtcctggttccgaggactgc

SEQ ID NO: 587 - DNA, 20 bp, Artificial sequence
  Synthetic oligonucleotide
aggtcctggttccgaggact

SEQ ID NO: 588 - DNA, 20 bp, Artificial sequence
  Synthetic oligonucleotide
cgaggtcctggttccgagga

SEQ ID NO: 589 - DNA, 20 bp, Artificial sequence
  Synthetic oligonucleotide
gccgaggtcctggttccgag

SEQ ID NO: 590 - DNA, 20 bp, Artificial sequence
  Synthetic oligonucleotide
acgccgaggtcctggttccg

SEQ ID NO: 591 - DNA, 20 bp, Artificial sequence
  Synthetic oligonucleotide
ccacgccgaggtcctggttc

SEQ ID NO: 592 - DNA, 20 bp, Artificial sequence
  Synthetic oligonucleotide
ggccacgccgaggtcctggt

SEQ ID NO: 593 - DNA, 20 bp, Artificial sequence
  Synthetic oligonucleotide
gctaggccacgccgaggtcc

SEQ ID NO: 594 - DNA, 20 bp, Artificial sequence
  Synthetic oligonucleotide
tcgctaggccacgccgaggt

SEQ ID NO: 595 - DNA, 20 bp, Artificial sequence
  Synthetic oligonucleotide
actcgctaggccacgccgag

SEQ ID NO: 596 - DNA, 20 bp, Artificial sequence
  Synthetic oligonucleotide
taactcgctaggccacgccg

SEQ ID NO: 597 - DNA, 20 bp, Artificial sequence
  Synthetic oligonucleotide
cataactcgctaggccacgc

SEQ ID NO: 598 - DNA, 20 bp, Artificial sequence
  Synthetic oligonucleotide
gccataactcgctaggccac

SEQ ID NO: 599 - DNA, 20 bp, Artificial sequence
  Synthetic oligonucleotide
tcgccataactcgctaggcc

SEQ ID NO: 600 - DNA, 20 bp, Artificial sequence
  Synthetic oligonucleotide
cgtcgccataactcgctagg

SEQ ID NO: 601 - DNA, 20 bp, Artificial sequence
  Synthetic oligonucleotide
cagcacgcacacggccttcg

SEQ ID NO: 602 - DNA, 20 bp, Artificial sequence
  Synthetic oligonucleotide
gccgtcgcccttcagcacgc

SEQ ID NO: 603 - DNA, 20 bp, Artificial sequence
  Synthetic oligonucleotide
ggccgtcgcccttcagcacg

SEQ ID NO: 604 - DNA, 20 bp, Artificial sequence
  Synthetic oligonucleotide
gggccgtcgcccttcagcac

SEQ ID NO: 605 - DNA, 20 bp, Artificial sequence
  Synthetic oligonucleotide
ctgggccgtcgcccttcagc

SEQ ID NO: 606 - DNA, 20 bp, Artificial sequence
  Synthetic oligonucleotide
cactgggccgtcgcccttca

SEQ ID NO: 607 - DNA, 20 bp, Artificial sequence
  Synthetic oligonucleotide
tgcactgggccgtcgccctt

SEQ ID NO: 608 - DNA, 20 bp, Artificial sequence
  Synthetic oligonucleotide
cctgcactgggccgtcgccc

SEQ ID NO: 609 - DNA, 20 bp, Artificial sequence
  Synthetic oligonucleotide
atgccctgcactgggccgtc

SEQ ID NO: 610 - DNA, 20 bp, Artificial sequence
  Synthetic oligonucleotide
tgatgccctgcactgggccg

SEQ ID NO: 611 - DNA, 20 bp, Artificial sequence
  Synthetic oligonucleotide
gatgatgccctgcactgggc

SEQ ID NO: 612 - DNA, 20 bp, Artificial sequence
  Synthetic oligonucleotide
ttgatgatgccctgcactgg

SEQ ID NO: 613 - DNA, 18 bp, Artificial sequence
  Synthetic oligonucleotide
ggcgatcccaattacacc

SEQ ID NO: 614 - DNA, 20 bp, Artificial sequence
  Synthetic oligonucleotide
tcgaaattgatgatgccctg

SEQ ID NO: 615 - DNA, 20 bp, Artificial sequence
  Synthetic oligonucleotide
gctcgaaattgatgatgccc

SEQ ID NO: 616 - DNA, 20 bp, Artificial sequence
  Synthetic oligonucleotide
ctgctcgaaattgatgatgc

SEQ ID NO: 617 - DNA, 20 bp, Artificial sequence
  Synthetic oligonucleotide
ttctgctcgaaattgatgat

SEQ ID NO: 618 - DNA, 20 bp, Artificial sequence
  Synthetic oligonucleotide
ttaatgcttccccacacctt

SEQ ID NO: 619 - DNA, 20 bp, Artificial sequence
  Synthetic oligonucleotide
ctttaatgcttccccacacc

SEQ ID NO: 620 - DNA, 20 bp, Artificial sequence
  Synthetic oligonucleotide
tcctttaatgcttccccaca

SEQ ID NO: 621 - DNA, 20 bp, Artificial sequence
  Synthetic oligonucleotide
tcagtcctttaatgcttccc

SEQ ID NO: 622 - DNA, 20 bp, Artificial sequence
  Synthetic oligonucleotide
agtcagtcctttaatgcttc

SEQ ID NO: 623 - DNA, 20 bp, Artificial sequence
  Synthetic oligonucleotide
tcagtcagtcctttaatgct

SEQ ID NO: 624 - DNA, 20 bp, Artificial sequence
  Synthetic oligonucleotide
cttcagtcagtcctttaatg

SEQ ID NO: 625 - DNA, 20 bp, Artificial sequence
  Synthetic oligonucleotide
gccttcagtcagtcctttaa

SEQ ID NO: 626 - DNA, 20 bp, Artificial sequence
  Synthetic oligonucleotide
gcaggccttcagtcagtcct

SEQ ID NO: 627 - DNA, 20 bp, Artificial sequence
  Synthetic oligonucleotide
atgcaggccttcagtcagtc

SEQ ID NO: 628 - DNA, 20 bp, Artificial sequence
  Synthetic oligonucleotide
ccatgcaggccttcagtcag

SEQ ID NO: 629 - DNA, 20 bp, Artificial sequence
  Synthetic oligonucleotide
catgaacatggaatccatgc

SEQ ID NO: 630 - DNA, 20 bp, Artificial sequence
  Synthetic oligonucleotide
ctcatgaacatggaatccat

SEQ ID NO: 631 - DNA, 20 bp, Artificial sequence
  Synthetic oligonucleotide
aactcatgaacatggaatcc

SEQ ID NO: 632 - DNA, 20 bp, Artificial sequence
  Synthetic oligonucleotide
ccaaactcatgaacatggaa

SEQ ID NO: 633 - DNA, 20 bp, Artificial sequence
  Synthetic oligonucleotide
ctccaaactcatgaacatgg

SEQ ID NO: 634 - DNA, 20 bp, Artificial sequence
  Synthetic oligonucleotide
atctccaaactcatgaacat

SEQ ID NO: 635 - DNA, 20 bp, Artificial sequence
  Synthetic oligonucleotide
ttatctccaaactcatgaac

SEQ ID NO: 636 - DNA, 20 bp, Artificial sequence
  Synthetic oligonucleotide
tattatctccaaactcatga

SEQ ID NO: 637 - DNA, 20 bp, Artificial sequence
  Synthetic oligonucleotide
tgtattatctccaaactcat

SEQ ID NO: 638 - DNA, 20 bp, Artificial sequence
  Synthetic oligonucleotide
ctgctgtattatctccaaac

SEQ ID NO: 639 - DNA, 20 bp, Artificial sequence
  Synthetic oligonucleotide
gcctgctgtattatctccaa

SEQ ID NO: 640 - DNA, 20 bp, Artificial sequence
  Synthetic oligonucleotide
cagcctgctgtattatctcc

SEQ ID NO: 641 - DNA, 20 bp, Artificial sequence
  Synthetic oligonucleotide
tacagcctgctgtattatct

SEQ ID NO: 642 - DNA, 20 bp, Artificial sequence
  Synthetic oligonucleotide
ggtacagcctgctgtattat

SEQ ID NO: 643 - DNA, 20 bp, Artificial sequence
  Synthetic oligonucleotide
ctggtacagcctgctgtatt

SEQ ID NO: 644 - DNA, 20 bp, Artificial sequence
  Synthetic oligonucleotide
cactggtacagcctgctgta

SEQ ID NO: 645 - DNA, 20 bp, Artificial sequence
  Synthetic oligonucleotide
tgcactggtacagcctgctg

SEQ ID NO: 646 - DNA, 20 bp, Artificial sequence
  Synthetic oligonucleotide
cctgcactggtacagcctgc

SEQ ID NO: 647 - DNA, 20 bp, Artificial sequence
  Synthetic oligonucleotide
ttctggatagaggattaaag

SEQ ID NO: 648 - DNA, 20 bp, Artificial sequence
  Synthetic oligonucleotide
ttttctggatagaggattaa

SEQ ID NO: 649 - DNA, 20 bp, Artificial sequence
  Synthetic oligonucleotide
tgttttctggatagaggatt

SEQ ID NO: 650 - DNA, 20 bp, Artificial sequence
  Synthetic oligonucleotide
cgtgttttctggatagagga

SEQ ID NO: 651 - DNA, 20 bp, Artificial sequence
  Synthetic oligonucleotide
accgtgttttctggatagag

SEQ ID NO: 652 - DNA, 20 bp, Artificial sequence
  Synthetic oligonucleotide
ccaccgtgttttctggatag

SEQ ID NO: 653 - DNA, 20 bp, Artificial sequence
  Synthetic oligonucleotide
gcccaccgtgttttctggat

SEQ ID NO: 654 - DNA, 20 bp, Artificial sequence
  Synthetic oligonucleotide
tggcccaccgtgttttctgg

SEQ ID NO: 655 - DNA, 20 bp, Artificial sequence
  Synthetic oligonucleotide
tttggcccaccgtgttttct

SEQ ID NO: 656 - DNA, 20 bp, Artificial sequence
  Synthetic oligonucleotide
cctttggcccaccgtgtttt

SEQ ID NO: 657 - DNA, 20 bp, Artificial sequence
  Synthetic oligonucleotide
agtctccaacatgcctctct

SEQ ID NO: 658 - DNA, 20 bp, Artificial sequence
  Synthetic oligonucleotide
caagtctccaacatgcctct

SEQ ID NO: 659 - DNA, 20 bp, Artificial sequence
  Synthetic oligonucleotide
cccaagtctccaacatgcct

SEQ ID NO: 660 - DNA, 20 bp, Artificial sequence
  Synthetic oligonucleotide
attgcccaagtctccaacat

SEQ ID NO: 661 - DNA, 20 bp, Artificial sequence
  Synthetic oligonucleotide
acattgcccaagtctccaac

SEQ ID NO: 662 - DNA, 20 bp, Artificial sequence
  Synthetic oligonucleotide
tcacattgcccaagtctcca

SEQ ID NO: 663 - DNA, 20 bp, Artificial sequence
  Synthetic oligonucleotide
agtcacattgcccaagtctc

SEQ ID NO: 664 - DNA, 20 bp, Artificial sequence
  Synthetic oligonucleotide
gcagtcacattgcccaagtc

SEQ ID NO: 665 - DNA, 20 bp, Artificial sequence
  Synthetic oligonucleotide
cagcagtcacattgcccaag

SEQ ID NO: 666 - DNA, 20 bp, Artificial sequence
  Synthetic oligonucleotide
gtcagcagtcacattgccca

SEQ ID NO: 667 - DNA, 20 bp, Artificial sequence
  Synthetic oligonucleotide
ttgtcagcagtcacattgcc

SEQ ID NO: 668 - DNA, 20 bp, Artificial sequence
  Synthetic oligonucleotide
ctttgtcagcagtcacattg

SEQ ID NO: 669 - DNA, 20 bp, Artificial sequence
  Synthetic oligonucleotide
atctttgtcagcagtcacat

SEQ ID NO: 670 - DNA, 20 bp, Artificial sequence
  Synthetic oligonucleotide
ccatctttgtcagcagtcac

SEQ ID NO: 671 - DNA, 20 bp, Artificial sequence
  Synthetic oligonucleotide
caccatctttgtcagcagtc

SEQ ID NO: 672 - DNA, 20 bp, Artificial sequence
  Synthetic oligonucleotide
cacaccatctttgtcagcag

SEQ ID NO: 673 - DNA, 20 bp, Artificial sequence
  Synthetic oligonucleotide
gccacaccatctttgtcagc

SEQ ID NO: 674 - DNA, 20 bp, Artificial sequence
  Synthetic oligonucleotide
cggccacaccatctttgtca

SEQ ID NO: 675 - DNA, 20 bp, Artificial sequence
  Synthetic oligonucleotide
atcggccacaccatctttgt

SEQ ID NO: 676 - DNA, 20 bp, Artificial sequence
  Synthetic oligonucleotide
acatcggccacaccatcttt

SEQ ID NO: 677 - DNA, 20 bp, Artificial sequence
  Synthetic oligonucleotide
agacacatcggccacaccat

SEQ ID NO: 678 - DNA, 20 bp, Artificial sequence
  Synthetic oligonucleotide
atagacacatcggccacacc

SEQ ID NO: 679 - DNA, 20 bp, Artificial sequence
  Synthetic oligonucleotide
caatagacacatcggccaca

SEQ ID NO: 680 - DNA, 20 bp, Artificial sequence
  Synthetic oligonucleotide
ttcaatagacacatcggcca

SEQ ID NO: 681 - DNA, 20 bp, Artificial sequence
  Synthetic oligonucleotide
tcttcaatagacacatcggc

SEQ ID NO: 682 - DNA, 20 bp, Artificial sequence
  Synthetic oligonucleotide
aatcttcaatagacacatcg

SEQ ID NO: 683 - DNA, 20 bp, Artificial sequence
  Synthetic oligonucleotide
agaatcttcaatagacacat

SEQ ID NO: 684 - DNA, 20 bp, Artificial sequence
  Synthetic oligonucleotide
acagaatcttcaatagacac

SEQ ID NO: 685 - DNA, 20 bp, Artificial sequence
  Synthetic oligonucleotide
tcacagaatcttcaatagac

SEQ ID NO: 686 - DNA, 20 bp, Artificial sequence
  Synthetic oligonucleotide
gatcacagaatcttcaatag

SEQ ID NO: 687 - DNA, 20 bp, Artificial sequence
  Synthetic oligonucleotide
gagatcacagaatcttcaat

SEQ ID NO: 688 - DNA, 20 bp, Artificial sequence
  Synthetic oligonucleotide
gtgagatcacagaatcttca

SEQ ID NO: 689 - DNA, 20 bp, Artificial sequence
  Synthetic oligonucleotide
gagtgagatcacagaatctt

SEQ ID NO: 690 - DNA, 20 bp, Artificial sequence
  Synthetic oligonucleotide
gagagtgagatcacagaatc

SEQ ID NO: 691 - DNA, 20 bp, Artificial sequence
  Synthetic oligonucleotide
ctgagagtgagatcacagaa

SEQ ID NO: 692 - DNA, 20 bp, Artificial sequence
  Synthetic oligonucleotide
tcctgagagtgagatcacag

SEQ ID NO: 693 - DNA, 20 bp, Artificial sequence
  Synthetic oligonucleotide
ggtctcctgagagtgagatc

SEQ ID NO: 694 - DNA, 20 bp, Artificial sequence
  Synthetic oligonucleotide
atggtctcctgagagtgaga

SEQ ID NO: 695 - DNA, 20 bp, Artificial sequence
  Synthetic oligonucleotide
caatggtctcctgagagtga

SEQ ID NO: 696 - DNA, 20 bp, Artificial sequence
  Synthetic oligonucleotide
tgcaatggtctcctgagagt

SEQ ID NO: 697 - DNA, 20 bp, Artificial sequence
  Synthetic oligonucleotide
gatgcaatggtctcctgaga

SEQ ID NO: 698 - DNA, 20 bp, Artificial sequence
  Synthetic oligonucleotide
atgatgcaatggtctcctga

SEQ ID NO: 699 - DNA, 20 bp, Artificial sequence
  Synthetic oligonucleotide
caatgatgcaatggtctcct

SEQ ID NO: 700 - DNA, 20 bp, Artificial sequence
  Synthetic oligonucleotide
gccaatgatgcaatggtctc

SEQ ID NO: 701 - DNA, 20 bp, Artificial sequence
  Synthetic oligonucleotide
cggccaatgatgcaatggtc

SEQ ID NO: 702 - DNA, 20 bp, Artificial sequence
  Synthetic oligonucleotide
tgcggccaatgatgcaatgg

SEQ ID NO: 703 - DNA, 20 bp, Artificial sequence
  Synthetic oligonucleotide
tgtgcggccaatgatgcaat

SEQ ID NO: 704 - DNA, 20 bp, Artificial sequence
  Synthetic oligonucleotide
agtgtgcggccaatgatgca

SEQ ID NO: 705 - DNA, 20 bp, Artificial sequence
  Synthetic oligonucleotide
ccagtgtgcggccaatgatg

SEQ ID NO: 706 - DNA, 20 bp, Artificial sequence
  Synthetic oligonucleotide
caccagtgtgcggccaatga

SEQ ID NO: 707 - DNA, 20 bp, Artificial sequence
  Synthetic oligonucleotide
ggaccaccagtgtgcggcca

SEQ ID NO: 708 - DNA, 20 bp, Artificial sequence
  Synthetic oligonucleotide
atggaccaccagtgtgcggc

SEQ ID NO: 709 - DNA, 20 bp, Artificial sequence
  Synthetic oligonucleotide
tttcatggaccaccagtgtg

SEQ ID NO: 710 - DNA, 20 bp, Artificial sequence
  Synthetic oligonucleotide
tttttcatggaccaccagtg

SEQ ID NO: 711 - DNA, 20 bp, Artificial sequence
  Synthetic oligonucleotide
gctttttcatggaccaccag

SEQ ID NO: 712 - DNA, 20 bp, Artificial sequence
  Synthetic oligonucleotide
tgtctttgtactttcttcat

SEQ ID NO: 713 - DNA, 20 bp, Artificial sequence
  Synthetic oligonucleotide
cctgtctttgtactttcttc

SEQ ID NO: 714 - DNA, 20 bp, Artificial sequence
  Synthetic oligonucleotide
ttcctgtctttgtactttct

SEQ ID NO: 715 - DNA, 20 bp, Artificial sequence
  Synthetic oligonucleotide
gtttcctgtctttgtacttt

SEQ ID NO: 716 - DNA, 20 bp, Artificial sequence
  Synthetic oligonucleotide
aagccaaacgacttccagcg

SEQ ID NO: 717 - DNA, 20 bp, Artificial sequence
  Synthetic oligonucleotide
acaagccaaacgacttccag

SEQ ID NO: 718 - DNA, 20 bp, Artificial sequence
  Synthetic oligonucleotide
ccacaagccaaacgacttcc

SEQ ID NO: 719 - DNA, 20 bp, Artificial sequence
  Synthetic oligonucleotide
caccacaagccaaacgactt

SEQ ID NO: 720 - DNA, 20 bp, Artificial sequence
  Synthetic oligonucleotide
tacaccacaagccaaacgac

SEQ ID NO: 721 - DNA, 20 bp, Artificial sequence
  Synthetic oligonucleotide
attacaccacaagccaaacg

SEQ ID NO: 722 - DNA, 20 bp, Artificial sequence
  Synthetic oligonucleotide
caattacaccacaagccaaa

SEQ ID NO: 723 - DNA, 20 bp, Artificial sequence
  Synthetic oligonucleotide
aggataacagatgagttaag

SEQ ID NO: 724 - DNA, 20 bp, Artificial sequence
  Synthetic oligonucleotide
ggatacatttctacagctag

SEQ ID NO: 725 - DNA, 20 bp, Artificial sequence
  Synthetic oligonucleotide
caggatacatttctacagct

SEQ ID NO: 726 - DNA, 20 bp, Artificial sequence
  Synthetic oligonucleotide
atcaggatacatttctacag

SEQ ID NO: 727 - DNA, 20 bp, Artificial sequence
  Synthetic oligonucleotide
ttatcaggatacatttctac

SEQ ID NO: 728 - DNA, 20 bp, Artificial sequence
  Synthetic oligonucleotide
gtttatcaggatacatttct

SEQ ID NO: 729 - DNA, 20 bp, Artificial sequence
  Synthetic oligonucleotide
atgtttatcaggatacattt

SEQ ID NO: 730 - DNA, 20 bp, Artificial sequence
  Synthetic oligonucleotide
taatgtttatcaggatacat

SEQ ID NO: 731 - DNA, 20 bp, Artificial sequence
  Synthetic oligonucleotide
tttaatgtttatcaggatac

SEQ ID NO: 732 - DNA, 20 bp, Artificial sequence
  Synthetic oligonucleotide
tgtttaatgtttatcaggat

SEQ ID NO: 733 - DNA, 20 bp, Artificial sequence
  Synthetic oligonucleotide
agtgtttaatgtttatcagg

SEQ ID NO: 734 - DNA, 20 bp, Artificial sequence
  Synthetic oligonucleotide
tttaagattacagtgtttaa

SEQ ID NO: 735 - DNA, 20 bp, Artificial sequence
  Synthetic oligonucleotide
cttttaagattacagtgttt

SEQ ID NO: 736 - DNA, 20 bp, Artificial sequence
  Synthetic oligonucleotide
cacttttaagattacagtgt

SEQ ID NO: 737 - DNA, 20 bp, Artificial sequence
  Synthetic oligonucleotide
tacacttttaagattacagt

SEQ ID NO: 738 - DNA, 20 bp, Artificial sequence
  Synthetic oligonucleotide
attacacttttaagattaca

SEQ ID NO: 739 - DNA, 20 bp, Artificial sequence
  Synthetic oligonucleotide
caattacacttttaagatta

SEQ ID NO: 740 - DNA, 20 bp, Artificial sequence
  Synthetic oligonucleotide
cacacaattacacttttaag

SEQ ID NO: 741 - DNA, 20 bp, Artificial sequence
  Synthetic oligonucleotide
gtcacacaattacactttta

SEQ ID NO: 742 - DNA, 20 bp, Artificial sequence
  Synthetic oligonucleotide
aagtcacacaattacacttt

SEQ ID NO: 743 - DNA, 20 bp, Artificial sequence
  Synthetic oligonucleotide
aaaagtcacacaattacact

SEQ ID NO: 744 - DNA, 20 bp, Artificial sequence
  Synthetic oligonucleotide
gaaaaagtcacacaattaca

SEQ ID NO: 745 - DNA, 20 bp, Artificial sequence
  Synthetic oligonucleotide
ctgaaaaagtcacacaatta

SEQ ID NO: 746 - DNA, 20 bp, Artificial sequence
  Synthetic oligonucleotide
ctctgaaaaagtcacacaat

SEQ ID NO: 747 - DNA, 20 bp, Artificial sequence
  Synthetic oligonucleotide
aactctgaaaaagtcacaca

SEQ ID NO: 748 - DNA, 20 bp, Artificial sequence
  Synthetic oligonucleotide
gcaactctgaaaaagtcaca

SEQ ID NO: 749 - DNA, 20 bp, Artificial sequence
  Synthetic oligonucleotide
aagcaactctgaaaaagtca

SEQ ID NO: 750 - DNA, 20 bp, Artificial sequence
  Synthetic oligonucleotide
ttaaagcaactctgaaaaag

SEQ ID NO: 751 - DNA, 20 bp, Artificial sequence
  Synthetic oligonucleotide
ctttaaagcaactctgaaaa

SEQ ID NO: 752 - DNA, 20 bp, Artificial sequence
  Synthetic oligonucleotide
tactttaaagcaactctgaa

SEQ ID NO: 753 - DNA, 20 bp, Artificial sequence
  Synthetic oligonucleotide
ggtactttaaagcaactctg

SEQ ID NO: 754 - DNA, 20 bp, Artificial sequence
  Synthetic oligonucleotide
caggtactttaaagcaactc

SEQ ID NO: 755 - DNA, 20 bp, Artificial sequence
  Synthetic oligonucleotide
tacaggtactttaaagcaac

SEQ ID NO: 756 - DNA, 20 bp, Artificial sequence
  Synthetic oligonucleotide
actacaggtactttaaagca

SEQ ID NO: 757 - DNA, 20 bp, Artificial sequence
  Synthetic oligonucleotide
tcactacaggtactttaaag

SEQ ID NO: 758 - DNA, 20 bp, Artificial sequence
  Synthetic oligonucleotide
tctcactacaggtactttaa

SEQ ID NO: 759 - DNA, 20 bp, Artificial sequence
  Synthetic oligonucleotide
tttctcactacaggtacttt

SEQ ID NO: 760 - DNA, 20 bp, Artificial sequence
  Synthetic oligonucleotide
agtttctcactacaggtact

SEQ ID NO: 761 - DNA, 20 bp, Artificial sequence
  Synthetic oligonucleotide
tcagtttctcactacaggta

SEQ ID NO: 762 - DNA, 20 bp, Artificial sequence
  Synthetic oligonucleotide
taaatcagtttctcactaca

SEQ ID NO: 763 - DNA, 20 bp, Artificial sequence
  Synthetic oligonucleotide
atcataaatcagtttctcac

SEQ ID NO: 764 - DNA, 20 bp, Artificial sequence
  Synthetic oligonucleotide
tgatcataaatcagtttctc

SEQ ID NO: 765 - DNA, 20 bp, Artificial sequence
  Synthetic oligonucleotide
agtgatcataaatcagtttc

SEQ ID NO: 766 - DNA, 20 bp, Artificial sequence
  Synthetic oligonucleotide
caagtgatcataaatcagtt

SEQ ID NO: 767 - DNA, 20 bp, Artificial sequence
  Synthetic oligonucleotide
tccaagtgatcataaatcag

SEQ ID NO: 768 - DNA, 20 bp, Artificial sequence
  Synthetic oligonucleotide
cttccaagtgatcataaatc

SEQ ID NO: 769 - DNA, 20 bp, Artificial sequence
  Synthetic oligonucleotide
atcttccaagtgatcataaa

SEQ ID NO: 770 - DNA, 20 bp, Artificial sequence
  Synthetic oligonucleotide
aaatcttccaagtgatcata

SEQ ID NO: 771 - DNA, 20 bp, Artificial sequence
  Synthetic oligonucleotide
ctgagttttataaaactata

SEQ ID NO: 772 - DNA, 20 bp, Artificial sequence
  Synthetic oligonucleotide
ttaactgagttttataaaac

SEQ ID NO: 773 - DNA, 20 bp, Artificial sequence
  Synthetic oligonucleotide
ttttaactgagttttataaa

SEQ ID NO: 774 - DNA, 20 bp, Artificial sequence
  Synthetic oligonucleotide
cattttaactgagttttata

SEQ ID NO: 775 - DNA, 20 bp, Artificial sequence
  Synthetic oligonucleotide
gacattttaactgagtttta

SEQ ID NO: 776 - DNA, 20 bp, Artificial sequence
  Synthetic oligonucleotide
cagacattttaactgagttt

SEQ ID NO: 777 - DNA, 20 bp, Artificial sequence
  Synthetic oligonucleotide
aacagacattttaactgagt

SEQ ID NO: 778 - DNA, 20 bp, Artificial sequence
  Synthetic oligonucleotide
gaaacagacattttaactga

SEQ ID NO: 779 - DNA, 20 bp, Artificial sequence
  Synthetic oligonucleotide
ttgaaacagacattttaact

SEQ ID NO: 780 - DNA, 20 bp, Artificial sequence
  Synthetic oligonucleotide
tttaagtctggcaaaataca

SEQ ID NO: 781 - DNA, 20 bp, Artificial sequence
  Synthetic oligonucleotide
gatttaagtctggcaaaata

SEQ ID NO: 782 - DNA, 20 bp, Artificial sequence
  Synthetic oligonucleotide
gtgatttaagtctggcaaaa

SEQ ID NO: 783 - DNA, 20 bp, Artificial sequence
  Synthetic oligonucleotide
ctgtgatttaagtctggcaa

SEQ ID NO: 784 - DNA, 20 bp, Artificial sequence
  Synthetic oligonucleotide
atctgtgatttaagtctggc

SEQ ID NO: 785 - DNA, 20 bp, Artificial sequence
  Synthetic oligonucleotide
acccatctgtgatttaagtc

SEQ ID NO: 786 - DNA, 20 bp, Artificial sequence
  Synthetic oligonucleotide
atacccatctgtgatttaag

SEQ ID NO: 787 - DNA, 20 bp, Artificial sequence
  Synthetic oligonucleotide
taatacccatctgtgattta

SEQ ID NO: 788 - DNA, 20 bp, Artificial sequence
  Synthetic oligonucleotide
aaagaaattctgacaagttt

SEQ ID NO: 789 - DNA, 20 bp, Artificial sequence
  Synthetic oligonucleotide
acaaagaaattctgacaagt

SEQ ID NO: 790 - DNA, 20 bp, Artificial sequence
  Synthetic oligonucleotide
tgacaaagaaattctgacaa

SEQ ID NO: 791 - DNA, 20 bp, Artificial sequence
  Synthetic oligonucleotide
aatgacaaagaaattctgac

SEQ ID NO: 792 - DNA, 20 bp, Artificial sequence
  Synthetic oligonucleotide
tgaatgacaaagaaattctg

SEQ ID NO: 793 - DNA, 20 bp, Artificial sequence
  Synthetic oligonucleotide
cttgaatgacaaagaaattc

SEQ ID NO: 794 - DNA, 20 bp, Artificial sequence
  Synthetic oligonucleotide
ggcttgaatgacaaagaaat

SEQ ID NO: 795 - DNA, 20 bp, Artificial sequence
  Synthetic oligonucleotide
caggcttgaatgacaaagaa

SEQ ID NO: 796 - DNA, 20 bp, Artificial sequence
  Synthetic oligonucleotide
cacaggcttgaatgacaaag

SEQ ID NO: 797 - DNA, 20 bp, Artificial sequence
  Synthetic oligonucleotide
ttcacaggcttgaatgacaa

SEQ ID NO: 798 - DNA, 20 bp, Artificial sequence
  Synthetic oligonucleotide
tattcacaggcttgaatgac

SEQ ID NO: 799 - DNA, 20 bp, Artificial sequence
  Synthetic oligonucleotide
ataagtgccatacagggttt

SEQ ID NO: 800 - DNA, 20 bp, Artificial sequence
  Synthetic oligonucleotide
cataataagtgccatacagg

SEQ ID NO: 801 - DNA, 20 bp, Artificial sequence
  Synthetic oligonucleotide
tagcctcataataagtgcca

SEQ ID NO: 802 - DNA, 20 bp, Artificial sequence
  Synthetic oligonucleotide
aatagcctcataataagtgc

SEQ ID NO: 803 - DNA, 20 bp, Artificial sequence
  Synthetic oligonucleotide
ttaatagcctcataataagt

SEQ ID NO: 804 - DNA, 20 bp, Artificial sequence
  Synthetic oligonucleotide
tcttttaatagcctcataat

SEQ ID NO: 805 - DNA, 20 bp, Artificial sequence
  Synthetic oligonucleotide
attcttttaatagcctcata

SEQ ID NO: 806 - DNA, 20 bp, Artificial sequence
  Synthetic oligonucleotide
ttggattcttttaatagcct

SEQ ID NO: 807 - DNA, 20 bp, Artificial sequence
  Synthetic oligonucleotide
atttggattcttttaatagc

SEQ ID NO: 808 - DNA, 20 bp, Artificial sequence
  Synthetic oligonucleotide
gaatttggattcttttaata

SEQ ID NO: 809 - DNA, 20 bp, Artificial sequence
  Synthetic oligonucleotide
ttgaatttggattcttttaa

SEQ ID NO: 810 - DNA, 20 bp, Artificial sequence
  Synthetic oligonucleotide
gtttgaatttggattctttt

SEQ ID NO: 811 - DNA, 20 bp, Artificial sequence
  Synthetic oligonucleotide
tagtttgaatttggattctt

SEQ ID NO: 812 - DNA, 20 bp, Artificial sequence
  Synthetic oligonucleotide
tttagtttgaatttggattc

SEQ ID NO: 813 - DNA, 20 bp, Artificial sequence
  Synthetic oligonucleotide
tttttagtttgaatttggat

SEQ ID NO: 814 - DNA, 20 bp, Artificial sequence
  Synthetic oligonucleotide
tttttttagtttgaatttgg

SEQ ID NO: 815 - DNA, 20 bp, Artificial sequence
  Synthetic oligonucleotide
cgtttcctgtctttgtactt

SEQ ID NO: 816 - DNA, 20 bp, Artificial sequence
  Synthetic oligonucleotide
caagccaaacgacttccagc

SEQ ID NO: 817 - DNA, 20 bp, Artificial sequence
  Synthetic oligonucleotide
cacaagccaaacgacttcca

SEQ ID NO: 818 - DNA, 20 bp, Artificial sequence
  Synthetic oligonucleotide
accacaagccaaacgacttc

SEQ ID NO: 819 - DNA, 20 bp, Artificial sequence
  Synthetic oligonucleotide
acaccacaagccaaacgact

SEQ ID NO: 820 - DNA, 20 bp, Artificial sequence
  Synthetic oligonucleotide
ttacaccacaagccaaacga

SEQ ID NO: 821 - DNA, 20 bp, Artificial sequence
  Synthetic oligonucleotide
ggataacagatgagttaagg

SEQ ID NO: 822 - DNA, 20 bp, Artificial sequence
  Synthetic oligonucleotide
aggatacatttctacagcta

SEQ ID NO: 823 - DNA, 20 bp, Artificial sequence
  Synthetic oligonucleotide
tcaggatacatttctacagc

SEQ ID NO: 824 - DNA, 20 bp, Artificial sequence
  Synthetic oligonucleotide
tatcaggatacatttctaca

SEQ ID NO: 825 - DNA, 20 bp, Artificial sequence
  Synthetic oligonucleotide
tgtttatcaggatacatttc

SEQ ID NO: 826 - DNA, 20 bp, Artificial sequence
  Synthetic oligonucleotide
aatgtttatcaggatacatt

SEQ ID NO: 827 - DNA, 20 bp, Artificial sequence
  Synthetic oligonucleotide
ttaatgtttatcaggataca

SEQ ID NO: 828 - DNA, 20 bp, Artificial sequence
  Synthetic oligonucleotide
gtttaatgtttatcaggata

SEQ ID NO: 829 - DNA, 20 bp, Artificial sequence
  Synthetic oligonucleotide
gtgtttaatgtttatcagga

SEQ ID NO: 830 - DNA, 20 bp, Artificial sequence
  Synthetic oligonucleotide
ttttaagattacagtgttta

SEQ ID NO: 831 - DNA, 20 bp, Artificial sequence
  Synthetic oligonucleotide
acttttaagattacagtgtt

SEQ ID NO: 832 - DNA, 20 bp, Artificial sequence
  Synthetic oligonucleotide
acacttttaagattacagtg

SEQ ID NO: 833 - DNA, 20 bp, Artificial sequence
  Synthetic oligonucleotide
ttacacttttaagattacag

SEQ ID NO: 834 - DNA, 20 bp, Artificial sequence
  Synthetic oligonucleotide
aattacacttttaagattac

SEQ ID NO: 835 - DNA, 20 bp, Artificial sequence
  Synthetic oligonucleotide
acacaattacacttttaaga

SEQ ID NO: 836 - DNA, 20 bp, Artificial sequence
  Synthetic oligonucleotide
tcacacaattacacttttaa

SEQ ID NO: 837 - DNA, 20 bp, Artificial sequence
  Synthetic oligonucleotide
aaagtcacacaattacactt

SEQ ID NO: 838 - DNA, 20 bp, Artificial sequence
  Synthetic oligonucleotide
tgaaaaagtcacacaattac

SEQ ID NO: 839 - DNA, 20 bp, Artificial sequence
  Synthetic oligonucleotide
tctgaaaaagtcacacaatt

SEQ ID NO: 840 - DNA, 20 bp, Artificial sequence
  Synthetic oligonucleotide
actctgaaaaagtcacacaa

SEQ ID NO: 841 - DNA, 20 bp, Artificial sequence
  Synthetic oligonucleotide
agcaactctgaaaaagtcac

SEQ ID NO: 842 - DNA, 20 bp, Artificial sequence
  Synthetic oligonucleotide
actttaaagcaactctgaaa

SEQ ID NO: 843 - DNA, 20 bp, Artificial sequence
  Synthetic oligonucleotide
gtactttaaagcaactctga

SEQ ID NO: 844 - DNA, 20 bp, Artificial sequence
  Synthetic oligonucleotide
aggtactttaaagcaactct

SEQ ID NO: 845 - DNA, 20 bp, Artificial sequence
  Synthetic oligonucleotide
cactacaggtactttaaagc

SEQ ID NO: 846 - DNA, 20 bp, Artificial sequence
  Synthetic oligonucleotide
ttctcactacaggtacttta

SEQ ID NO: 847 - DNA, 20 bp, Artificial sequence
  Synthetic oligonucleotide
gtttctcactacaggtactt

SEQ ID NO: 848 - DNA, 20 bp, Artificial sequence
  Synthetic oligonucleotide
cagtttctcactacaggtac

SEQ ID NO: 849 - DNA, 20 bp, Artificial sequence
  Synthetic oligonucleotide
atcagtttctcactacaggt

SEQ ID NO: 850 - DNA, 20 bp, Artificial sequence
  Synthetic oligonucleotide
aaatcagtttctcactacag

SEQ ID NO: 851 - DNA, 20 bp, Artificial sequence
  Synthetic oligonucleotide
tcataaatcagtttctcact

SEQ ID NO: 852 - DNA, 20 bp, Artificial sequence
  Synthetic oligonucleotide
gtgatcataaatcagtttct

SEQ ID NO: 853 - DNA, 20 bp, Artificial sequence
  Synthetic oligonucleotide
aagtgatcataaatcagttt

SEQ ID NO: 854 - DNA, 20 bp, Artificial sequence
  Synthetic oligonucleotide
ccaagtgatcataaatcagt

SEQ ID NO: 855 - DNA, 20 bp, Artificial sequence
  Synthetic oligonucleotide
ttccaagtgatcataaatca

SEQ ID NO: 856 - DNA, 20 bp, Artificial sequence
  Synthetic oligonucleotide
tcttccaagtgatcataaat

SEQ ID NO: 857 - DNA, 20 bp, Artificial sequence
  Synthetic oligonucleotide
taactgagttttataaaact

SEQ ID NO: 858 - DNA, 20 bp, Artificial sequence
  Synthetic oligonucleotide
aaacagacattttaactgag

SEQ ID NO: 859 - DNA, 20 bp, Artificial sequence
  Synthetic oligonucleotide
tgaaacagacattttaactg

SEQ ID NO: 860 - DNA, 20 bp, Artificial sequence
  Synthetic oligonucleotide
atttaagtctggcaaaatac

SEQ ID NO: 861 - DNA, 20 bp, Artificial sequence
  Synthetic oligonucleotide
tgtgatttaagtctggcaaa

SEQ ID NO: 862 - DNA, 20 bp, Artificial sequence
  Synthetic oligonucleotide
tctgtgatttaagtctggca

SEQ ID NO: 863 - DNA, 20 bp, Artificial sequence
  Synthetic oligonucleotide
catctgtgatttaagtctgg

SEQ ID NO: 864 - DNA, 20 bp, Artificial sequence
  Synthetic oligonucleotide
cccatctgtgatttaagtct

SEQ ID NO: 865 - DNA, 20 bp, Artificial sequence
  Synthetic oligonucleotide
tacccatctgtgatttaagt

SEQ ID NO: 866 - DNA, 20 bp, Artificial sequence
  Synthetic oligonucleotide
aatacccatctgtgatttaa

SEQ ID NO: 867 - DNA, 20 bp, Artificial sequence
  Synthetic oligonucleotide
ttaatacccatctgtgattt

SEQ ID NO: 868 - DNA, 20 bp, Artificial sequence
  Synthetic oligonucleotide
gacaaagaaattctgacaag

SEQ ID NO: 869 - DNA, 20 bp, Artificial sequence
  Synthetic oligonucleotide
gaatgacaaagaaattctga

SEQ ID NO: 870 - DNA, 20 bp, Artificial sequence
  Synthetic oligonucleotide
aggcttgaatgacaaagaaa

SEQ ID NO: 871 - DNA, 20 bp, Artificial sequence
  Synthetic oligonucleotide
taagtgccatacagggtttt

SEQ ID NO: 872 - DNA, 20 bp, Artificial sequence
  Synthetic oligonucleotide
ataataagtgccatacaggg

SEQ ID NO: 873 - DNA, 20 bp, Artificial sequence
  Synthetic oligonucleotide
cctcataataagtgccatac

SEQ ID NO: 874 - DNA, 20 bp, Artificial sequence
  Synthetic oligonucleotide
agcctcataataagtgccat

SEQ ID NO: 875 - DNA, 20 bp, Artificial sequence
  Synthetic oligonucleotide
atagcctcataataagtgcc

SEQ ID NO: 876 - DNA, 20 bp, Artificial sequence
  Synthetic oligonucleotide
cttttaatagcctcataata

SEQ ID NO: 877 - DNA, 20 bp, Artificial sequence
  Synthetic oligonucleotide
ttcttttaatagcctcataa

SEQ ID NO: 878 - DNA, 20 bp, Artificial sequence
  Synthetic oligonucleotide
gattcttttaatagcctcat

SEQ ID NO: 879 - DNA, 20 bp, Artificial sequence
  Synthetic oligonucleotide
tggattcttttaatagcctc

SEQ ID NO: 880 - DNA, 20 bp, Artificial sequence
  Synthetic oligonucleotide
tttggattcttttaatagcc

SEQ ID NO: 881 - DNA, 20 bp, Artificial sequence
  Synthetic oligonucleotide
aatttggattcttttaatag

SEQ ID NO: 882 - DNA, 20 bp, Artificial sequence
  Synthetic oligonucleotide
tgaatttggattcttttaat

SEQ ID NO: 883 - DNA, 20 bp, Artificial sequence
  Synthetic oligonucleotide
ttagtttgaatttggattct

SEQ ID NO: 884 - DNA, 20 bp, Artificial sequence
  Synthetic oligonucleotide
ttttagtttgaatttggatt

SEQ ID NO: 885 - DNA, 20 bp, Artificial sequence
  Synthetic oligonucleotide
ttttttagtttgaatttgga

SEQ ID NO: 886 - DNA, 20 bp, Artificial sequence
  Synthetic oligonucleotide
cagtcctttaatgcttcccc

SEQ ID NO: 887 - DNA, 20 bp, Artificial sequence
  Synthetic oligonucleotide
gtcagtcctttaatgcttcc

SEQ ID NO: 888 - DNA, 20 bp, Artificial sequence
  Synthetic oligonucleotide
cagtcagtcctttaatgctt

SEQ ID NO: 889 - DNA, 20 bp, Artificial sequence
  Synthetic oligonucleotide
ttcagtcagtcctttaatgc

SEQ ID NO: 890 - DNA, 20 bp, Artificial sequence
  Synthetic oligonucleotide
ggccttcagtcagtccttta

SEQ ID NO: 891 - DNA, 20 bp, Artificial sequence
  Synthetic oligonucleotide
tgcaggccttcagtcagtcc

SEQ ID NO: 892 - DNA, 20 bp, Artificial sequence
  Synthetic oligonucleotide
catgcaggccttcagtcagt

SEQ ID NO: 893 - DNA, 20 bp, Artificial sequence
  Synthetic oligonucleotide
tcatgaacatggaatccatg

SEQ ID NO: 894 - DNA, 20 bp, Artificial sequence
  Synthetic oligonucleotide
actcatgaacatggaatcca

SEQ ID NO: 895 - DNA, 20 bp, Artificial sequence
  Synthetic oligonucleotide
ctgtattatctccaaactca

SEQ ID NO: 896 - DNA, 20 bp, Artificial sequence
  Synthetic oligonucleotide
actggtacagcctgctgtat

SEQ ID NO: 897 - DNA, 20 bp, Artificial sequence
  Synthetic oligonucleotide
gcactggtacagcctgctgt

SEQ ID NO: 898 - DNA, 20 bp, Artificial sequence
  Synthetic oligonucleotide
ctgcactggtacagcctgct

SEQ ID NO: 899 - DNA, 20 bp, Artificial sequence
  Synthetic oligonucleotide
acctgcactggtacagcctg

SEQ ID NO: 900 - DNA, 20 bp, Artificial sequence
  Synthetic oligonucleotide
tttctggatagaggattaaa

SEQ ID NO: 901 - DNA, 20 bp, Artificial sequence
  Synthetic oligonucleotide
gttttctggatagaggatta

SEQ ID NO: 902 - DNA, 20 bp, Artificial sequence
  Synthetic oligonucleotide
ccgtgttttctggatagagg

SEQ ID NO: 903 - DNA, 20 bp, Artificial sequence
  Synthetic oligonucleotide
caccgtgttttctggataga

SEQ ID NO: 904 - DNA, 20 bp, Artificial sequence
  Synthetic oligonucleotide
cccaccgtgttttctggata

SEQ ID NO: 905 - DNA, 20 bp, Artificial sequence
  Synthetic oligonucleotide
ggcccaccgtgttttctgga

SEQ ID NO: 906 - DNA, 20 bp, Artificial sequence
  Synthetic oligonucleotide
ttggcccaccgtgttttctg

SEQ ID NO: 907 - DNA, 20 bp, Artificial sequence
  Synthetic oligonucleotide
ctttggcccaccgtgttttc

SEQ ID NO: 908 - DNA, 20 bp, Artificial sequence
  Synthetic oligonucleotide
tcctttggcccaccgtgttt

SEQ ID NO: 909 - DNA, 20 bp, Artificial sequence
  Synthetic oligonucleotide
aagtctccaacatgcctctc

SEQ ID NO: 910 - DNA, 20 bp, Artificial sequence
  Synthetic oligonucleotide
gcccaagtctccaacatgcc

SEQ ID NO: 911 - DNA, 20 bp, Artificial sequence
  Synthetic oligonucleotide
ttgcccaagtctccaacatg

SEQ ID NO: 912 - DNA, 20 bp, Artificial sequence
  Synthetic oligonucleotide
cattgcccaagtctccaaca

SEQ ID NO: 913 - DNA, 20 bp, Artificial sequence
  Synthetic oligonucleotide
cagtcacattgcccaagtct

SEQ ID NO: 914 - DNA, 20 bp, Artificial sequence
  Synthetic oligonucleotide
tcagcagtcacattgcccaa

SEQ ID NO: 915 - DNA, 20 bp, Artificial sequence
  Synthetic oligonucleotide
tgtcagcagtcacattgccc

SEQ ID NO: 916 - DNA, 20 bp, Artificial sequence
  Synthetic oligonucleotide
tttgtcagcagtcacattgc

SEQ ID NO: 917 - DNA, 20 bp, Artificial sequence
  Synthetic oligonucleotide
tctttgtcagcagtcacatt

SEQ ID NO: 918 - DNA, 20 bp, Artificial sequence
  Synthetic oligonucleotide
catctttgtcagcagtcaca

SEQ ID NO: 919 - DNA, 20 bp, Artificial sequence
  Synthetic oligonucleotide
accatctttgtcagcagtca

SEQ ID NO: 920 - DNA, 20 bp, Artificial sequence
  Synthetic oligonucleotide
ccacaccatctttgtcagca

SEQ ID NO: 921 - DNA, 20 bp, Artificial sequence
  Synthetic oligonucleotide
ggccacaccatctttgtcag

SEQ ID NO: 922 - DNA, 20 bp, Artificial sequence
  Synthetic oligonucleotide
cacatcggccacaccatctt

SEQ ID NO: 923 - DNA, 20 bp, Artificial sequence
  Synthetic oligonucleotide
gacacatcggccacaccatc

SEQ ID NO: 924 - DNA, 20 bp, Artificial sequence
  Synthetic oligonucleotide
aatagacacatcggccacac

SEQ ID NO: 925 - DNA, 20 bp, Artificial sequence
  Synthetic oligonucleotide
tcaatagacacatcggccac

SEQ ID NO: 926 - DNA, 20 bp, Artificial sequence
  Synthetic oligonucleotide
cttcaatagacacatcggcc

SEQ ID NO: 927 - DNA, 20 bp, Artificial sequence
  Synthetic oligonucleotide
atcttcaatagacacatcgg

SEQ ID NO: 928 - DNA, 20 bp, Artificial sequence
  Synthetic oligonucleotide
gaatcttcaatagacacatc

SEQ ID NO: 929 - DNA, 20 bp, Artificial sequence
  Synthetic oligonucleotide
cagaatcttcaatagacaca

SEQ ID NO: 930 - DNA, 20 bp, Artificial sequence
  Synthetic oligonucleotide
cacagaatcttcaatagaca

SEQ ID NO: 931 - DNA, 20 bp, Artificial sequence
  Synthetic oligonucleotide
atcacagaatcttcaataga

SEQ ID NO: 932 - DNA, 20 bp, Artificial sequence
  Synthetic oligonucleotide
agatcacagaatcttcaata

SEQ ID NO: 933 - DNA, 20 bp, Artificial sequence
  Synthetic oligonucleotide
tgagatcacagaatcttcaa

SEQ ID NO: 934 - DNA, 20 bp, Artificial sequence
  Synthetic oligonucleotide
agtgagatcacagaatcttc

SEQ ID NO: 935 - DNA, 20 bp, Artificial sequence
  Synthetic oligonucleotide
tgagagtgagatcacagaat

SEQ ID NO: 936 - DNA, 20 bp, Artificial sequence
  Synthetic oligonucleotide
gtctcctgagagtgagatca

SEQ ID NO: 937 - DNA, 20 bp, Artificial sequence
  Synthetic oligonucleotide
tggtctcctgagagtgagat

SEQ ID NO: 938 - DNA, 20 bp, Artificial sequence
  Synthetic oligonucleotide
aatggtctcctgagagtgag

SEQ ID NO: 939 - DNA, 20 bp, Artificial sequence
  Synthetic oligonucleotide
gcaatggtctcctgagagtg

SEQ ID NO: 940 - DNA, 20 bp, Artificial sequence
  Synthetic oligonucleotide
atgcaatggtctcctgagag

SEQ ID NO: 941 - DNA, 20 bp, Artificial sequence
  Synthetic oligonucleotide
tgatgcaatggtctcctgag

SEQ ID NO: 942 - DNA, 20 bp, Artificial sequence
  Synthetic oligonucleotide
aatgatgcaatggtctcctg

SEQ ID NO: 943 - DNA, 20 bp, Artificial sequence
  Synthetic oligonucleotide
ccaatgatgcaatggtctcc

SEQ ID NO: 944 - DNA, 20 bp, Artificial sequence
  Synthetic oligonucleotide
ggccaatgatgcaatggtct

SEQ ID NO: 945 - DNA, 20 bp, Artificial sequence
  Synthetic oligonucleotide
gcggccaatgatgcaatggt

SEQ ID NO: 946 - DNA, 20 bp, Artificial sequence
  Synthetic oligonucleotide
gtgcggccaatgatgcaatg

SEQ ID NO: 947 - DNA, 20 bp, Artificial sequence
  Synthetic oligonucleotide
gtgtgcggccaatgatgcaa

SEQ ID NO: 948 - DNA, 20 bp, Artificial sequence
  Synthetic oligonucleotide
cagtgtgcggccaatgatgc

SEQ ID NO: 949 - DNA, 20 bp, Artificial sequence
  Synthetic oligonucleotide
accagtgtgcggccaatgat

SEQ ID NO: 950 - DNA, 20 bp, Artificial sequence
  Synthetic oligonucleotide
ccaccagtgtgcggccaatg

SEQ ID NO: 951 - DNA, 20 bp, Artificial sequence
  Synthetic oligonucleotide
gaccaccagtgtgcggccaa

SEQ ID NO: 952 - DNA, 20 bp, Artificial sequence
  Synthetic oligonucleotide
tggaccaccagtgtgcggcc

SEQ ID NO: 953 - DNA, 20 bp, Artificial sequence
  Synthetic oligonucleotide
ttcatggaccaccagtgtgc

SEQ ID NO: 954 - DNA, 20 bp, Artificial sequence
  Synthetic oligonucleotide
ttttcatggaccaccagtgt

SEQ ID NO: 955 - DNA, 20 bp, Artificial sequence
  Synthetic oligonucleotide
ctttttcatggaccaccagt

SEQ ID NO: 956 - DNA, 17 bp, Artificial sequence
  Synthetic oligonucleotide
ccactctggccccaaac

SEQ ID NO: 957 - DNA, 17 bp, Artificial sequence
  Synthetic oligonucleotide
cccactctggccccaaa

SEQ ID NO: 958 - DNA, 17 bp, Artificial sequence
  Synthetic oligonucleotide
gcccactctggccccaa

SEQ ID NO: 959 - DNA, 17 bp, Artificial sequence
  Synthetic oligonucleotide
cgcccactctggcccca

SEQ ID NO: 960 - DNA, 17 bp, Artificial sequence
  Synthetic oligonucleotide
cgactactttataggcc

SEQ ID NO: 961 - DNA, 17 bp, Artificial sequence
  Synthetic oligonucleotide
gcgactactttataggc

SEQ ID NO: 962 - DNA, 17 bp, Artificial sequence
  Synthetic oligonucleotide
cgcgactactttatagg

SEQ ID NO: 963 - DNA, 17 bp, Artificial sequence
  Synthetic oligonucleotide
ccgcgactactttatag

SEQ ID NO: 964 - DNA, 17 bp, Artificial sequence
  Synthetic oligonucleotide
cgctgcaggagactacg

SEQ ID NO: 965 - DNA, 17 bp, Artificial sequence
  Synthetic oligonucleotide
acgctgcaggagactac

SEQ ID NO: 966 - DNA, 17 bp, Artificial sequence
  Synthetic oligonucleotide
tcgcccttcagcacgca

SEQ ID NO: 967 - DNA, 17 bp, Artificial sequence
  Synthetic oligonucleotide
gtcgcccttcagcacgc

SEQ ID NO: 968 - DNA, 17 bp, Artificial sequence
  Synthetic oligonucleotide
cgtcgcccttcagcacg

SEQ ID NO: 969 - DNA, 17 bp, Artificial sequence
  Synthetic oligonucleotide
ccgtcgcccttcagcac

SEQ ID NO: 970 - DNA, 17 bp, Artificial sequence
  Synthetic oligonucleotide
gccgtcgcccttcagca

SEQ ID NO: 971 - DNA, 17 bp, Artificial sequence
  Synthetic oligonucleotide
tctgctcgaaattgatg

SEQ ID NO: 972 - DNA, 17 bp, Artificial sequence
  Synthetic oligonucleotide
ttctgctcgaaattgat

SEQ ID NO: 973 - DNA, 17 bp, Artificial sequence
  Synthetic oligonucleotide
cttctgctcgaaattga

SEQ ID NO: 974 - DNA, 17 bp, Artificial sequence
  Synthetic oligonucleotide
ccttctgctcgaaattg

SEQ ID NO: 975 - DNA, 17 bp, Artificial sequence
  Synthetic oligonucleotide
tccttctgctcgaaatt

SEQ ID NO: 976 - DNA, 17 bp, Artificial sequence
  Synthetic oligonucleotide
ttccttctgctcgaaat

SEQ ID NO: 977 - DNA, 17 bp, Artificial sequence
  Synthetic oligonucleotide
tttccttctgctcgaaa

SEQ ID NO: 978 - DNA, 17 bp, Artificial sequence
  Synthetic oligonucleotide
ctttccttctgctcgaa

SEQ ID NO: 979 - DNA, 17 bp, Artificial sequence
  Synthetic oligonucleotide
actttccttctgctcga

SEQ ID NO: 980 - DNA, 17 bp, Artificial sequence
  Synthetic oligonucleotide
tactttccttctgctcg

SEQ ID NO: 981 - DNA, 17 bp, Artificial sequence
  Synthetic oligonucleotide
ttactttccttctgctc

SEQ ID NO: 982 - DNA, 17 bp, Artificial sequence
  Synthetic oligonucleotide
attactttccttctgct

SEQ ID NO: 983 - DNA, 17 bp, Artificial sequence
  Synthetic oligonucleotide
cattactttccttctgc

SEQ ID NO: 984 - DNA, 17 bp, Artificial sequence
  Synthetic oligonucleotide
ccattactttccttctg

SEQ ID NO: 985 - DNA, 17 bp, Artificial sequence
  Synthetic oligonucleotide
tccattactttccttct

SEQ ID NO: 986 - DNA, 17 bp, Artificial sequence
  Synthetic oligonucleotide
gtccattactttccttc

SEQ ID NO: 987 - DNA, 17 bp, Artificial sequence
  Synthetic oligonucleotide
ggtccattactttcctt

SEQ ID NO: 988 - DNA, 17 bp, Artificial sequence
  Synthetic oligonucleotide
tggtccattactttcct

SEQ ID NO: 989 - DNA, 17 bp, Artificial sequence
  Synthetic oligonucleotide
ctggtccattactttcc

SEQ ID NO: 990 - DNA, 17 bp, Artificial sequence
  Synthetic oligonucleotide
actggtccattactttc

SEQ ID NO: 991 - DNA, 17 bp, Artificial sequence
  Synthetic oligonucleotide
cactggtccattacttt

SEQ ID NO: 992 - DNA, 17 bp, Artificial sequence
  Synthetic oligonucleotide
tcactggtccattactt

SEQ ID NO: 993 - DNA, 17 bp, Artificial sequence
  Synthetic oligonucleotide
ttcactggtccattact

SEQ ID NO: 994 - DNA, 17 bp, Artificial sequence
  Synthetic oligonucleotide
cttcactggtccattac

SEQ ID NO: 995 - DNA, 17 bp, Artificial sequence
  Synthetic oligonucleotide
ccttcactggtccatta

SEQ ID NO: 996 - DNA, 17 bp, Artificial sequence
  Synthetic oligonucleotide
accttcactggtccatt

SEQ ID NO: 997 - DNA, 17 bp, Artificial sequence
  Synthetic oligonucleotide
caccttcactggtccat

SEQ ID NO: 998 - DNA, 17 bp, Artificial sequence
  Synthetic oligonucleotide
acaccttcactggtcca

SEQ ID NO: 999 - DNA, 17 bp, Artificial sequence
  Synthetic oligonucleotide
cacaccttcactggtcc

SEQ ID NO: 1000 - DNA, 17 bp, Artificial sequence
  Synthetic oligonucleotide
ccacaccttcactggtc

SEQ ID NO: 1001 - DNA, 17 bp, Artificial sequence
  Synthetic oligonucleotide
cccacaccttcactggt

SEQ ID NO: 1002 - DNA, 17 bp, Artificial sequence
  Synthetic oligonucleotide
ccccacaccttcactgg

SEQ ID NO: 1003 - DNA, 17 bp, Artificial sequence
  Synthetic oligonucleotide
ttccccacaccttcact

SEQ ID NO: 1004 - DNA, 17 bp, Artificial sequence
  Synthetic oligonucleotide
cttccccacaccttcac

SEQ ID NO: 1005 - DNA, 17 bp, Artificial sequence
  Synthetic oligonucleotide
gcttccccacaccttca

SEQ ID NO: 1006 - DNA, 17 bp, Artificial sequence
  Synthetic oligonucleotide
tgcttccccacaccttc

SEQ ID NO: 1007 - DNA, 17 bp, Artificial sequence
  Synthetic oligonucleotide
atgcttccccacacctt

SEQ ID NO: 1008 - DNA, 17 bp, Artificial sequence
  Synthetic oligonucleotide
aatgcttccccacacct

SEQ ID NO: 1009 - DNA, 17 bp, Artificial sequence
  Synthetic oligonucleotide
taatgcttccccacacc

SEQ ID NO: 1010 - DNA, 17 bp, Artificial sequence
  Synthetic oligonucleotide
atgcaggccttcagtca

SEQ ID NO: 1011 - DNA, 17 bp, Artificial sequence
  Synthetic oligonucleotide
catgcaggccttcagtc

SEQ ID NO: 1012 - DNA, 17 bp, Artificial sequence
  Synthetic oligonucleotide
ccatgcaggccttcagt

SEQ ID NO: 1013 - DNA, 17 bp, Artificial sequence
  Synthetic oligonucleotide
tccatgcaggccttcag

SEQ ID NO: 1014 - DNA, 17 bp, Artificial sequence
  Synthetic oligonucleotide
atccatgcaggccttca

SEQ ID NO: 1015 - DNA, 17 bp, Artificial sequence
  Synthetic oligonucleotide
aatccatgcaggccttc

SEQ ID NO: 1016 - DNA, 17 bp, Artificial sequence
  Synthetic oligonucleotide
gaatccatgcaggcctt

SEQ ID NO: 1017 - DNA, 17 bp, Artificial sequence
  Synthetic oligonucleotide
ggaatccatgcaggcct

SEQ ID NO: 1018 - DNA, 17 bp, Artificial sequence
  Synthetic oligonucleotide
tggaatccatgcaggcc

SEQ ID NO: 1019 - DNA, 17 bp, Artificial sequence
  Synthetic oligonucleotide
atggaatccatgcaggc

SEQ ID NO: 1020 - DNA, 17 bp, Artificial sequence
  Synthetic oligonucleotide
catggaatccatgcagg

SEQ ID NO: 1021 - DNA, 17 bp, Artificial sequence
  Synthetic oligonucleotide
acatggaatccatgcag

SEQ ID NO: 1022 - DNA, 17 bp, Artificial sequence
  Synthetic oligonucleotide
aacatggaatccatgca

SEQ ID NO: 1023 - DNA, 17 bp, Artificial sequence
  Synthetic oligonucleotide
gaacatggaatccatgc

SEQ ID NO: 1024 - DNA, 17 bp, Artificial sequence
  Synthetic oligonucleotide
tgaacatggaatccatg

SEQ ID NO: 1025 - DNA, 17 bp, Artificial sequence
  Synthetic oligonucleotide
atgaacatggaatccat

SEQ ID NO: 1026 - DNA, 17 bp, Artificial sequence
  Synthetic oligonucleotide
ctgcactggtacagcct

SEQ ID NO: 1027 - DNA, 17 bp, Artificial sequence
  Synthetic oligonucleotide
cctgcactggtacagcc

SEQ ID NO: 1028 - DNA, 17 bp, Artificial sequence
  Synthetic oligonucleotide
acctgcactggtacagc

SEQ ID NO: 1029 - DNA, 17 bp, Artificial sequence
  Synthetic oligonucleotide
gacctgcactggtacag

SEQ ID NO: 1030 - DNA, 17 bp, Artificial sequence
  Synthetic oligonucleotide
ggacctgcactggtaca

SEQ ID NO: 1031 - DNA, 17 bp, Artificial sequence
  Synthetic oligonucleotide
aggacctgcactggtac

SEQ ID NO: 1032 - DNA, 17 bp, Artificial sequence
  Synthetic oligonucleotide
gaggacctgcactggta

SEQ ID NO: 1033 - DNA, 17 bp, Artificial sequence
  Synthetic oligonucleotide
tgaggacctgcactggt

SEQ ID NO: 1034 - DNA, 17 bp, Artificial sequence
  Synthetic oligonucleotide
gtgaggacctgcactgg

SEQ ID NO: 1035 - DNA, 17 bp, Artificial sequence
  Synthetic oligonucleotide
agtgaggacctgcactg

SEQ ID NO: 1036 - DNA, 17 bp, Artificial sequence
  Synthetic oligonucleotide
aagtgaggacctgcact

SEQ ID NO: 1037 - DNA, 17 bp, Artificial sequence
  Synthetic oligonucleotide
aaagtgaggacctgcac

SEQ ID NO: 1038 - DNA, 17 bp, Artificial sequence
  Synthetic oligonucleotide
taaagtgaggacctgca

SEQ ID NO: 1039 - DNA, 17 bp, Artificial sequence
  Synthetic oligonucleotide
ttaaagtgaggacctgc

SEQ ID NO: 1040 - DNA, 17 bp, Artificial sequence
  Synthetic oligonucleotide
attaaagtgaggacctg

SEQ ID NO: 1041 - DNA, 17 bp, Artificial sequence
  Synthetic oligonucleotide
gattaaagtgaggacct

SEQ ID NO: 1042 - DNA, 17 bp, Artificial sequence
  Synthetic oligonucleotide
ggattaaagtgaggacc

SEQ ID NO: 1043 - DNA, 17 bp, Artificial sequence
  Synthetic oligonucleotide
aggattaaagtgaggac

SEQ ID NO: 1044 - DNA, 17 bp, Artificial sequence
  Synthetic oligonucleotide
gaggattaaagtgagga

SEQ ID NO: 1045 - DNA, 17 bp, Artificial sequence
  Synthetic oligonucleotide
agaggattaaagtgagg

SEQ ID NO: 1046 - DNA, 17 bp, Artificial sequence
  Synthetic oligonucleotide
tagaggattaaagtgag

SEQ ID NO: 1047 - DNA, 17 bp, Artificial sequence
  Synthetic oligonucleotide
atagaggattaaagtga

SEQ ID NO: 1048 - DNA, 17 bp, Artificial sequence
  Synthetic oligonucleotide
gatagaggattaaagtg

SEQ ID NO: 1049 - DNA, 17 bp, Artificial sequence
  Synthetic oligonucleotide
ggatagaggattaaagt

SEQ ID NO: 1050 - DNA, 17 bp, Artificial sequence
  Synthetic oligonucleotide
tggatagaggattaaag

SEQ ID NO: 1051 - DNA, 17 bp, Artificial sequence
  Synthetic oligonucleotide
ctggatagaggattaaa

SEQ ID NO: 1052 - DNA, 17 bp, Artificial sequence
  Synthetic oligonucleotide
tctggatagaggattaa

SEQ ID NO: 1053 - DNA, 17 bp, Artificial sequence
  Synthetic oligonucleotide
ctttggcccaccgtgtt

SEQ ID NO: 1054 - DNA, 17 bp, Artificial sequence
  Synthetic oligonucleotide
cctttggcccaccgtgt

SEQ ID NO: 1055 - DNA, 17 bp, Artificial sequence
  Synthetic oligonucleotide
tcctttggcccaccgtg

SEQ ID NO: 1056 - DNA, 17 bp, Artificial sequence
  Synthetic oligonucleotide
atcctttggcccaccgt

SEQ ID NO: 1057 - DNA, 17 bp, Artificial sequence
  Synthetic oligonucleotide
catcctttggcccaccg

SEQ ID NO: 1058 - DNA, 17 bp, Artificial sequence
  Synthetic oligonucleotide
tcatcctttggcccacc

SEQ ID NO: 1059 - DNA, 17 bp, Artificial sequence
  Synthetic oligonucleotide
ttcatcctttggcccac

SEQ ID NO: 1060 - DNA, 17 bp, Artificial sequence
  Synthetic oligonucleotide
cttcatcctttggccca

SEQ ID NO: 1061 - DNA, 17 bp, Artificial sequence
  Synthetic oligonucleotide
tcttcatcctttggccc

SEQ ID NO: 1062 - DNA, 17 bp, Artificial sequence
  Synthetic oligonucleotide
ctcttcatcctttggcc

SEQ ID NO: 1063 - DNA, 17 bp, Artificial sequence
  Synthetic oligonucleotide
tctcttcatcctttggc

SEQ ID NO: 1064 - DNA, 17 bp, Artificial sequence
  Synthetic oligonucleotide
ctctcttcatcctttgg

SEQ ID NO: 1065 - DNA, 17 bp, Artificial sequence
  Synthetic oligonucleotide
tgcctctcttcatcctt

SEQ ID NO: 1066 - DNA, 17 bp, Artificial sequence
  Synthetic oligonucleotide
atgcctctcttcatcct

SEQ ID NO: 1067 - DNA, 17 bp, Artificial sequence
  Synthetic oligonucleotide
catgcctctcttcatcc

SEQ ID NO: 1068 - DNA, 17 bp, Artificial sequence
  Synthetic oligonucleotide
acatgcctctcttcatc

SEQ ID NO: 1069 - DNA, 17 bp, Artificial sequence
  Synthetic oligonucleotide
aacatgcctctcttcat

SEQ ID NO: 1070 - DNA, 17 bp, Artificial sequence
  Synthetic oligonucleotide
caacatgcctctcttca

SEQ ID NO: 1071 - DNA, 17 bp, Artificial sequence
  Synthetic oligonucleotide
ccaacatgcctctcttc

SEQ ID NO: 1072 - DNA, 17 bp, Artificial sequence
  Synthetic oligonucleotide
tccaacatgcctctctt

SEQ ID NO: 1073 - DNA, 17 bp, Artificial sequence
  Synthetic oligonucleotide
ctccaacatgcctctct

SEQ ID NO: 1074 - DNA, 17 bp, Artificial sequence
  Synthetic oligonucleotide
tctccaacatgcctctc

SEQ ID NO: 1075 - DNA, 17 bp, Artificial sequence
  Synthetic oligonucleotide
gtctccaacatgcctct

SEQ ID NO: 1076 - DNA, 17 bp, Artificial sequence
  Synthetic oligonucleotide
agcagtcacattgccca

SEQ ID NO: 1077 - DNA, 17 bp, Artificial sequence
  Synthetic oligonucleotide
cagcagtcacattgccc

SEQ ID NO: 1078 - DNA, 17 bp, Artificial sequence
  Synthetic oligonucleotide
agacacatcggccacac

SEQ ID NO: 1079 - DNA, 17 bp, Artificial sequence
  Synthetic oligonucleotide
cttcaatagacacatcg

SEQ ID NO: 1080 - DNA, 17 bp, Artificial sequence
  Synthetic oligonucleotide
gagatcacagaatcttc

SEQ ID NO: 1081 - DNA, 17 bp, Artificial sequence
  Synthetic oligonucleotide
tttttcatggaccacca

SEQ ID NO: 1082 - DNA, 17 bp, Artificial sequence
  Synthetic oligonucleotide
ctttttcatggaccacc

SEQ ID NO: 1083 - DNA, 17 bp, Artificial sequence
  Synthetic oligonucleotide
gctttttcatggaccac

SEQ ID NO: 1084 - DNA, 17 bp, Artificial sequence
  Synthetic oligonucleotide
tgctttttcatggacca

SEQ ID NO: 1085 - DNA, 17 bp, Artificial sequence
  Synthetic oligonucleotide
ctgctttttcatggacc

SEQ ID NO: 1086 - DNA, 17 bp, Artificial sequence
  Synthetic oligonucleotide
tctgctttttcatggac

SEQ ID NO: 1087 - DNA, 17 bp, Artificial sequence
  Synthetic oligonucleotide
atctgctttttcatgga

SEQ ID NO: 1088 - DNA, 17 bp, Artificial sequence
  Synthetic oligonucleotide
catctgctttttcatgg

SEQ ID NO: 1089 - DNA, 17 bp, Artificial sequence
  Synthetic oligonucleotide
tcatctgctttttcatg

SEQ ID NO: 1090 - DNA, 17 bp, Artificial sequence
  Synthetic oligonucleotide
gtcatctgctttttcat

SEQ ID NO: 1091 - DNA, 17 bp, Artificial sequence
  Synthetic oligonucleotide
agtcatctgctttttca

SEQ ID NO: 1092 - DNA, 17 bp, Artificial sequence
  Synthetic oligonucleotide
aagtcatctgctttttc

SEQ ID NO: 1093 - DNA, 17 bp, Artificial sequence
  Synthetic oligonucleotide
caagtcatctgcttttt

SEQ ID NO: 1094 - DNA, 17 bp, Artificial sequence
  Synthetic oligonucleotide
ccaagtcatctgctttt

SEQ ID NO: 1095 - DNA, 17 bp, Artificial sequence
  Synthetic oligonucleotide
cccaagtcatctgcttt

SEQ ID NO: 1096 - DNA, 17 bp, Artificial sequence
  Synthetic oligonucleotide
gcccaagtcatctgctt

SEQ ID NO: 1097 - DNA, 17 bp, Artificial sequence
  Synthetic oligonucleotide
tgcccaagtcatctgct

SEQ ID NO: 1098 - DNA, 17 bp, Artificial sequence
  Synthetic oligonucleotide
ttgcccaagtcatctgc

SEQ ID NO: 1099 - DNA, 17 bp, Artificial sequence
  Synthetic oligonucleotide
ccacctttgcccaagtc

SEQ ID NO: 1100 - DNA, 17 bp, Artificial sequence
  Synthetic oligonucleotide
tccacctttgcccaagt

SEQ ID NO: 1101 - DNA, 17 bp, Artificial sequence
  Synthetic oligonucleotide
ttccacctttgcccaag

SEQ ID NO: 1102 - DNA, 17 bp, Artificial sequence
  Synthetic oligonucleotide
tttccacctttgcccaa

SEQ ID NO: 1103 - DNA, 17 bp, Artificial sequence
  Synthetic oligonucleotide
atttccacctttgccca

SEQ ID NO: 1104 - DNA, 17 bp, Artificial sequence
  Synthetic oligonucleotide
catttccacctttgccc

SEQ ID NO: 1105 - DNA, 17 bp, Artificial sequence
  Synthetic oligonucleotide
tcatttccacctttgcc

SEQ ID NO: 1106 - DNA, 17 bp, Artificial sequence
  Synthetic oligonucleotide
ttcatttccacctttgc

SEQ ID NO: 1107 - DNA, 17 bp, Artificial sequence
  Synthetic oligonucleotide
tcttcatttccaccttt

SEQ ID NO: 1108 - DNA, 17 bp, Artificial sequence
  Synthetic oligonucleotide
ctttcttcatttccacc

SEQ ID NO: 1109 - DNA, 17 bp, Artificial sequence
  Synthetic oligonucleotide
actttcttcatttccac

SEQ ID NO: 1110 - DNA, 17 bp, Artificial sequence
  Synthetic oligonucleotide
tactttcttcatttcca

SEQ ID NO: 1111 - DNA, 17 bp, Artificial sequence
  Synthetic oligonucleotide
aattacaccacaagcca

SEQ ID NO: 1112 - DNA, 17 bp, Artificial sequence
  Synthetic oligonucleotide
caattacaccacaagcc

SEQ ID NO: 1113 - DNA, 17 bp, Artificial sequence
  Synthetic oligonucleotide
ccaattacaccacaagc

SEQ ID NO: 1114 - DNA, 17 bp, Artificial sequence
  Synthetic oligonucleotide
cccaattacaccacaag

SEQ ID NO: 1115 - DNA, 17 bp, Artificial sequence
  Synthetic oligonucleotide
gatcccaattacaccac

SEQ ID NO: 1116 - DNA, 17 bp, Artificial sequence
  Synthetic oligonucleotide
cgatcccaattacacca

SEQ ID NO: 1117 - DNA, 17 bp, Artificial sequence
  Synthetic oligonucleotide
gcgatcccaattacacc

SEQ ID NO: 1118 - DNA, 17 bp, Artificial sequence
  Synthetic oligonucleotide
ggcgatcccaattacac

SEQ ID NO: 1119 - DNA, 17 bp, Artificial sequence
  Synthetic oligonucleotide
gggcgatcccaattaca

SEQ ID NO: 1120 - DNA, 17 bp, Artificial sequence
  Synthetic oligonucleotide
tgggcgatcccaattac

SEQ ID NO: 1121 - DNA, 17 bp, Artificial sequence
  Synthetic oligonucleotide
ttgggcgatcccaatta

SEQ ID NO: 1122 - DNA, 17 bp, Artificial sequence
  Synthetic oligonucleotide
attgggcgatcccaatt

SEQ ID NO: 1123 - DNA, 17 bp, Artificial sequence
  Synthetic oligonucleotide
tattgggcgatcccaat

SEQ ID NO: 1124 - DNA, 17 bp, Artificial sequence
  Synthetic oligonucleotide
ttattgggcgatcccaa

SEQ ID NO: 1125 - DNA, 17 bp, Artificial sequence
  Synthetic oligonucleotide
tttattgggcgatccca

SEQ ID NO: 1126 - DNA, 17 bp, Artificial sequence
  Synthetic oligonucleotide
gtttattgggcgatccc

SEQ ID NO: 1127 - DNA, 17 bp, Artificial sequence
  Synthetic oligonucleotide
tgtttattgggcgatcc

SEQ ID NO: 1128 - DNA, 17 bp, Artificial sequence
  Synthetic oligonucleotide
atgtttattgggcgatc

SEQ ID NO: 1129 - DNA, 17 bp, Artificial sequence
  Synthetic oligonucleotide
aatgtttattgggcgat

SEQ ID NO: 1130 - DNA, 17 bp, Artificial sequence
  Synthetic oligonucleotide
gaatgtttattgggcga

SEQ ID NO: 1131 - DNA, 17 bp, Artificial sequence
  Synthetic oligonucleotide
ggaatgtttattgggcg

SEQ ID NO: 1132 - DNA, 17 bp, Artificial sequence
  Synthetic oligonucleotide
aagggaatgtttattgg

SEQ ID NO: 1133 - DNA, 17 bp, Artificial sequence
  Synthetic oligonucleotide
caagggaatgtttattg

SEQ ID NO: 1134 - DNA, 17 bp, Artificial sequence
  Synthetic oligonucleotide
ccaagggaatgtttatt

SEQ ID NO: 1135 - DNA, 17 bp, Artificial sequence
  Synthetic oligonucleotide
tccaagggaatgtttat

SEQ ID NO: 1136 - DNA, 17 bp, Artificial sequence
  Synthetic oligonucleotide
atccaagggaatgttta

SEQ ID NO: 1137 - DNA, 17 bp, Artificial sequence
  Synthetic oligonucleotide
catccaagggaatgttt

SEQ ID NO: 1138 - DNA, 17 bp, Artificial sequence
  Synthetic oligonucleotide
acatccaagggaatgtt

SEQ ID NO: 1139 - DNA, 17 bp, Artificial sequence
  Synthetic oligonucleotide
tacatccaagggaatgt

SEQ ID NO: 1140 - DNA, 17 bp, Artificial sequence
  Synthetic oligonucleotide
ctacatccaagggaatg

SEQ ID NO: 1141 - DNA, 17 bp, Artificial sequence
  Synthetic oligonucleotide
actacatccaagggaat

SEQ ID NO: 1142 - DNA, 17 bp, Artificial sequence
  Synthetic oligonucleotide
gactacatccaagggaa

SEQ ID NO: 1143 - DNA, 17 bp, Artificial sequence
  Synthetic oligonucleotide
agactacatccaaggga

SEQ ID NO: 1144 - DNA, 17 bp, Artificial sequence
  Synthetic oligonucleotide
cagactacatccaaggg

SEQ ID NO: 1145 - DNA, 17 bp, Artificial sequence
  Synthetic oligonucleotide
tcagactacatccaagg

SEQ ID NO: 1146 - DNA, 17 bp, Artificial sequence
  Synthetic oligonucleotide
ctcagactacatccaag

SEQ ID NO: 1147 - DNA, 17 bp, Artificial sequence
  Synthetic oligonucleotide
cctcagactacatccaa

SEQ ID NO: 1148 - DNA, 17 bp, Artificial sequence
  Synthetic oligonucleotide
gcctcagactacatcca

SEQ ID NO: 1149 - DNA, 17 bp, Artificial sequence
  Synthetic oligonucleotide
ggcctcagactacatcc

SEQ ID NO: 1150 - DNA, 17 bp, Artificial sequence
  Synthetic oligonucleotide
gggcctcagactacatc

SEQ ID NO: 1151 - DNA, 17 bp, Artificial sequence
  Synthetic oligonucleotide
gataacagatgagttaa

SEQ ID NO: 1152 - DNA, 17 bp, Artificial sequence
  Synthetic oligonucleotide
ggataacagatgagtta

SEQ ID NO: 1153 - DNA, 17 bp, Artificial sequence
  Synthetic oligonucleotide
aggataacagatgagtt

SEQ ID NO: 1154 - DNA, 17 bp, Artificial sequence
  Synthetic oligonucleotide
caggataacagatgagt

SEQ ID NO: 1155 - DNA, 17 bp, Artificial sequence
  Synthetic oligonucleotide
gcaggataacagatgag

SEQ ID NO: 1156 - DNA, 17 bp, Artificial sequence
  Synthetic oligonucleotide
agcaggataacagatga

SEQ ID NO: 1157 - DNA, 17 bp, Artificial sequence
  Synthetic oligonucleotide
tagcaggataacagatg

SEQ ID NO: 1158 - DNA, 17 bp, Artificial sequence
  Synthetic oligonucleotide
ctagcaggataacagat

SEQ ID NO: 1159 - DNA, 17 bp, Artificial sequence
  Synthetic oligonucleotide
gctagcaggataacaga

SEQ ID NO: 1160 - DNA, 17 bp, Artificial sequence
  Synthetic oligonucleotide
agctagcaggataacag

SEQ ID NO: 1161 - DNA, 17 bp, Artificial sequence
  Synthetic oligonucleotide
cagctagcaggataaca

SEQ ID NO: 1162 - DNA, 17 bp, Artificial sequence
  Synthetic oligonucleotide
acagctagcaggataac

SEQ ID NO: 1163 - DNA, 17 bp, Artificial sequence
  Synthetic oligonucleotide
tacagctagcaggataa

SEQ ID NO: 1164 - DNA, 17 bp, Artificial sequence
  Synthetic oligonucleotide
ctacagctagcaggata

SEQ ID NO: 1165 - DNA, 17 bp, Artificial sequence
  Synthetic oligonucleotide
tctacagctagcaggat

SEQ ID NO: 1166 - DNA, 17 bp, Artificial sequence
  Synthetic oligonucleotide
ttctacagctagcagga

SEQ ID NO: 1167 - DNA, 17 bp, Artificial sequence
  Synthetic oligonucleotide
tttctacagctagcagg

SEQ ID NO: 1168 - DNA, 17 bp, Artificial sequence
  Synthetic oligonucleotide
atttctacagctagcag

SEQ ID NO: 1169 - DNA, 17 bp, Artificial sequence
  Synthetic oligonucleotide
catttctacagctagca

SEQ ID NO: 1170 - DNA, 17 bp, Artificial sequence
  Synthetic oligonucleotide
atacatttctacagcta

SEQ ID NO: 1171 - DNA, 17 bp, Artificial sequence
  Synthetic oligonucleotide
gatacatttctacagct

SEQ ID NO: 1172 - DNA, 17 bp, Artificial sequence
  Synthetic oligonucleotide
gtgtttaatgtttatca

SEQ ID NO: 1173 - DNA, 17 bp, Artificial sequence
  Synthetic oligonucleotide
agtgtttaatgtttatc

SEQ ID NO: 1174 - DNA, 17 bp, Artificial sequence
  Synthetic oligonucleotide
cagtgtttaatgtttat

SEQ ID NO: 1175 - DNA, 17 bp, Artificial sequence
  Synthetic oligonucleotide
acagtgtttaatgttta

SEQ ID NO: 1176 - DNA, 17 bp, Artificial sequence
  Synthetic oligonucleotide
tacagtgtttaatgttt

SEQ ID NO: 1177 - DNA, 17 bp, Artificial sequence
  Synthetic oligonucleotide
ttacagtgtttaatgtt

SEQ ID NO: 1178 - DNA, 17 bp, Artificial sequence
  Synthetic oligonucleotide
attacagtgtttaatgt

SEQ ID NO: 1179 - DNA, 17 bp, Artificial sequence
  Synthetic oligonucleotide
gattacagtgtttaatg

SEQ ID NO: 1180 - DNA, 17 bp, Artificial sequence
  Synthetic oligonucleotide
agattacagtgtttaat

SEQ ID NO: 1181 - DNA, 17 bp, Artificial sequence
  Synthetic oligonucleotide
aagattacagtgtttaa

SEQ ID NO: 1182 - DNA, 17 bp, Artificial sequence
  Synthetic oligonucleotide
taagattacagtgttta

SEQ ID NO: 1183 - DNA, 17 bp, Artificial sequence
  Synthetic oligonucleotide
ttaagattacagtgttt

SEQ ID NO: 1184 - DNA, 17 bp, Artificial sequence
  Synthetic oligonucleotide
atcttccaagtgatcat

SEQ ID NO: 1185 - DNA, 17 bp, Artificial sequence
  Synthetic oligonucleotide
aatcttccaagtgatca

SEQ ID NO: 1186 - DNA, 17 bp, Artificial sequence
  Synthetic oligonucleotide
aaatcttccaagtgatc

SEQ ID NO: 1187 - DNA, 17 bp, Artificial sequence
  Synthetic oligonucleotide
caaatcttccaagtgat

SEQ ID NO: 1188 - DNA, 17 bp, Artificial sequence
  Synthetic oligonucleotide
tacaaatcttccaagtg

SEQ ID NO: 1189 - DNA, 17 bp, Artificial sequence
  Synthetic oligonucleotide
atacaaatcttccaagt

SEQ ID NO: 1190 - DNA, 17 bp, Artificial sequence
  Synthetic oligonucleotide
tatacaaatcttccaag

SEQ ID NO: 1191 - DNA, 17 bp, Artificial sequence
  Synthetic oligonucleotide
ctatacaaatcttccaa

SEQ ID NO: 1192 - DNA, 17 bp, Artificial sequence
  Synthetic oligonucleotide
actatacaaatcttcca

SEQ ID NO: 1193 - DNA, 17 bp, Artificial sequence
  Synthetic oligonucleotide
aactatacaaatcttcc

SEQ ID NO: 1194 - DNA, 17 bp, Artificial sequence
  Synthetic oligonucleotide
aaactatacaaatcttc

SEQ ID NO: 1195 - DNA, 17 bp, Artificial sequence
  Synthetic oligonucleotide
ataaaactatacaaatc

SEQ ID NO: 1196 - DNA, 17 bp, Artificial sequence
  Synthetic oligonucleotide
gttttataaaactatac

SEQ ID NO: 1197 - DNA, 17 bp, Artificial sequence
  Synthetic oligonucleotide
gagttttataaaactat

SEQ ID NO: 1198 - DNA, 17 bp, Artificial sequence
  Synthetic oligonucleotide
attgaaacagacatttt

SEQ ID NO: 1199 - DNA, 17 bp, Artificial sequence
  Synthetic oligonucleotide
cattgaaacagacattt

SEQ ID NO: 1200 - DNA, 17 bp, Artificial sequence
  Synthetic oligonucleotide
tcattgaaacagacatt

SEQ ID NO: 1201 - DNA, 17 bp, Artificial sequence
  Synthetic oligonucleotide
gtcattgaaacagacat

SEQ ID NO: 1202 - DNA, 17 bp, Artificial sequence
  Synthetic oligonucleotide
ggtcattgaaacagaca

SEQ ID NO: 1203 - DNA, 17 bp, Artificial sequence
  Synthetic oligonucleotide
aggtcattgaaacagac

SEQ ID NO: 1204 - DNA, 17 bp, Artificial sequence
  Synthetic oligonucleotide
caggtcattgaaacaga

SEQ ID NO: 1205 - DNA, 17 bp, Artificial sequence
  Synthetic oligonucleotide
acaggtcattgaaacag

SEQ ID NO: 1206 - DNA, 17 bp, Artificial sequence
  Synthetic oligonucleotide
tacaggtcattgaaaca

SEQ ID NO: 1207 - DNA, 17 bp, Artificial sequence
  Synthetic oligonucleotide
atacaggtcattgaaac

SEQ ID NO: 1208 - DNA, 17 bp, Artificial sequence
  Synthetic oligonucleotide
aatacaggtcattgaaa

SEQ ID NO: 1209 - DNA, 17 bp, Artificial sequence
  Synthetic oligonucleotide
aaatacaggtcattgaa

SEQ ID NO: 1210 - DNA, 17 bp, Artificial sequence
  Synthetic oligonucleotide
aaaatacaggtcattga

SEQ ID NO: 1211 - DNA, 17 bp, Artificial sequence
  Synthetic oligonucleotide
caaaatacaggtcattg

SEQ ID NO: 1212 - DNA, 17 bp, Artificial sequence
  Synthetic oligonucleotide
gcaaaatacaggtcatt

SEQ ID NO: 1213 - DNA, 17 bp, Artificial sequence
  Synthetic oligonucleotide
ggcaaaatacaggtcat

SEQ ID NO: 1214 - DNA, 17 bp, Artificial sequence
  Synthetic oligonucleotide
tggcaaaatacaggtca

SEQ ID NO: 1215 - DNA, 17 bp, Artificial sequence
  Synthetic oligonucleotide
ctggcaaaatacaggtc

SEQ ID NO: 1216 - DNA, 17 bp, Artificial sequence
  Synthetic oligonucleotide
tctggcaaaatacaggt

SEQ ID NO: 1217 - DNA, 17 bp, Artificial sequence
  Synthetic oligonucleotide
gtctggcaaaatacagg

SEQ ID NO: 1218 - DNA, 17 bp, Artificial sequence
  Synthetic oligonucleotide
agtctggcaaaatacag

SEQ ID NO: 1219 - DNA, 17 bp, Artificial sequence
  Synthetic oligonucleotide
aagtctggcaaaataca

SEQ ID NO: 1220 - DNA, 17 bp, Artificial sequence
  Synthetic oligonucleotide
taagtctggcaaaatac

SEQ ID NO: 1221 - DNA, 17 bp, Artificial sequence
  Synthetic oligonucleotide
ttaagtctggcaaaata

SEQ ID NO: 1222 - DNA, 17 bp, Artificial sequence
  Synthetic oligonucleotide
aatacccatctgtgatt

SEQ ID NO: 1223 - DNA, 17 bp, Artificial sequence
  Synthetic oligonucleotide
taatacccatctgtgat

SEQ ID NO: 1224 - DNA, 17 bp, Artificial sequence
  Synthetic oligonucleotide
ttaatacccatctgtga

SEQ ID NO: 1225 - DNA, 17 bp, Artificial sequence
  Synthetic oligonucleotide
tttaatacccatctgtg

SEQ ID NO: 1226 - DNA, 17 bp, Artificial sequence
  Synthetic oligonucleotide
gtttaatacccatctgt

SEQ ID NO: 1227 - DNA, 17 bp, Artificial sequence
  Synthetic oligonucleotide
agtttaatacccatctg

SEQ ID NO: 1228 - DNA, 17 bp, Artificial sequence
  Synthetic oligonucleotide
aagtttaatacccatct

SEQ ID NO: 1229 - DNA, 17 bp, Artificial sequence
  Synthetic oligonucleotide
caagtttaatacccatc

SEQ ID NO: 1230 - DNA, 17 bp, Artificial sequence
  Synthetic oligonucleotide
acaagtttaatacccat

SEQ ID NO: 1231 - DNA, 17 bp, Artificial sequence
  Synthetic oligonucleotide
gacaagtttaataccca

SEQ ID NO: 1232 - DNA, 17 bp, Artificial sequence
  Synthetic oligonucleotide
tgacaagtttaataccc

SEQ ID NO: 1233 - DNA, 17 bp, Artificial sequence
  Synthetic oligonucleotide
ctgacaagtttaatacc

SEQ ID NO: 1234 - DNA, 17 bp, Artificial sequence
  Synthetic oligonucleotide
tctgacaagtttaatac

SEQ ID NO: 1235 - DNA, 17 bp, Artificial sequence
  Synthetic oligonucleotide
ttctgacaagtttaata

SEQ ID NO: 1236 - DNA, 17 bp, Artificial sequence
  Synthetic oligonucleotide
attctgacaagtttaat

SEQ ID NO: 1237 - DNA, 17 bp, Artificial sequence
  Synthetic oligonucleotide
aattctgacaagtttaa

SEQ ID NO: 1238 - DNA, 17 bp, Artificial sequence
  Synthetic oligonucleotide
aaattctgacaagttta

SEQ ID NO: 1239 - DNA, 17 bp, Artificial sequence
  Synthetic oligonucleotide
gaaattctgacaagttt

SEQ ID NO: 1240 - DNA, 17 bp, Artificial sequence
  Synthetic oligonucleotide
agaaattctgacaagtt

SEQ ID NO: 1241 - DNA, 17 bp, Artificial sequence
  Synthetic oligonucleotide
aagaaattctgacaagt

SEQ ID NO: 1242 - DNA, 17 bp, Artificial sequence
  Synthetic oligonucleotide
ttcacaggcttgaatga

SEQ ID NO: 1243 - DNA, 17 bp, Artificial sequence
  Synthetic oligonucleotide
attcacaggcttgaatg

SEQ ID NO: 1244 - DNA, 17 bp, Artificial sequence
  Synthetic oligonucleotide
tattcacaggcttgaat

SEQ ID NO: 1245 - DNA, 17 bp, Artificial sequence
  Synthetic oligonucleotide
ttattcacaggcttgaa

SEQ ID NO: 1246 - DNA, 17 bp, Artificial sequence
  Synthetic oligonucleotide
tttattcacaggcttga

SEQ ID NO: 1247 - DNA, 17 bp, Artificial sequence
  Synthetic oligonucleotide
ttttattcacaggcttg

SEQ ID NO: 1248 - DNA, 17 bp, Artificial sequence
  Synthetic oligonucleotide
tttttattcacaggctt

SEQ ID NO: 1249 - DNA, 17 bp, Artificial sequence
  Synthetic oligonucleotide
gtttttattcacaggct

SEQ ID NO: 1250 - DNA, 17 bp, Artificial sequence
  Synthetic oligonucleotide
ggtttttattcacaggc

SEQ ID NO: 1251 - DNA, 17 bp, Artificial sequence
  Synthetic oligonucleotide
gggtttttattcacagg

SEQ ID NO: 1252 - DNA, 17 bp, Artificial sequence
  Synthetic oligonucleotide
agggtttttattcacag

SEQ ID NO: 1253 - DNA, 17 bp, Artificial sequence
  Synthetic oligonucleotide
cagggtttttattcaca

SEQ ID NO: 1254 - DNA, 17 bp, Artificial sequence
  Synthetic oligonucleotide
acagggtttttattcac

SEQ ID NO: 1255 - DNA, 17 bp, Artificial sequence
  Synthetic oligonucleotide
tacagggtttttattca

SEQ ID NO: 1256 - DNA, 17 bp, Artificial sequence
  Synthetic oligonucleotide
atacagggtttttattc

SEQ ID NO: 1257 - DNA, 17 bp, Artificial sequence
  Synthetic oligonucleotide
catacagggtttttatt

SEQ ID NO: 1258 - DNA, 17 bp, Artificial sequence
  Synthetic oligonucleotide
ccatacagggtttttat

SEQ ID NO: 1259 - DNA, 17 bp, Artificial sequence
  Synthetic oligonucleotide
gccatacagggttttta

SEQ ID NO: 1260 - DNA, 17 bp, Artificial sequence
  Synthetic oligonucleotide
tgccatacagggttttt

SEQ ID NO: 1261 - DNA, 17 bp, Artificial sequence
  Synthetic oligonucleotide
gtgccatacagggtttt

SEQ ID NO: 1262 - DNA, 17 bp, Artificial sequence
  Synthetic oligonucleotide
agtgccatacagggttt

SEQ ID NO: 1263 - DNA, 17 bp, Artificial sequence
  Synthetic oligonucleotide
ttggattcttttaatag

SEQ ID NO: 1264 - DNA, 17 bp, Artificial sequence
  Synthetic oligonucleotide
ttttagtttgaatttgg

SEQ ID NO: 1265 - DNA, 20 bp, Artificial sequence
  Synthetic oligonucleotide
ctcgcccactctggccccaa

SEQ ID NO: 1266 - DNA, 20 bp, Artificial sequence
  Synthetic oligonucleotide
gcctcgcccactctggcccc

SEQ ID NO: 1267 - DNA, 20 bp, Artificial sequence
  Synthetic oligonucleotide
gcgcctcgcccactctggcc

SEQ ID NO: 1268 - DNA, 20 bp, Artificial sequence
  Synthetic oligonucleotide
ccgcgcctcgcccactctgg

SEQ ID NO: 1269 - DNA, 20 bp, Artificial sequence
  Synthetic oligonucleotide
ctccgcgcctcgcccactct

SEQ ID NO: 1270 - DNA, 20 bp, Artificial sequence
  Synthetic oligonucleotide
acctccgcgcctcgcccact

SEQ ID NO: 1271 - DNA, 20 bp, Artificial sequence
  Synthetic oligonucleotide
agacctccgcgcctcgccca

SEQ ID NO: 1272 - DNA, 20 bp, Artificial sequence
  Synthetic oligonucleotide
ccagacctccgcgcctcgcc

SEQ ID NO: 1273 - DNA, 20 bp, Artificial sequence
  Synthetic oligonucleotide
ggccagacctccgcgcctcg

SEQ ID NO: 1274 - DNA, 20 bp, Artificial sequence
  Synthetic oligonucleotide
tataggccagacctccgcgc

SEQ ID NO: 1275 - DNA, 20 bp, Artificial sequence
  Synthetic oligonucleotide
tttataggccagacctccgc

SEQ ID NO: 1276 - DNA, 20 bp, Artificial sequence
  Synthetic oligonucleotide
gactactttataggccagac

SEQ ID NO: 1277 - DNA, 20 bp, Artificial sequence
  Synthetic oligonucleotide
gcgactactttataggccag

SEQ ID NO: 1278 - DNA, 20 bp, Artificial sequence
  Synthetic oligonucleotide
ctccgcgactactttatagg

SEQ ID NO: 1279 - DNA, 20 bp, Artificial sequence
  Synthetic oligonucleotide
gtctccgcgactactttata

SEQ ID NO: 1280 - DNA, 20 bp, Artificial sequence
  Synthetic oligonucleotide
ccgtctccgcgactacttta

SEQ ID NO: 1281 - DNA, 20 bp, Artificial sequence
  Synthetic oligonucleotide
ccccgtctccgcgactactt

SEQ ID NO: 1282 - DNA, 20 bp, Artificial sequence
  Synthetic oligonucleotide
caccccgtctccgcgactac

SEQ ID NO: 1283 - DNA, 20 bp, Artificial sequence
  Synthetic oligonucleotide
agcaccccgtctccgcgact

SEQ ID NO: 1284 - DNA, 20 bp, Artificial sequence
  Synthetic oligonucleotide
ccagcaccccgtctccgcga

SEQ ID NO: 1285 - DNA, 20 bp, Artificial sequence
  Synthetic oligonucleotide
aaccagcaccccgtctccgc

SEQ ID NO: 1286 - DNA, 20 bp, Artificial sequence
  Synthetic oligonucleotide
caaaccagcaccccgtctcc

SEQ ID NO: 1287 - DNA, 20 bp, Artificial sequence
  Synthetic oligonucleotide
cgcaaaccagcaccccgtct

SEQ ID NO: 1288 - DNA, 20 bp, Artificial sequence
  Synthetic oligonucleotide
acgacgcaaaccagcacccc

SEQ ID NO: 1289 - DNA, 20 bp, Artificial sequence
  Synthetic oligonucleotide
ctacgacgcaaaccagcacc

SEQ ID NO: 1290 - DNA, 20 bp, Artificial sequence
  Synthetic oligonucleotide
gactacgacgcaaaccagca

SEQ ID NO: 1291 - DNA, 20 bp, Artificial sequence
  Synthetic oligonucleotide
gagactacgacgcaaaccag

SEQ ID NO: 1292 - DNA, 20 bp, Artificial sequence
  Synthetic oligonucleotide
aggagactacgacgcaaacc

SEQ ID NO: 1293 - DNA, 20 bp, Artificial sequence
  Synthetic oligonucleotide
gcaggagactacgacgcaaa

SEQ ID NO: 1294 - DNA, 20 bp, Artificial sequence
  Synthetic oligonucleotide
ctgcaggagactacgacgca

SEQ ID NO: 1295 - DNA, 20 bp, Artificial sequence
  Synthetic oligonucleotide
cgctgcaggagactacgacg

SEQ ID NO: 1296 - DNA, 20 bp, Artificial sequence
  Synthetic oligonucleotide
tgcaacggaaaccccagacg

SEQ ID NO: 1297 - DNA, 20 bp, Artificial sequence
  Synthetic oligonucleotide
actgcaacggaaaccccaga

SEQ ID NO: 1298 - DNA, 20 bp, Artificial sequence
  Synthetic oligonucleotide
gaggactgcaacggaaaccc

SEQ ID NO: 1299 - DNA, 20 bp, Artificial sequence
  Synthetic oligonucleotide
ccgaggactgcaacggaaac

SEQ ID NO: 1300 - DNA, 20 bp, Artificial sequence
  Synthetic oligonucleotide
ttccgaggactgcaacggaa

SEQ ID NO: 1301 - DNA, 20 bp, Artificial sequence
  Synthetic oligonucleotide
ctggttccgaggactgcaac

SEQ ID NO: 1302 - DNA, 20 bp, Artificial sequence
  Synthetic oligonucleotide
ggtcctggttccgaggactg

SEQ ID NO: 1303 - DNA, 20 bp, Artificial sequence
  Synthetic oligonucleotide
ccgaggtcctggttccgagg

SEQ ID NO: 1304 - DNA, 20 bp, Artificial sequence
  Synthetic oligonucleotide
cgccgaggtcctggttccga

SEQ ID NO: 1305 - DNA, 20 bp, Artificial sequence
  Synthetic oligonucleotide
cacgccgaggtcctggttcc

SEQ ID NO: 1306 - DNA, 20 bp, Artificial sequence
  Synthetic oligonucleotide
gccacgccgaggtcctggtt

SEQ ID NO: 1307 - DNA, 20 bp, Artificial sequence
  Synthetic oligonucleotide
ctaggccacgccgaggtcct

SEQ ID NO: 1308 - DNA, 20 bp, Artificial sequence
  Synthetic oligonucleotide
cgctaggccacgccgaggtc

SEQ ID NO: 1309 - DNA, 20 bp, Artificial sequence
  Synthetic oligonucleotide
ctcgctaggccacgccgagg

SEQ ID NO: 1310 - DNA, 20 bp, Artificial sequence
  Synthetic oligonucleotide
aactcgctaggccacgccga

SEQ ID NO: 1311 - DNA, 20 bp, Artificial sequence
  Synthetic oligonucleotide
ataactcgctaggccacgcc

SEQ ID NO: 1312 - DNA, 20 bp, Artificial sequence
  Synthetic oligonucleotide
ccataactcgctaggccacg

SEQ ID NO: 1313 - DNA, 20 bp, Artificial sequence
  Synthetic oligonucleotide
cgccataactcgctaggcca

SEQ ID NO: 1314 - DNA, 20 bp, Artificial sequence
  Synthetic oligonucleotide
tgggccgtcgcccttcagca

SEQ ID NO: 1315 - DNA, 20 bp, Artificial sequence
  Synthetic oligonucleotide
actgggccgtcgcccttcag

SEQ ID NO: 1316 - DNA, 20 bp, Artificial sequence
  Synthetic oligonucleotide
gcactgggccgtcgcccttc

SEQ ID NO: 1317 - DNA, 20 bp, Artificial sequence
  Synthetic oligonucleotide
ctgcactgggccgtcgccct

SEQ ID NO: 1318 - DNA, 20 bp, Artificial sequence
  Synthetic oligonucleotide
tgccctgcactgggccgtcg

SEQ ID NO: 1319 - DNA, 20 bp, Artificial sequence
  Synthetic oligonucleotide
gatgccctgcactgggccgt

SEQ ID NO: 1320 - DNA, 20 bp, Artificial sequence
  Synthetic oligonucleotide
atgatgccctgcactgggcc

SEQ ID NO: 1321 - DNA, 20 bp, Artificial sequence
  Synthetic oligonucleotide
attgatgatgccctgcactg

SEQ ID NO: 1322 - DNA, 20 bp, Artificial sequence
  Synthetic oligonucleotide
aaattgatgatgccctgcac

SEQ ID NO: 1323 - DNA, 20 bp, Artificial sequence
  Synthetic oligonucleotide
cgaaattgatgatgccctgc

SEQ ID NO: 1324 - DNA, 20 bp, Artificial sequence
  Synthetic oligonucleotide
ctcgaaattgatgatgccct

SEQ ID NO: 1325 - DNA, 20 bp, Artificial sequence
  Synthetic oligonucleotide
tgctcgaaattgatgatgcc

SEQ ID NO: 1326 - DNA, 20 bp, Artificial sequence
  Synthetic oligonucleotide
tctgctcgaaattgatgatg

SEQ ID NO: 1327 - DNA, 20 bp, Artificial sequence
  Synthetic oligonucleotide
cttctgctcgaaattgatga

SEQ ID NO: 1328 - DNA, 20 bp, Artificial sequence
  Synthetic oligonucleotide
tttaatgcttccccacacct

SEQ ID NO: 1329 - DNA, 20 bp, Artificial sequence
  Synthetic oligonucleotide
cctttaatgcttccccacac

SEQ ID NO: 1330 - DNA, 20 bp, Artificial sequence
  Synthetic oligonucleotide
gtcctttaatgcttccccac

SEQ ID NO: 1331 - DNA, 17 bp, Artificial sequence
  Synthetic oligonucleotide
cccttcagcacgcacac

SEQ ID NO: 1332 - DNA, 17 bp, Artificial sequence
  Synthetic oligonucleotide
gcccttcagcacgcaca

SEQ ID NO: 1333 - DNA, 17 bp, Artificial sequence
  Synthetic oligonucleotide
cgcccttcagcacgcac

SEQ ID NO: 1334 - DNA, 17 bp, Artificial sequence
  Synthetic oligonucleotide
caccacaagccaaacga

SEQ ID NO: 1335 - DNA, 17 bp, Artificial sequence
  Synthetic oligonucleotide
acaccacaagccaaacg

SEQ ID NO: 1336 - DNA, 17 bp, Artificial sequence
  Synthetic oligonucleotide
tacaccacaagccaaac

SEQ ID NO: 1337 - DNA, 17 bp, Artificial sequence
  Synthetic oligonucleotide
ttacaccacaagccaaa

SEQ ID NO: 1338 - DNA, 17 bp, Artificial sequence
  Synthetic oligonucleotide
attacaccacaagccaa

SEQ ID NO: 1339 - DNA, 17 bp, Artificial sequence
  Synthetic oligonucleotide
aacagatgagttaaggg

SEQ ID NO: 1340 - DNA, 17 bp, Artificial sequence
  Synthetic oligonucleotide
taacagatgagttaagg

SEQ ID NO: 1341 - DNA, 17 bp, Artificial sequence
  Synthetic oligonucleotide
ataacagatgagttaag

SEQ ID NO: 1342 - DNA, 17 bp, Artificial sequence
  Synthetic oligonucleotide
ggatacatttctacagc

SEQ ID NO: 1343 - DNA, 17 bp, Artificial sequence
  Synthetic oligonucleotide
aggatacatttctacag

SEQ ID NO: 1344 - DNA, 17 bp, Artificial sequence
  Synthetic oligonucleotide
caggatacatttctaca

SEQ ID NO: 1345 - DNA, 17 bp, Artificial sequence
  Synthetic oligonucleotide
ttatcaggatacatttc

SEQ ID NO: 1346 - DNA, 17 bp, Artificial sequence
  Synthetic oligonucleotide
gtttatcaggatacatt

SEQ ID NO: 1347 - DNA, 17 bp, Artificial sequence
  Synthetic oligonucleotide
tgtttatcaggatacat

SEQ ID NO: 1348 - DNA, 17 bp, Artificial sequence
  Synthetic oligonucleotide
atgtttatcaggataca

SEQ ID NO: 1349 - DNA, 17 bp, Artificial sequence
  Synthetic oligonucleotide
aatgtttatcaggatac

SEQ ID NO: 1350 - DNA, 17 bp, Artificial sequence
  Synthetic oligonucleotide
taatgtttatcaggata

SEQ ID NO: 1351 - DNA, 17 bp, Artificial sequence
  Synthetic oligonucleotide
ttaatgtttatcaggat

SEQ ID NO: 1352 - DNA, 17 bp, Artificial sequence
  Synthetic oligonucleotide
gtttaatgtttatcagg

SEQ ID NO: 1353 - DNA, 17 bp, Artificial sequence
  Synthetic oligonucleotide
cttttaagattacagtg

SEQ ID NO: 1354 - DNA, 17 bp, Artificial sequence
  Synthetic oligonucleotide
cacttttaagattacag

SEQ ID NO: 1355 - DNA, 17 bp, Artificial sequence
  Synthetic oligonucleotide
tcacacaattacacttt

SEQ ID NO: 1356 - DNA, 17 bp, Artificial sequence
  Synthetic oligonucleotide
gtcacacaattacactt

SEQ ID NO: 1357 - DNA, 17 bp, Artificial sequence
  Synthetic oligonucleotide
aagtcacacaattacac

SEQ ID NO: 1358 - DNA, 17 bp, Artificial sequence
  Synthetic oligonucleotide
aggtactttaaagcaac

SEQ ID NO: 1359 - DNA, 17 bp, Artificial sequence
  Synthetic oligonucleotide
acaggtactttaaagca

SEQ ID NO: 1360 - DNA, 17 bp, Artificial sequence
  Synthetic oligonucleotide
tacaggtactttaaagc

SEQ ID NO: 1361 - DNA, 17 bp, Artificial sequence
  Synthetic oligonucleotide
ctacaggtactttaaag

SEQ ID NO: 1362 - DNA, 17 bp, Artificial sequence
  Synthetic oligonucleotide
cactacaggtactttaa

SEQ ID NO: 1363 - DNA, 17 bp, Artificial sequence
  Synthetic oligonucleotide
tcactacaggtacttta

SEQ ID NO: 1364 - DNA, 17 bp, Artificial sequence
  Synthetic oligonucleotide
ctcactacaggtacttt

SEQ ID NO: 1365 - DNA, 17 bp, Artificial sequence
  Synthetic oligonucleotide
tctcactacaggtactt

SEQ ID NO: 1366 - DNA, 17 bp, Artificial sequence
  Synthetic oligonucleotide
ttctcactacaggtact

SEQ ID NO: 1367 - DNA, 17 bp, Artificial sequence
  Synthetic oligonucleotide
tttctcactacaggtac

SEQ ID NO: 1368 - DNA, 17 bp, Artificial sequence
  Synthetic oligonucleotide
gtttctcactacaggta

SEQ ID NO: 1369 - DNA, 17 bp, Artificial sequence
  Synthetic oligonucleotide
agtttctcactacaggt

SEQ ID NO: 1370 - DNA, 17 bp, Artificial sequence
  Synthetic oligonucleotide
cagtttctcactacagg

SEQ ID NO: 1371 - DNA, 17 bp, Artificial sequence
  Synthetic oligonucleotide
tcagtttctcactacag

SEQ ID NO: 1372 - DNA, 17 bp, Artificial sequence
  Synthetic oligonucleotide
atcagtttctcactaca

SEQ ID NO: 1373 - DNA, 17 bp, Artificial sequence
  Synthetic oligonucleotide
aatcagtttctcactac

SEQ ID NO: 1374 - DNA, 17 bp, Artificial sequence
  Synthetic oligonucleotide
gatcataaatcagtttc

SEQ ID NO: 1375 - DNA, 17 bp, Artificial sequence
  Synthetic oligonucleotide
tgatcataaatcagttt

SEQ ID NO: 1376 - DNA, 17 bp, Artificial sequence
  Synthetic oligonucleotide
gtgatcataaatcagtt

SEQ ID NO: 1377 - DNA, 17 bp, Artificial sequence
  Synthetic oligonucleotide
agtgatcataaatcagt

SEQ ID NO: 1378 - DNA, 17 bp, Artificial sequence
  Synthetic oligonucleotide
caagtgatcataaatca

SEQ ID NO: 1379 - DNA, 17 bp, Artificial sequence
  Synthetic oligonucleotide
ccaagtgatcataaatc

SEQ ID NO: 1380 - DNA, 17 bp, Artificial sequence
  Synthetic oligonucleotide
tccaagtgatcataaat

SEQ ID NO: 1381 - DNA, 17 bp, Artificial sequence
  Synthetic oligonucleotide
cttccaagtgatcataa

SEQ ID NO: 1382 - DNA, 17 bp, Artificial sequence
  Synthetic oligonucleotide
tcttccaagtgatcata

SEQ ID NO: 1383 - DNA, 17 bp, Artificial sequence
  Synthetic oligonucleotide
agacattttaactgagt

SEQ ID NO: 1384 - DNA, 17 bp, Artificial sequence
  Synthetic oligonucleotide
gatttaagtctggcaaa

SEQ ID NO: 1385 - DNA, 17 bp, Artificial sequence
  Synthetic oligonucleotide
tgatttaagtctggcaa

SEQ ID NO: 1386 - DNA, 17 bp, Artificial sequence
  Synthetic oligonucleotide
gtgatttaagtctggca

SEQ ID NO: 1387 - DNA, 17 bp, Artificial sequence
  Synthetic oligonucleotide
tgtgatttaagtctggc

SEQ ID NO: 1388 - DNA, 17 bp, Artificial sequence
  Synthetic oligonucleotide
ctgtgatttaagtctgg

SEQ ID NO: 1389 - DNA, 17 bp, Artificial sequence
  Synthetic oligonucleotide
tctgtgatttaagtctg

SEQ ID NO: 1390 - DNA, 17 bp, Artificial sequence
  Synthetic oligonucleotide
atctgtgatttaagtct

SEQ ID NO: 1391 - DNA, 17 bp, Artificial sequence
  Synthetic oligonucleotide
catctgtgatttaagtc

SEQ ID NO: 1392 - DNA, 17 bp, Artificial sequence
  Synthetic oligonucleotide
ccatctgtgatttaagt

SEQ ID NO: 1393 - DNA, 17 bp, Artificial sequence
  Synthetic oligonucleotide
cccatctgtgatttaag

SEQ ID NO: 1394 - DNA, 17 bp, Artificial sequence
  Synthetic oligonucleotide
acccatctgtgatttaa

SEQ ID NO: 1395 - DNA, 17 bp, Artificial sequence
  Synthetic oligonucleotide
tacccatctgtgattta

SEQ ID NO: 1396 - DNA, 17 bp, Artificial sequence
  Synthetic oligonucleotide
gcttgaatgacaaagaa

SEQ ID NO: 1397 - DNA, 17 bp, Artificial sequence
  Synthetic oligonucleotide
ggcttgaatgacaaaga

SEQ ID NO: 1398 - DNA, 17 bp, Artificial sequence
  Synthetic oligonucleotide
cacaggcttgaatgaca

SEQ ID NO: 1399 - DNA, 17 bp, Artificial sequence
  Synthetic oligonucleotide
tcacaggcttgaatgac

SEQ ID NO: 1400 - DNA, 17 bp, Artificial sequence
  Synthetic oligonucleotide
aagtgccatacagggtt

SEQ ID NO: 1401 - DNA, 17 bp, Artificial sequence
  Synthetic oligonucleotide
taagtgccatacagggt

SEQ ID NO: 1402 - DNA, 17 bp, Artificial sequence
  Synthetic oligonucleotide
ataagtgccatacaggg

SEQ ID NO: 1403 - DNA, 17 bp, Artificial sequence
  Synthetic oligonucleotide
aataagtgccatacagg

SEQ ID NO: 1404 - DNA, 17 bp, Artificial sequence
  Synthetic oligonucleotide
taataagtgccatacag

SEQ ID NO: 1405 - DNA, 17 bp, Artificial sequence
  Synthetic oligonucleotide
ataataagtgccataca

SEQ ID NO: 1406 - DNA, 17 bp, Artificial sequence
  Synthetic oligonucleotide
cataataagtgccatac

SEQ ID NO: 1407 - DNA, 17 bp, Artificial sequence
  Synthetic oligonucleotide
tcataataagtgccata

SEQ ID NO: 1408 - DNA, 17 bp, Artificial sequence
  Synthetic oligonucleotide
ctcataataagtgccat

SEQ ID NO: 1409 - DNA, 17 bp, Artificial sequence
  Synthetic oligonucleotide
cctcataataagtgcca

SEQ ID NO: 1410 - DNA, 17 bp, Artificial sequence
  Synthetic oligonucleotide
gcctcataataagtgcc

SEQ ID NO: 1411 - DNA, 17 bp, Artificial sequence
  Synthetic oligonucleotide
agcctcataataagtgc

SEQ ID NO: 1412 - DNA, 17 bp, Artificial sequence
  Synthetic oligonucleotide
tagcctcataataagtg

SEQ ID NO: 1413 - DNA, 17 bp, Artificial sequence
  Synthetic oligonucleotide
atagcctcataataagt

SEQ ID NO: 1414 - DNA, 17 bp, Artificial sequence
  Synthetic oligonucleotide
aatagcctcataataag

SEQ ID NO: 1415 - DNA, 17 bp, Artificial sequence
  Synthetic oligonucleotide
cttttaatagcctcata

SEQ ID NO: 1416 - DNA, 17 bp, Artificial sequence
  Synthetic oligonucleotide
tcttttaatagcctcat

SEQ ID NO: 1417 - DNA, 17 bp, Artificial sequence
  Synthetic oligonucleotide
ggattcttttaatagcc

SEQ ID NO: 1418 - DNA, 17 bp, Artificial sequence
  Synthetic oligonucleotide
ttagtttgaatttggat

SEQ ID NO: 1419 - DNA, 18 bp, Artificial sequence
  Synthetic oligonucleotide
gtcgcccttcagcacgca

SEQ ID NO: 1420 - DNA, 16 bp, Artificial sequence
  Synthetic oligonucleotide
cccacaccttcactgg

SEQ ID NO: 1421 - DNA, 18 bp, Artificial sequence
  Synthetic oligonucleotide
ttccccacaccttcactg

SEQ ID NO: 1422 - DNA, 16 bp, Artificial sequence
  Synthetic oligonucleotide
ccccacaccttcactg

SEQ ID NO: 1423 - DNA, 18 bp, Artificial sequence
  Synthetic oligonucleotide
cttccccacaccttcact

SEQ ID NO: 1424 - DNA, 16 bp, Artificial sequence
  Synthetic oligonucleotide
tccccacaccttcact

SEQ ID NO: 1425 - DNA, 18 bp, Artificial sequence
  Synthetic oligonucleotide
gcttccccacaccttcac

SEQ ID NO: 1426 - DNA, 16 bp, Artificial sequence
  Synthetic oligonucleotide
ttccccacaccttcac

SEQ ID NO: 1427 - DNA, 16 bp, Artificial sequence
  Synthetic oligonucleotide
cttccccacaccttca

SEQ ID NO: 1428 - DNA, 19 bp, Artificial sequence
  Synthetic oligonucleotide
aggatacatttctacagct

SEQ ID NO: 1429 - DNA, 18 bp, Artificial sequence
  Synthetic oligonucleotide
atacatttctacagctag

SEQ ID NO: 1430 - DNA, 18 bp, Artificial sequence
  Synthetic oligonucleotide
gatacatttctacagcta

SEQ ID NO: 1431 - DNA, 16 bp, Artificial sequence
  Synthetic oligonucleotide
tacatttctacagcta

SEQ ID NO: 1432 - DNA, 18 bp, Artificial sequence
  Synthetic oligonucleotide
ggatacatttctacagct

SEQ ID NO: 1433 - DNA, 16 bp, Artificial sequence
  Synthetic oligonucleotide
atacatttctacagct

SEQ ID NO: 1434 - DNA, 18 bp, Artificial sequence
  Synthetic oligonucleotide
aggatacatttctacagc

SEQ ID NO: 1435 - DNA, 16 bp, Artificial sequence
  Synthetic oligonucleotide
gatacatttctacagc

SEQ ID NO: 1436 - DNA, 18 bp, Artificial sequence
  Synthetic oligonucleotide
caggatacatttctacag

SEQ ID NO: 1437 - DNA, 16 bp, Artificial sequence
  Synthetic oligonucleotide
atgtttatcaggatac

SEQ ID NO: 1438 - DNA, 18 bp, Artificial sequence
  Synthetic oligonucleotide
ttaatgtttatcaggata

SEQ ID NO: 1439 - DNA, 18 bp, Artificial sequence
  Synthetic oligonucleotide
tttaatgtttatcaggat

SEQ ID NO: 1440 - DNA, 18 bp, Artificial sequence
  Synthetic oligonucleotide
gtttaatgtttatcagga

SEQ ID NO: 1441 - DNA, 16 bp, Artificial sequence
  Synthetic oligonucleotide
ttaatgtttatcagga

SEQ ID NO: 1442 - DNA, 18 bp, Artificial sequence
  Synthetic oligonucleotide
tgtttaatgtttatcagg

SEQ ID NO: 1443 - DNA, 16 bp, Artificial sequence
  Synthetic oligonucleotide
tttaatgtttatcagg

SEQ ID NO: 1444 - DNA, 18 bp, Artificial sequence
  Synthetic oligonucleotide
gtgtttaatgtttatcag

SEQ ID NO: 1445 - DNA, 16 bp, Artificial sequence
  Synthetic oligonucleotide
gtttaatgtttatcag

SEQ ID NO: 1446 - DNA, 18 bp, Artificial sequence
  Synthetic oligonucleotide
agtgtttaatgtttatca

SEQ ID NO: 1447 - DNA, 16 bp, Artificial sequence
  Synthetic oligonucleotide
tgtttaatgtttatca

SEQ ID NO: 1448 - DNA, 18 bp, Artificial sequence
  Synthetic oligonucleotide
cagtgtttaatgtttatc

SEQ ID NO: 1449 - DNA, 16 bp, Artificial sequence
  Synthetic oligonucleotide
gtgtttaatgtttatc

SEQ ID NO: 1450 - DNA, 18 bp, Artificial sequence
  Synthetic oligonucleotide
acagtgtttaatgtttat

SEQ ID NO: 1451 - DNA, 18 bp, Artificial sequence
  Synthetic oligonucleotide
tacagtgtttaatgttta

SEQ ID NO: 1452 - DNA, 16 bp, Artificial sequence
  Synthetic oligonucleotide
cagtgtttaatgttta

SEQ ID NO: 1453 - DNA, 18 bp, Artificial sequence
  Synthetic oligonucleotide
ttacagtgtttaatgttt

SEQ ID NO: 1454 - DNA, 16 bp, Artificial sequence
  Synthetic oligonucleotide
acagtgtttaatgttt

SEQ ID NO: 1455 - DNA, 16 bp, Artificial sequence
  Synthetic oligonucleotide
ggatacatttctacag

SEQ ID NO: 1456 - DNA, 16 bp, Artificial sequence
  Synthetic oligonucleotide
taatgtttatcaggat

SEQ ID NO: 1457 - DNA, 16 bp, Artificial sequence
  Synthetic oligonucleotide
agtgtttaatgtttat

SEQ ID NO: 1458 - DNA, 16 bp, Artificial sequence
  Synthetic oligonucleotide
catttctacagctagc

SEQ ID NO: 1459 - DNA, 16 bp, Artificial sequence
  Synthetic oligonucleotide
acatttctacagctag

SEQ ID NO: 1460 - DNA, 16 bp, Artificial sequence
  Synthetic oligonucleotide
aatgtttatcaggata

SEQ ID NO: 1461 - DNA, 19 bp, Artificial sequence
  Synthetic oligonucleotide
caggatacatttctacagc